European Patent Specification EP 3 927 817 B1, published August 20, 2025. Title: NEW RECOMBINANT DIAMINE OXIDASE AND ITS USE FOR THE TREATMENT OF DISEASES CHARACTERIZED BY EXCESS HISTAMINE. Applicant: Medizinische Universität Wien Universität für Bodenkultur Wien. The sequence listing filed with the application follows.

SEQUENCE LISTING (106 sequences)

SEQ ID NO: 1 - protein, 751 aa, Homo sapiens
MPALGWAVAAILMLQTAMAEPSPGTLPRKAGVFSDLSNQELKAVHSFLWSKKELRLQPSSTTTMAKNTVFLIEMLLPKKYHVLRFLDKGERHPVREARAVIFFGDQEHPNVTEFAVGPLPGPCYMRALSPRPGYQSSWASRPISTAEYALLYHTLQEATKPLHQFFLNTTGFSFQDCHDRCLAFTDVAPRGVASGQRRSWLIIQRYVEGYFLHPTGLELLVDHGSTDAGHWAVEQVWYNGKFYGSPEELARKYADGEVDVVVLEDPLPGGKGHDSTEEPPLFSSHKPRGDFPSPIHVSGPRLVQPHGPRFRLEGNAVLYGGWSFAFRLRSSSGLQVLNVHFGGERIAYEVSVQEAVALYGGHTPAGMQTKYLDVGWGLGSVTHELAPGIDCPETATFLDTFHYYDADDPVHYPRALCLFEMPTGVPLRRHFNSNFKGGFNFYAGLKGQVLVLRTTSTVYNYDYIWDFIFYPNGVMEAKMHATGYVHATFYTPEGLRHGTRLHTHLIGNIHTHLVHYRVDLDVAGTKNSFQTLQMKLENITNPWSPRHRVVQPTLEQTQYSWERQAAFRFKRKLPKYLLFTSPQENPWGHKRSYRLQIHSMADQVLPPGWQEEQAITWARYPLAVTKYRESELCSSSIYHQNDPWHPPVVFEQFLHNNENIENEDLVAWVTVGFLHIPHSEDIPNTATPGNSVGFLLRPFNFFPEDPSLASRDTVIVWPRDNGPNYVQRWIPEDRDCSMPPPFSYNGTYRPV

SEQ ID NO: 2 - protein, 751 aa, Artificial Sequence
  hDAO-Hepmut1
MPALGWAVAAILMLQTAMAEPSPGTLPRKAGVFSDLSNQELKAVHSFLWSKKELRLQPSSTTTMAKNTVFLIEMLLPKKYHVLRFLDKGERHPVREARAVIFFGDQEHPNVTEFAVGPLPGPCYMRALSPRPGYQSSWASRPISTAEYALLYHTLQEATKPLHQFFLNTTGFSFQDCHDRCLAFTDVAPRGVASGQRRSWLIIQRYVEGYFLHPTGLELLVDHGSTDAGHWAVEQVWYNGKFYGSPEELARKYADGEVDVVVLEDPLPGGKGHDSTEEPPLFSSHKPRGDFPSPIHVSGPRLVQPHGPRFRLEGNAVLYGGWSFAFRLRSSSGLQVLNVHFGGERIAYEVSVQEAVALYGGHTPAGMQTKYLDVGWGLGSVTHELAPGIDCPETATFLDTFHYYDADDPVHYPRALCLFEMPTGVPLRRHFNSNFKGGFNFYAGLKGQVLVLRTTSTVYNYDYIWDFIFYPNGVMEAKMHATGYVHATFYTPEGLRHGTRLHTHLIGNIHTHLVHYRVDLDVAGTKNSFQTLQMKLENITNPWSPRHRVVQPTLEQTQYSWERQAAFSFKRKLPKYLLFTSPQENPWGHKRSYRLQIHSMADQVLPPGWQEEQAITWARYPLAVTKYRESELCSSSIYHQNDPWHPPVVFEQFLHNNENIENEDLVAWVTVGFLHIPHSEDIPNTATPGNSVGFLLRPFNFFPEDPSLASRDTVIVWPRDNGPNYVQRWIPEDRDCSMPPPFSYNGTYRPV

SEQ ID NO: 3 - protein, 751 aa, Artificial Sequence
  hDAO-Hepmut2
MPALGWAVAAILMLQTAMAEPSPGTLPRKAGVFSDLSNQELKAVHSFLWSKKELRLQPSSTTTMAKNTVFLIEMLLPKKYHVLRFLDKGERHPVREARAVIFFGDQEHPNVTEFAVGPLPGPCYMRALSPRPGYQSSWASRPISTAEYALLYHTLQEATKPLHQFFLNTTGFSFQDCHDRCLAFTDVAPRGVASGQRRSWLIIQRYVEGYFLHPTGLELLVDHGSTDAGHWAVEQVWYNGKFYGSPEELARKYADGEVDVVVLEDPLPGGKGHDSTEEPPLFSSHKPRGDFPSPIHVSGPRLVQPHGPRFRLEGNAVLYGGWSFAFRLRSSSGLQVLNVHFGGERIAYEVSVQEAVALYGGHTPAGMQTKYLDVGWGLGSVTHELAPGIDCPETATFLDTFHYYDADDPVHYPRALCLFEMPTGVPLRRHFNSNFKGGFNFYAGLKGQVLVLRTTSTVYNYDYIWDFIFYPNGVMEAKMHATGYVHATFYTPEGLRHGTRLHTHLIGNIHTHLVHYRVDLDVAGTKNSFQTLQMKLENITNPWSPRHRVVQPTLEQTQYSWERQAAFRFKRKLPTYLLFTSPQENPWGHKRSYRLQIHSMADQVLPPGWQEEQAITWARYPLAVTKYRESELCSSSIYHQNDPWHPPVVFEQFLHNNENIENEDLVAWVTVGFLHIPHSEDIPNTATPGNSVGFLLRPFNFFPEDPSLASRDTVIVWPRDNGPNYVQRWIPEDRDCSMPPPFSYNGTYRPV

SEQ ID NO: 4 - protein, 751 aa, Artificial Sequence
  hDAO-Hepmut3
MPALGWAVAAILMLQTAMAEPSPGTLPRKAGVFSDLSNQELKAVHSFLWSKKELRLQPSSTTTMAKNTVFLIEMLLPKKYHVLRFLDKGERHPVREARAVIFFGDQEHPNVTEFAVGPLPGPCYMRALSPRPGYQSSWASRPISTAEYALLYHTLQEATKPLHQFFLNTTGFSFQDCHDRCLAFTDVAPRGVASGQRRSWLIIQRYVEGYFLHPTGLELLVDHGSTDAGHWAVEQVWYNGKFYGSPEELARKYADGEVDVVVLEDPLPGGKGHDSTEEPPLFSSHKPRGDFPSPIHVSGPRLVQPHGPRFRLEGNAVLYGGWSFAFRLRSSSGLQVLNVHFGGERIAYEVSVQEAVALYGGHTPAGMQTKYLDVGWGLGSVTHELAPGIDCPETATFLDTFHYYDADDPVHYPRALCLFEMPTGVPLRRHFNSNFKGGFNFYAGLKGQVLVLRTTSTVYNYDYIWDFIFYPNGVMEAKMHATGYVHATFYTPEGLRHGTRLHTHLIGNIHTHLVHYRVDLDVAGTKNSFQTLQMKLENITNPWSPRHRVVQPTLEQTQYSWERQAAFRFKTKLPKYLLFTSPQENPWGHKRSYRLQIHSMADQVLPPGWQEEQAITWARYPLAVTKYRESELCSSSIYHQNDPWHPPVVFEQFLHNNENIENEDLVAWVTVGFLHIPHSEDIPNTATPGNSVGFLLRPFNFFPEDPSLASRDTVIVWPRDNGPNYVQRWIPEDRDCSMPPPFSYNGTYRPV

SEQ ID NO: 5 - protein, 751 aa, Artificial Sequence
  hDAO-Hepmut4
MPALGWAVAAILMLQTAMAEPSPGTLPRKAGVFSDLSNQELKAVHSFLWSKKELRLQPSSTTTMAKNTVFLIEMLLPKKYHVLRFLDKGERHPVREARAVIFFGDQEHPNVTEFAVGPLPGPCYMRALSPRPGYQSSWASRPISTAEYALLYHTLQEATKPLHQFFLNTTGFSFQDCHDRCLAFTDVAPRGVASGQRRSWLIIQRYVEGYFLHPTGLELLVDHGSTDAGHWAVEQVWYNGKFYGSPEELARKYADGEVDVVVLEDPLPGGKGHDSTEEPPLFSSHKPRGDFPSPIHVSGPRLVQPHGPRFRLEGNAVLYGGWSFAFRLRSSSGLQVLNVHFGGERIAYEVSVQEAVALYGGHTPAGMQTKYLDVGWGLGSVTHELAPGIDCPETATFLDTFHYYDADDPVHYPRALCLFEMPTGVPLRRHFNSNFKGGFNFYAGLKGQVLVLRTTSTVYNYDYIWDFIFYPNGVMEAKMHATGYVHATFYTPEGLRHGTRLHTHLIGNIHTHLVHYRVDLDVAGTKNSFQTLQMKLENITNPWSPRHRVVQPTLEQTQYSWERQAAFSFKTKLPKYLLFTSPQENPWGHKRSYRLQIHSMADQVLPPGWQEEQAITWARYPLAVTKYRESELCSSSIYHQNDPWHPPVVFEQFLHNNENIENEDLVAWVTVGFLHIPHSEDIPNTATPGNSVGFLLRPFNFFPEDPSLASRDTVIVWPRDNGPNYVQRWIPEDRDCSMPPPFSYNGTYRPV

SEQ ID NO: 6 - protein, 751 aa, Artificial Sequence
  hDAO-Hepmut5
MPALGWAVAAILMLQTAMAEPSPGTLPRKAGVFSDLSNQELKAVHSFLWSKKELRLQPSSTTTMAKNTVFLIEMLLPKKYHVLRFLDKGERHPVREARAVIFFGDQEHPNVTEFAVGPLPGPCYMRALSPRPGYQSSWASRPISTAEYALLYHTLQEATKPLHQFFLNTTGFSFQDCHDRCLAFTDVAPRGVASGQRRSWLIIQRYVEGYFLHPTGLELLVDHGSTDAGHWAVEQVWYNGKFYGSPEELARKYADGEVDVVVLEDPLPGGKGHDSTEEPPLFSSHKPRGDFPSPIHVSGPRLVQPHGPRFRLEGNAVLYGGWSFAFRLRSSSGLQVLNVHFGGERIAYEVSVQEAVALYGGHTPAGMQTKYLDVGWGLGSVTHELAPGIDCPETATFLDTFHYYDADDPVHYPRALCLFEMPTGVPLRRHFNSNFKGGFNFYAGLKGQVLVLRTTSTVYNYDYIWDFIFYPNGVMEAKMHATGYVHATFYTPEGLRHGTRLHTHLIGNIHTHLVHYRVDLDVAGTKNSFQTLQMKLENITNPWSPRHRVVQPTLEQTQYSWERQAAFRFKTKLPTYLLFTSPQENPWGHKRSYRLQIHSMADQVLPPGWQEEQAITWARYPLAVTKYRESELCSSSIYHQNDPWHPPVVFEQFLHNNENIENEDLVAWVTVGFLHIPHSEDIPNTATPGNSVGFLLRPFNFFPEDPSLASRDTVIVWPRDNGPNYVQRWIPEDRDCSMPPPFSYNGTYRPV

SEQ ID NO: 7 - protein, 751 aa, Artificial Sequence
  hDAO-Hepmut6
MPALGWAVAAILMLQTAMAEPSPGTLPRKAGVFSDLSNQELKAVHSFLWSKKELRLQPSSTTTMAKNTVFLIEMLLPKKYHVLRFLDKGERHPVREARAVIFFGDQEHPNVTEFAVGPLPGPCYMRALSPRPGYQSSWASRPISTAEYALLYHTLQEATKPLHQFFLNTTGFSFQDCHDRCLAFTDVAPRGVASGQRRSWLIIQRYVEGYFLHPTGLELLVDHGSTDAGHWAVEQVWYNGKFYGSPEELARKYADGEVDVVVLEDPLPGGKGHDSTEEPPLFSSHKPRGDFPSPIHVSGPRLVQPHGPRFRLEGNAVLYGGWSFAFRLRSSSGLQVLNVHFGGERIAYEVSVQEAVALYGGHTPAGMQTKYLDVGWGLGSVTHELAPGIDCPETATFLDTFHYYDADDPVHYPRALCLFEMPTGVPLRRHFNSNFKGGFNFYAGLKGQVLVLRTTSTVYNYDYIWDFIFYPNGVMEAKMHATGYVHATFYTPEGLRHGTRLHTHLIGNIHTHLVHYRVDLDVAGTKNSFQTLQMKLENITNPWSPRHRVVQPTLEQTQYSWERQAAFRFGQTLPKYLLFTSPQENPWGHKRSYRLQIHSMADQVLPPGWQEEQAITWARYPLAVTKYRESELCSSSIYHQNDPWHPPVVFEQFLHNNENIENEDLVAWVTVGFLHIPHSEDIPNTATPGNSVGFLLRPFNFFPEDPSLASRDTVIVWPRDNGPNYVQRWIPEDRDCSMPPPFSYNGTYRPV

SEQ ID NO: 8 - protein, 751 aa, Artificial Sequence
  hDAO-Hepmut7
MPALGWAVAAILMLQTAMAEPSPGTLPRKAGVFSDLSNQELKAVHSFLWSKKELRLQPSSTTTMAKNTVFLIEMLLPKKYHVLRFLDKGERHPVREARAVIFFGDQEHPNVTEFAVGPLPGPCYMRALSPRPGYQSSWASRPISTAEYALLYHTLQEATKPLHQFFLNTTGFSFQDCHDRCLAFTDVAPRGVASGQRRSWLIIQRYVEGYFLHPTGLELLVDHGSTDAGHWAVEQVWYNGKFYGSPEELARKYADGEVDVVVLEDPLPGGKGHDSTEEPPLFSSHKPRGDFPSPIHVSGPRLVQPHGPRFRLEGNAVLYGGWSFAFRLRSSSGLQVLNVHFGGERIAYEVSVQEAVALYGGHTPAGMQTKYLDVGWGLGSVTHELAPGIDCPETATFLDTFHYYDADDPVHYPRALCLFEMPTGVPLRRHFNSNFKGGFNFYAGLKGQVLVLRTTSTVYNYDYIWDFIFYPNGVMEAKMHATGYVHATFYTPEGLRHGTRLHTHLIGNIHTHLVHYRVDLDVAGTKNSFQTLQMKLENITNPWSPRHRVVQPTLEQTQYSWERQAAFSFKRKLPTYLLFTSPQENPWGHKRSYRLQIHSMADQVLPPGWQEEQAITWARYPLAVTKYRESELCSSSIYHQNDPWHPPVVFEQFLHNNENIENEDLVAWVTVGFLHIPHSEDIPNTATPGNSVGFLLRPFNFFPEDPSLASRDTVIVWPRDNGPNYVQRWIPEDRDCSMPPPFSYNGTYRPV

SEQ ID NO: 9 - protein, 751 aa, Artificial Sequence
  hDAO-Cysmut
MPALGWAVAAILMLQTAMAEPSPGTLPRKAGVFSDLSNQELKAVHSFLWSKKELRLQPSSTTTMAKNTVFLIEMLLPKKYHVLRFLDKGERHPVREARAVIFFGDQEHPNVTEFAVGPLPGPAYMRALSPRPGYQSSWASRPISTAEYALLYHTLQEATKPLHQFFLNTTGFSFQDCHDRCLAFTDVAPRGVASGQRRSWLIIQRYVEGYFLHPTGLELLVDHGSTDAGHWAVEQVWYNGKFYGSPEELARKYADGEVDVVVLEDPLPGGKGHDSTEEPPLFSSHKPRGDFPSPIHVSGPRLVQPHGPRFRLEGNAVLYGGWSFAFRLRSSSGLQVLNVHFGGERIAYEVSVQEAVALYGGHTPAGMQTKYLDVGWGLGSVTHELAPGIDCPETATFLDTFHYYDADDPVHYPRALCLFEMPTGVPLRRHFNSNFKGGFNFYAGLKGQVLVLRTTSTVYNYDYIWDFIFYPNGVMEAKMHATGYVHATFYTPEGLRHGTRLHTHLIGNIHTHLVHYRVDLDVAGTKNSFQTLQMKLENITNPWSPRHRVVQPTLEQTQYSWERQAAFRFKRKLPKYLLFTSPQENPWGHKRSYRLQIHSMADQVLPPGWQEEQAITWARYPLAVTKYRESELCSSSIYHQNDPWHPPVVFEQFLHNNENIENEDLVAWVTVGFLHIPHSEDIPNTATPGNSVGFLLRPFNFFPEDPSLASRDTVIVWPRDNGPNYVQRWIPEDRDCSMPPPFSYNGTYRPV

SEQ ID NO: 10 - protein, 751 aa, Artificial Sequence
  hDAO-Hepmut1-Cysmut
MPALGWAVAAILMLQTAMAEPSPGTLPRKAGVFSDLSNQELKAVHSFLWSKKELRLQPSSTTTMAKNTVFLIEMLLPKKYHVLRFLDKGERHPVREARAVIFFGDQEHPNVTEFAVGPLPGPAYMRALSPRPGYQSSWASRPISTAEYALLYHTLQEATKPLHQFFLNTTGFSFQDCHDRCLAFTDVAPRGVASGQRRSWLIIQRYVEGYFLHPTGLELLVDHGSTDAGHWAVEQVWYNGKFYGSPEELARKYADGEVDVVVLEDPLPGGKGHDSTEEPPLFSSHKPRGDFPSPIHVSGPRLVQPHGPRFRLEGNAVLYGGWSFAFRLRSSSGLQVLNVHFGGERIAYEVSVQEAVALYGGHTPAGMQTKYLDVGWGLGSVTHELAPGIDCPETATFLDTFHYYDADDPVHYPRALCLFEMPTGVPLRRHFNSNFKGGFNFYAGLKGQVLVLRTTSTVYNYDYIWDFIFYPNGVMEAKMHATGYVHATFYTPEGLRHGTRLHTHLIGNIHTHLVHYRVDLDVAGTKNSFQTLQMKLENITNPWSPRHRVVQPTLEQTQYSWERQAAFSFKRKLPKYLLFTSPQENPWGHKRSYRLQIHSMADQVLPPGWQEEQAITWARYPLAVTKYRESELCSSSIYHQNDPWHPPVVFEQFLHNNENIENEDLVAWVTVGFLHIPHSEDIPNTATPGNSVGFLLRPFNFFPEDPSLASRDTVIVWPRDNGPNYVQRWIPEDRDCSMPPPFSYNGTYRPV

SEQ ID NO: 11 - protein, 751 aa, Artificial Sequence
  hDAO-Hepmut2-Cysmut
MPALGWAVAAILMLQTAMAEPSPGTLPRKAGVFSDLSNQELKAVHSFLWSKKELRLQPSSTTTMAKNTVFLIEMLLPKKYHVLRFLDKGERHPVREARAVIFFGDQEHPNVTEFAVGPLPGPAYMRALSPRPGYQSSWASRPISTAEYALLYHTLQEATKPLHQFFLNTTGFSFQDCHDRCLAFTDVAPRGVASGQRRSWLIIQRYVEGYFLHPTGLELLVDHGSTDAGHWAVEQVWYNGKFYGSPEELARKYADGEVDVVVLEDPLPGGKGHDSTEEPPLFSSHKPRGDFPSPIHVSGPRLVQPHGPRFRLEGNAVLYGGWSFAFRLRSSSGLQVLNVHFGGERIAYEVSVQEAVALYGGHTPAGMQTKYLDVGWGLGSVTHELAPGIDCPETATFLDTFHYYDADDPVHYPRALCLFEMPTGVPLRRHFNSNFKGGFNFYAGLKGQVLVLRTTSTVYNYDYIWDFIFYPNGVMEAKMHATGYVHATFYTPEGLRHGTRLHTHLIGNIHTHLVHYRVDLDVAGTKNSFQTLQMKLENITNPWSPRHRVVQPTLEQTQYSWERQAAFRFKRKLPTYLLFTSPQENPWGHKRSYRLQIHSMADQVLPPGWQEEQAITWARYPLAVTKYRESELCSSSIYHQNDPWHPPVVFEQFLHNNENIENEDLVAWVTVGFLHIPHSEDIPNTATPGNSVGFLLRPFNFFPEDPSLASRDTVIVWPRDNGPNYVQRWIPEDRDCSMPPPFSYNGTYRPV

SEQ ID NO: 12 - protein, 751 aa, Artificial Sequence
  hDAO-Hepmut3-Cysmut
MPALGWAVAAILMLQTAMAEPSPGTLPRKAGVFSDLSNQELKAVHSFLWSKKELRLQPSSTTTMAKNTVFLIEMLLPKKYHVLRFLDKGERHPVREARAVIFFGDQEHPNVTEFAVGPLPGPAYMRALSPRPGYQSSWASRPISTAEYALLYHTLQEATKPLHQFFLNTTGFSFQDCHDRCLAFTDVAPRGVASGQRRSWLIIQRYVEGYFLHPTGLELLVDHGSTDAGHWAVEQVWYNGKFYGSPEELARKYADGEVDVVVLEDPLPGGKGHDSTEEPPLFSSHKPRGDFPSPIHVSGPRLVQPHGPRFRLEGNAVLYGGWSFAFRLRSSSGLQVLNVHFGGERIAYEVSVQEAVALYGGHTPAGMQTKYLDVGWGLGSVTHELAPGIDCPETATFLDTFHYYDADDPVHYPRALCLFEMPTGVPLRRHFNSNFKGGFNFYAGLKGQVLVLRTTSTVYNYDYIWDFIFYPNGVMEAKMHATGYVHATFYTPEGLRHGTRLHTHLIGNIHTHLVHYRVDLDVAGTKNSFQTLQMKLENITNPWSPRHRVVQPTLEQTQYSWERQAAFRFKTKLPKYLLFTSPQENPWGHKRSYRLQIHSMADQVLPPGWQEEQAITWARYPLAVTKYRESELCSSSIYHQNDPWHPPVVFEQFLHNNENIENEDLVAWVTVGFLHIPHSEDIPNTATPGNSVGFLLRPFNFFPEDPSLASRDTVIVWPRDNGPNYVQRWIPEDRDCSMPPPFSYNGTYRPV

SEQ ID NO: 13 - protein, 751 aa, Artificial Sequence
  hDAO-Hepmut4-Cysmut
MPALGWAVAAILMLQTAMAEPSPGTLPRKAGVFSDLSNQELKAVHSFLWSKKELRLQPSSTTTMAKNTVFLIEMLLPKKYHVLRFLDKGERHPVREARAVIFFGDQEHPNVTEFAVGPLPGPAYMRALSPRPGYQSSWASRPISTAEYALLYHTLQEATKPLHQFFLNTTGFSFQDCHDRCLAFTDVAPRGVASGQRRSWLIIQRYVEGYFLHPTGLELLVDHGSTDAGHWAVEQVWYNGKFYGSPEELARKYADGEVDVVVLEDPLPGGKGHDSTEEPPLFSSHKPRGDFPSPIHVSGPRLVQPHGPRFRLEGNAVLYGGWSFAFRLRSSSGLQVLNVHFGGERIAYEVSVQEAVALYGGHTPAGMQTKYLDVGWGLGSVTHELAPGIDCPETATFLDTFHYYDADDPVHYPRALCLFEMPTGVPLRRHFNSNFKGGFNFYAGLKGQVLVLRTTSTVYNYDYIWDFIFYPNGVMEAKMHATGYVHATFYTPEGLRHGTRLHTHLIGNIHTHLVHYRVDLDVAGTKNSFQTLQMKLENITNPWSPRHRVVQPTLEQTQYSWERQAAFSFKTKLPKYLLFTSPQENPWGHKRSYRLQIHSMADQVLPPGWQEEQAITWARYPLAVTKYRESELCSSSIYHQNDPWHPPVVFEQFLHNNENIENEDLVAWVTVGFLHIPHSEDIPNTATPGNSVGFLLRPFNFFPEDPSLASRDTVIVWPRDNGPNYVQRWIPEDRDCSMPPPFSYNGTYRPV

SEQ ID NO: 14 - protein, 751 aa, Artificial Sequence
  hDAO-Hepmut5-Cysmut
MPALGWAVAAILMLQTAMAEPSPGTLPRKAGVFSDLSNQELKAVHSFLWSKKELRLQPSSTTTMAKNTVFLIEMLLPKKYHVLRFLDKGERHPVREARAVIFFGDQEHPNVTEFAVGPLPGPAYMRALSPRPGYQSSWASRPISTAEYALLYHTLQEATKPLHQFFLNTTGFSFQDCHDRCLAFTDVAPRGVASGQRRSWLIIQRYVEGYFLHPTGLELLVDHGSTDAGHWAVEQVWYNGKFYGSPEELARKYADGEVDVVVLEDPLPGGKGHDSTEEPPLFSSHKPRGDFPSPIHVSGPRLVQPHGPRFRLEGNAVLYGGWSFAFRLRSSSGLQVLNVHFGGERIAYEVSVQEAVALYGGHTPAGMQTKYLDVGWGLGSVTHELAPGIDCPETATFLDTFHYYDADDPVHYPRALCLFEMPTGVPLRRHFNSNFKGGFNFYAGLKGQVLVLRTTSTVYNYDYIWDFIFYPNGVMEAKMHATGYVHATFYTPEGLRHGTRLHTHLIGNIHTHLVHYRVDLDVAGTKNSFQTLQMKLENITNPWSPRHRVVQPTLEQTQYSWERQAAFRFKTKLPTYLLFTSPQENPWGHKRSYRLQIHSMADQVLPPGWQEEQAITWARYPLAVTKYRESELCSSSIYHQNDPWHPPVVFEQFLHNNENIENEDLVAWVTVGFLHIPHSEDIPNTATPGNSVGFLLRPFNFFPEDPSLASRDTVIVWPRDNGPNYVQRWIPEDRDCSMPPPFSYNGTYRPV

SEQ ID NO: 15 - protein, 751 aa, Artificial Sequence
  hDAO-Hepmut6-Cysmut
MPALGWAVAAILMLQTAMAEPSPGTLPRKAGVFSDLSNQELKAVHSFLWSKKELRLQPSSTTTMAKNTVFLIEMLLPKKYHVLRFLDKGERHPVREARAVIFFGDQEHPNVTEFAVGPLPGPAYMRALSPRPGYQSSWASRPISTAEYALLYHTLQEATKPLHQFFLNTTGFSFQDCHDRCLAFTDVAPRGVASGQRRSWLIIQRYVEGYFLHPTGLELLVDHGSTDAGHWAVEQVWYNGKFYGSPEELARKYADGEVDVVVLEDPLPGGKGHDSTEEPPLFSSHKPRGDFPSPIHVSGPRLVQPHGPRFRLEGNAVLYGGWSFAFRLRSSSGLQVLNVHFGGERIAYEVSVQEAVALYGGHTPAGMQTKYLDVGWGLGSVTHELAPGIDCPETATFLDTFHYYDADDPVHYPRALCLFEMPTGVPLRRHFNSNFKGGFNFYAGLKGQVLVLRTTSTVYNYDYIWDFIFYPNGVMEAKMHATGYVHATFYTPEGLRHGTRLHTHLIGNIHTHLVHYRVDLDVAGTKNSFQTLQMKLENITNPWSPRHRVVQPTLEQTQYSWERQAAFRFGQTLPKYLLFTSPQENPWGHKRSYRLQIHSMADQVLPPGWQEEQAITWARYPLAVTKYRESELCSSSIYHQNDPWHPPVVFEQFLHNNENIENEDLVAWVTVGFLHIPHSEDIPNTATPGNSVGFLLRPFNFFPEDPSLASRDTVIVWPRDNGPNYVQRWIPEDRDCSMPPPFSYNGTYRPV

SEQ ID NO: 16 - protein, 751 aa, Artificial Sequence
  hDAO-Hepmut7-Cysmut
MPALGWAVAAILMLQTAMAEPSPGTLPRKAGVFSDLSNQELKAVHSFLWSKKELRLQPSSTTTMAKNTVFLIEMLLPKKYHVLRFLDKGERHPVREARAVIFFGDQEHPNVTEFAVGPLPGPAYMRALSPRPGYQSSWASRPISTAEYALLYHTLQEATKPLHQFFLNTTGFSFQDCHDRCLAFTDVAPRGVASGQRRSWLIIQRYVEGYFLHPTGLELLVDHGSTDAGHWAVEQVWYNGKFYGSPEELARKYADGEVDVVVLEDPLPGGKGHDSTEEPPLFSSHKPRGDFPSPIHVSGPRLVQPHGPRFRLEGNAVLYGGWSFAFRLRSSSGLQVLNVHFGGERIAYEVSVQEAVALYGGHTPAGMQTKYLDVGWGLGSVTHELAPGIDCPETATFLDTFHYYDADDPVHYPRALCLFEMPTGVPLRRHFNSNFKGGFNFYAGLKGQVLVLRTTSTVYNYDYIWDFIFYPNGVMEAKMHATGYVHATFYTPEGLRHGTRLHTHLIGNIHTHLVHYRVDLDVAGTKNSFQTLQMKLENITNPWSPRHRVVQPTLEQTQYSWERQAAFSFKRKLPTYLLFTSPQENPWGHKRSYRLQIHSMADQVLPPGWQEEQAITWARYPLAVTKYRESELCSSSIYHQNDPWHPPVVFEQFLHNNENIENEDLVAWVTVGFLHIPHSEDIPNTATPGNSVGFLLRPFNFFPEDPSLASRDTVIVWPRDNGPNYVQRWIPEDRDCSMPPPFSYNGTYRPV

SEQ ID NO: 17 - DNA, 2256 bp, Homo sapiens
atgccggccctgggctgggccgtggctgccatcctgatgctgcagacggccatggcggagccctccccggggactctgcccaggaaggcaggggtgttttcagacctaagcaaccaagagctgaaggcagtgcacagcttcctctggtccaagaaggagctgaggctgcagccctccagtaccaccaccatggccaagaacaccgtgtttctcatcgagatgctgctgcccaagaagtaccatgtgctgaggtttctggataaaggtgaaaggcatcctgtgcgggaagcccgtgccgtcatcttctttggtgaccaggagcatcccaatgtcaccgagtttgctgtggggcccctgccagggccctgctacatgcgagcactgtcccccaggcctgggtaccagtcctcctgggcatcgaggcccatctccacagcagagtatgccctcctctaccacaccctgcaggaagccaccaagcccctgcatcagttcttcctcaataccacaggcttctcattccaagactgccatgacagatgcctggccttcaccgatgtggccccccggggtgtggcttctggccagcgccgcagttggcttatcatacagcgctatgtagaaggctactttctgcaccccactgggctggagctcctcgtggatcatgggagcacagatgctgggcactgggccgtggagcaggtgtggtacaacgggaagttctatgggagcccagaggaactggctcggaagtatgcagatggagaggtggacgtggtggtcctggaggacccgctgcctgggggcaaggggcatgacagcacagaggagccgcccctcttctcctcccacaagccccgcggggacttccccagccccatccatgtgagcggcccccgcttggtccagccccacggccctcgcttcaggctggagggcaacgctgtgctctacggcggctggagctttgccttccggctgcgctcctcctccgggctgcaggtcctgaacgtgcacttcggcggagagcgcattgcctatgaggtcagcgtgcaagaggcagtggcgctgtatggaggacacacacctgcaggcatgcagaccaagtacctcgatgtcggctggggcctgggcagcgtcactcatgagttagcccccggcatcgactgcccggagaccgccaccttcctggacactttccactactatgatgccgatgacccggtccattatccccgagccctctgcctctttgaaatgcccacaggggtgccccttcggcggcactttaattccaactttaaaggtggcttcaacttctatgcggggctgaagggccaggtgctggtgctgcggacaacttcaactgtctacaattatgattacatttgggactttatcttctaccccaacggggtgatggaggccaagatgcatgccactggctacgtccacgccaccttctacacccccgaggggctgcgccacggcactcgcctgcacacccacctgattggcaacatacacactcacttggtgcactaccgcgtagacctggatgtggcaggcaccaagaacagcttccagacactgcagatgaagctagaaaacatcaccaacccctggagcccaagacaccgcgtggtccagccaactctggagcagacgcagtactcctgggagcgccaggcggccttccgcttcaaaaggaagctgcccaagtacctgctctttaccagcccccaggagaacccctggggccacaagcgcagctaccgcctgcagatccactccatggccgaccaggtgctgcccccaggctggcaggaggagcaggccatcacctgggcaaggtaccccctggcagtgaccaagtaccgggagtcggagctgtgcagcagcagcatctaccaccagaacgacccctggcacccgcccgtggtctttgagcagtttcttcacaacaacgagaacattgaaaatgaggacctggtggcctgggtgacggtgggcttcctgcacatcccccactcagaggacattcccaacacagccacacctgggaactccgtgggcttcctgctccggccattcaacttcttcccagaggacccctccctggcatccagagacactgtgatcgtgtggcctcgggacaacggccccaactacgtccagcgctggatccctgaggacagggactgctcgatgcctcccccttttagctacaatgggacctatagacctgtgtga

SEQ ID NO: 18 - DNA, 2256 bp, Artificial Sequence
  hDAO-Hepmut1
atgccggccctgggctgggccgtggctgccatcctgatgctgcagacggccatggcggagccctccccggggactctgcccaggaaggcaggggtgttttcagacctaagcaaccaagagctgaaggcagtgcacagcttcctctggtccaagaaggagctgaggctgcagccctccagtaccaccaccatggccaagaacaccgtgtttctcatcgagatgctgctgcccaagaagtaccatgtgctgaggtttctggataaaggtgaaaggcatcctgtgcgggaagcccgtgccgtcatcttctttggtgaccaggagcatcccaatgtcaccgagtttgctgtggggcccctgccagggccctgctacatgcgagcactgtcccccaggcctgggtaccagtcctcctgggcatcgaggcccatctccacagcagagtatgccctcctctaccacaccctgcaggaagccaccaagcccctgcatcagttcttcctcaataccacaggcttctcattccaagactgccatgacagatgcctggccttcaccgatgtggccccccggggtgtggcttctggccagcgccgcagttggcttatcatacagcgctatgtagaaggctactttctgcaccccactgggctggagctcctcgtggatcatgggagcacagatgctgggcactgggccgtggagcaggtgtggtacaacgggaagttctatgggagcccagaggaactggctcggaagtatgcagatggagaggtggacgtggtggtcctggaggacccgctgcctgggggcaaggggcatgacagcacagaggagccgcccctcttctcctcccacaagccccgcggggacttccccagccccatccatgtgagcggcccccgcttggtccagccccacggccctcgcttcaggctggagggcaacgctgtgctctacggcggctggagctttgccttccggctgcgctcctcctccgggctgcaggtcctgaacgtgcacttcggcggagagcgcattgcctatgaggtcagcgtgcaagaggcagtggcgctgtatggaggacacacacctgcaggcatgcagaccaagtacctcgatgtcggctggggcctgggcagcgtcactcatgagttagcccccggcatcgactgcccggagaccgccaccttcctggacactttccactactatgatgccgatgacccggtccattatccccgagccctctgcctctttgaaatgcccacaggggtgccccttcggcggcactttaattccaactttaaaggtggcttcaacttctatgcggggctgaagggccaggtgctggtgctgcggacaacttcaactgtctacaattatgattacatttgggactttatcttctaccccaacggggtgatggaggccaagatgcatgccactggctacgtccacgccaccttctacacccccgaggggctgcgccacggcactcgcctgcacacccacctgattggcaacatacacactcacttggtgcactaccgcgtagacctggatgtggcaggcaccaagaacagcttccagacactgcagatgaagctagaaaacatcaccaacccctggagcccaagacaccgcgtggtccagccaactctggagcagacgcagtactcctgggagcgccaggcggccttcagcttcaaaaggaagctgcccaagtacctgctctttaccagcccccaggagaacccctggggccacaagcgcagctaccgcctgcagatccactccatggccgaccaggtgctgcccccaggctggcaggaggagcaggccatcacctgggcaaggtaccccctggcagtgaccaagtaccgggagtcggagctgtgcagcagcagcatctaccaccagaacgacccctggcacccgcccgtggtctttgagcagtttcttcacaacaacgagaacattgaaaatgaggacctggtggcctgggtgacggtgggcttcctgcacatcccccactcagaggacattcccaacacagccacacctgggaactccgtgggcttcctgctccggccattcaacttcttcccagaggacccctccctggcatccagagacactgtgatcgtgtggcctcgggacaacggccccaactacgtccagcgctggatccctgaggacagggactgctcgatgcctcccccttttagctacaatgggacctatagacctgtgtga

SEQ ID NO: 19 - DNA, 2256 bp, Artificial Sequence
  hDAO-Hepmut2
atgccggccctgggctgggccgtggctgccatcctgatgctgcagacggccatggcggagccctccccggggactctgcccaggaaggcaggggtgttttcagacctaagcaaccaagagctgaaggcagtgcacagcttcctctggtccaagaaggagctgaggctgcagccctccagtaccaccaccatggccaagaacaccgtgtttctcatcgagatgctgctgcccaagaagtaccatgtgctgaggtttctggataaaggtgaaaggcatcctgtgcgggaagcccgtgccgtcatcttctttggtgaccaggagcatcccaatgtcaccgagtttgctgtggggcccctgccagggccctgctacatgcgagcactgtcccccaggcctgggtaccagtcctcctgggcatcgaggcccatctccacagcagagtatgccctcctctaccacaccctgcaggaagccaccaagcccctgcatcagttcttcctcaataccacaggcttctcattccaagactgccatgacagatgcctggccttcaccgatgtggccccccggggtgtggcttctggccagcgccgcagttggcttatcatacagcgctatgtagaaggctactttctgcaccccactgggctggagctcctcgtggatcatgggagcacagatgctgggcactgggccgtggagcaggtgtggtacaacgggaagttctatgggagcccagaggaactggctcggaagtatgcagatggagaggtggacgtggtggtcctggaggacccgctgcctgggggcaaggggcatgacagcacagaggagccgcccctcttctcctcccacaagccccgcggggacttccccagccccatccatgtgagcggcccccgcttggtccagccccacggccctcgcttcaggctggagggcaacgctgtgctctacggcggctggagctttgccttccggctgcgctcctcctccgggctgcaggtcctgaacgtgcacttcggcggagagcgcattgcctatgaggtcagcgtgcaagaggcagtggcgctgtatggaggacacacacctgcaggcatgcagaccaagtacctcgatgtcggctggggcctgggcagcgtcactcatgagttagcccccggcatcgactgcccggagaccgccaccttcctggacactttccactactatgatgccgatgacccggtccattatccccgagccctctgcctctttgaaatgcccacaggggtgccccttcggcggcactttaattccaactttaaaggtggcttcaacttctatgcggggctgaagggccaggtgctggtgctgcggacaacttcaactgtctacaattatgattacatttgggactttatcttctaccccaacggggtgatggaggccaagatgcatgccactggctacgtccacgccaccttctacacccccgaggggctgcgccacggcactcgcctgcacacccacctgattggcaacatacacactcacttggtgcactaccgcgtagacctggatgtggcaggcaccaagaacagcttccagacactgcagatgaagctagaaaacatcaccaacccctggagcccaagacaccgcgtggtccagccaactctggagcagacgcagtactcctgggagcgccaggcggccttccgcttcaaaaggaagctgcccacgtacctgctctttaccagcccccaggagaacccctggggccacaagcgcagctaccgcctgcagatccactccatggccgaccaggtgctgcccccaggctggcaggaggagcaggccatcacctgggcaaggtaccccctggcagtgaccaagtaccgggagtcggagctgtgcagcagcagcatctaccaccagaacgacccctggcacccgcccgtggtctttgagcagtttcttcacaacaacgagaacattgaaaatgaggacctggtggcctgggtgacggtgggcttcctgcacatcccccactcagaggacattcccaacacagccacacctgggaactccgtgggcttcctgctccggccattcaacttcttcccagaggacccctccctggcatccagagacactgtgatcgtgtggcctcgggacaacggccccaactacgtccagcgctggatccctgaggacagggactgctcgatgcctcccccttttagctacaatgggacctatagacctgtgtga

SEQ ID NO: 20 - DNA, 2256 bp, Artificial Sequence
  hDAO-Hepmut3
atgccggccctgggctgggccgtggctgccatcctgatgctgcagacggccatggcggagccctccccggggactctgcccaggaaggcaggggtgttttcagacctaagcaaccaagagctgaaggcagtgcacagcttcctctggtccaagaaggagctgaggctgcagccctccagtaccaccaccatggccaagaacaccgtgtttctcatcgagatgctgctgcccaagaagtaccatgtgctgaggtttctggataaaggtgaaaggcatcctgtgcgggaagcccgtgccgtcatcttctttggtgaccaggagcatcccaatgtcaccgagtttgctgtggggcccctgccagggccctgctacatgcgagcactgtcccccaggcctgggtaccagtcctcctgggcatcgaggcccatctccacagcagagtatgccctcctctaccacaccctgcaggaagccaccaagcccctgcatcagttcttcctcaataccacaggcttctcattccaagactgccatgacagatgcctggccttcaccgatgtggccccccggggtgtggcttctggccagcgccgcagttggcttatcatacagcgctatgtagaaggctactttctgcaccccactgggctggagctcctcgtggatcatgggagcacagatgctgggcactgggccgtggagcaggtgtggtacaacgggaagttctatgggagcccagaggaactggctcggaagtatgcagatggagaggtggacgtggtggtcctggaggacccgctgcctgggggcaaggggcatgacagcacagaggagccgcccctcttctcctcccacaagccccgcggggacttccccagccccatccatgtgagcggcccccgcttggtccagccccacggccctcgcttcaggctggagggcaacgctgtgctctacggcggctggagctttgccttccggctgcgctcctcctccgggctgcaggtcctgaacgtgcacttcggcggagagcgcattgcctatgaggtcagcgtgcaagaggcagtggcgctgtatggaggacacacacctgcaggcatgcagaccaagtacctcgatgtcggctggggcctgggcagcgtcactcatgagttagcccccggcatcgactgcccggagaccgccaccttcctggacactttccactactatgatgccgatgacccggtccattatccccgagccctctgcctctttgaaatgcccacaggggtgccccttcggcggcactttaattccaactttaaaggtggcttcaacttctatgcggggctgaagggccaggtgctggtgctgcggacaacttcaactgtctacaattatgattacatttgggactttatcttctaccccaacggggtgatggaggccaagatgcatgccactggctacgtccacgccaccttctacacccccgaggggctgcgccacggcactcgcctgcacacccacctgattggcaacatacacactcacttggtgcactaccgcgtagacctggatgtggcaggcaccaagaacagcttccagacactgcagatgaagctagaaaacatcaccaacccctggagcccaagacaccgcgtggtccagccaactctggagcagacgcagtactcctgggagcgccaggcggccttccgcttcaaaacgaagctgcccaagtacctgctctttaccagcccccaggagaacccctggggccacaagcgcagctaccgcctgcagatccactccatggccgaccaggtgctgcccccaggctggcaggaggagcaggccatcacctgggcaaggtaccccctggcagtgaccaagtaccgggagtcggagctgtgcagcagcagcatctaccaccagaacgacccctggcacccgcccgtggtctttgagcagtttcttcacaacaacgagaacattgaaaatgaggacctggtggcctgggtgacggtgggcttcctgcacatcccccactcagaggacattcccaacacagccacacctgggaactccgtgggcttcctgctccggccattcaacttcttcccagaggacccctccctggcatccagagacactgtgatcgtgtggcctcgggacaacggccccaactacgtccagcgctggatccctgaggacagggactgctcgatgcctcccccttttagctacaatgggacctatagacctgtgtga

SEQ ID NO: 21 - DNA, 2256 bp, Artificial Sequence
  hDAO-Hepmut4
atgccggccctgggctgggccgtggctgccatcctgatgctgcagacggccatggcggagccctccccggggactctgcccaggaaggcaggggtgttttcagacctaagcaaccaagagctgaaggcagtgcacagcttcctctggtccaagaaggagctgaggctgcagccctccagtaccaccaccatggccaagaacaccgtgtttctcatcgagatgctgctgcccaagaagtaccatgtgctgaggtttctggataaaggtgaaaggcatcctgtgcgggaagcccgtgccgtcatcttctttggtgaccaggagcatcccaatgtcaccgagtttgctgtggggcccctgccagggccctgctacatgcgagcactgtcccccaggcctgggtaccagtcctcctgggcatcgaggcccatctccacagcagagtatgccctcctctaccacaccctgcaggaagccaccaagcccctgcatcagttcttcctcaataccacaggcttctcattccaagactgccatgacagatgcctggccttcaccgatgtggccccccggggtgtggcttctggccagcgccgcagttggcttatcatacagcgctatgtagaaggctactttctgcaccccactgggctggagctcctcgtggatcatgggagcacagatgctgggcactgggccgtggagcaggtgtggtacaacgggaagttctatgggagcccagaggaactggctcggaagtatgcagatggagaggtggacgtggtggtcctggaggacccgctgcctgggggcaaggggcatgacagcacagaggagccgcccctcttctcctcccacaagccccgcggggacttccccagccccatccatgtgagcggcccccgcttggtccagccccacggccctcgcttcaggctggagggcaacgctgtgctctacggcggctggagctttgccttccggctgcgctcctcctccgggctgcaggtcctgaacgtgcacttcggcggagagcgcattgcctatgaggtcagcgtgcaagaggcagtggcgctgtatggaggacacacacctgcaggcatgcagaccaagtacctcgatgtcggctggggcctgggcagcgtcactcatgagttagcccccggcatcgactgcccggagaccgccaccttcctggacactttccactactatgatgccgatgacccggtccattatccccgagccctctgcctctttgaaatgcccacaggggtgccccttcggcggcactttaattccaactttaaaggtggcttcaacttctatgcggggctgaagggccaggtgctggtgctgcggacaacttcaactgtctacaattatgattacatttgggactttatcttctaccccaacggggtgatggaggccaagatgcatgccactggctacgtccacgccaccttctacacccccgaggggctgcgccacggcactcgcctgcacacccacctgattggcaacatacacactcacttggtgcactaccgcgtagacctggatgtggcaggcaccaagaacagcttccagacactgcagatgaagctagaaaacatcaccaacccctggagcccaagacaccgcgtggtccagccaactctggagcagacgcagtactcctgggagcgccaggcggccttcagcttcaaaacgaagctgcccaagtacctgctctttaccagcccccaggagaacccctggggccacaagcgcagctaccgcctgcagatccactccatggccgaccaggtgctgcccccaggctggcaggaggagcaggccatcacctgggcaaggtaccccctggcagtgaccaagtaccgggagtcggagctgtgcagcagcagcatctaccaccagaacgacccctggcacccgcccgtggtctttgagcagtttcttcacaacaacgagaacattgaaaatgaggacctggtggcctgggtgacggtgggcttcctgcacatcccccactcagaggacattcccaacacagccacacctgggaactccgtgggcttcctgctccggccattcaacttcttcccagaggacccctccctggcatccagagacactgtgatcgtgtggcctcgggacaacggccccaactacgtccagcgctggatccctgaggacagggactgctcgatgcctcccccttttagctacaatgggacctatagacctgtgtga

SEQ ID NO: 22 - DNA, 2256 bp, Artificial Sequence
  hDAO-Hepmut5
atgccggccctgggctgggccgtggctgccatcctgatgctgcagacggccatggcggagccctccccggggactctgcccaggaaggcaggggtgttttcagacctaagcaaccaagagctgaaggcagtgcacagcttcctctggtccaagaaggagctgaggctgcagccctccagtaccaccaccatggccaagaacaccgtgtttctcatcgagatgctgctgcccaagaagtaccatgtgctgaggtttctggataaaggtgaaaggcatcctgtgcgggaagcccgtgccgtcatcttctttggtgaccaggagcatcccaatgtcaccgagtttgctgtggggcccctgccagggccctgctacatgcgagcactgtcccccaggcctgggtaccagtcctcctgggcatcgaggcccatctccacagcagagtatgccctcctctaccacaccctgcaggaagccaccaagcccctgcatcagttcttcctcaataccacaggcttctcattccaagactgccatgacagatgcctggccttcaccgatgtggccccccggggtgtggcttctggccagcgccgcagttggcttatcatacagcgctatgtagaaggctactttctgcaccccactgggctggagctcctcgtggatcatgggagcacagatgctgggcactgggccgtggagcaggtgtggtacaacgggaagttctatgggagcccagaggaactggctcggaagtatgcagatggagaggtggacgtggtggtcctggaggacccgctgcctgggggcaaggggcatgacagcacagaggagccgcccctcttctcctcccacaagccccgcggggacttccccagccccatccatgtgagcggcccccgcttggtccagccccacggccctcgcttcaggctggagggcaacgctgtgctctacggcggctggagctttgccttccggctgcgctcctcctccgggctgcaggtcctgaacgtgcacttcggcggagagcgcattgcctatgaggtcagcgtgcaagaggcagtggcgctgtatggaggacacacacctgcaggcatgcagaccaagtacctcgatgtcggctggggcctgggcagcgtcactcatgagttagcccccggcatcgactgcccggagaccgccaccttcctggacactttccactactatgatgccgatgacccggtccattatccccgagccctctgcctctttgaaatgcccacaggggtgccccttcggcggcactttaattccaactttaaaggtggcttcaacttctatgcggggctgaagggccaggtgctggtgctgcggacaacttcaactgtctacaattatgattacatttgggactttatcttctaccccaacggggtgatggaggccaagatgcatgccactggctacgtccacgccaccttctacacccccgaggggctgcgccacggcactcgcctgcacacccacctgattggcaacatacacactcacttggtgcactaccgcgtagacctggatgtggcaggcaccaagaacagcttccagacactgcagatgaagctagaaaacatcaccaacccctggagcccaagacaccgcgtggtccagccaactctggagcagacgcagtactcctgggagcgccaggcggccttccgcttcaaaacgaagctgcccacgtacctgctctttaccagcccccaggagaacccctggggccacaagcgcagctaccgcctgcagatccactccatggccgaccaggtgctgcccccaggctggcaggaggagcaggccatcacctgggcaaggtaccccctggcagtgaccaagtaccgggagtcggagctgtgcagcagcagcatctaccaccagaacgacccctggcacccgcccgtggtctttgagcagtttcttcacaacaacgagaacattgaaaatgaggacctggtggcctgggtgacggtgggcttcctgcacatcccccactcagaggacattcccaacacagccacacctgggaactccgtgggcttcctgctccggccattcaacttcttcccagaggacccctccctggcatccagagacactgtgatcgtgtggcctcgggacaacggccccaactacgtccagcgctggatccctgaggacagggactgctcgatgcctcccccttttagctacaatgggacctatagacctgtgtga

SEQ ID NO: 23 - DNA, 2256 bp, Artificial Sequence
  hDAO-Hepmut6
atgccggccctgggctgggccgtggctgccatcctgatgctgcagacggccatggcggagccctccccggggactctgcccaggaaggcaggggtgttttcagacctaagcaaccaagagctgaaggcagtgcacagcttcctctggtccaagaaggagctgaggctgcagccctccagtaccaccaccatggccaagaacaccgtgtttctcatcgagatgctgctgcccaagaagtaccatgtgctgaggtttctggataaaggtgaaaggcatcctgtgcgggaagcccgtgccgtcatcttctttggtgaccaggagcatcccaatgtcaccgagtttgctgtggggcccctgccagggccctgctacatgcgagcactgtcccccaggcctgggtaccagtcctcctgggcatcgaggcccatctccacagcagagtatgccctcctctaccacaccctgcaggaagccaccaagcccctgcatcagttcttcctcaataccacaggcttctcattccaagactgccatgacagatgcctggccttcaccgatgtggccccccggggtgtggcttctggccagcgccgcagttggcttatcatacagcgctatgtagaaggctactttctgcaccccactgggctggagctcctcgtggatcatgggagcacagatgctgggcactgggccgtggagcaggtgtggtacaacgggaagttctatgggagcccagaggaactggctcggaagtatgcagatggagaggtggacgtggtggtcctggaggacccgctgcctgggggcaaggggcatgacagcacagaggagccgcccctcttctcctcccacaagccccgcggggacttccccagccccatccatgtgagcggcccccgcttggtccagccccacggccctcgcttcaggctggagggcaacgctgtgctctacggcggctggagctttgccttccggctgcgctcctcctccgggctgcaggtcctgaacgtgcacttcggcggagagcgcattgcctatgaggtcagcgtgcaagaggcagtggcgctgtatggaggacacacacctgcaggcatgcagaccaagtacctcgatgtcggctggggcctgggcagcgtcactcatgagttagcccccggcatcgactgcccggagaccgccaccttcctggacactttccactactatgatgccgatgacccggtccattatccccgagccctctgcctctttgaaatgcccacaggggtgccccttcggcggcactttaattccaactttaaaggtggcttcaacttctatgcggggctgaagggccaggtgctggtgctgcggacaacttcaactgtctacaattatgattacatttgggactttatcttctaccccaacggggtgatggaggccaagatgcatgccactggctacgtccacgccaccttctacacccccgaggggctgcgccacggcactcgcctgcacacccacctgattggcaacatacacactcacttggtgcactaccgcgtagacctggatgtggcaggcaccaagaacagcttccagacactgcagatgaagctagaaaacatcaccaacccctggagcccaagacaccgcgtggtccagccaactctggagcagacgcagtactcctgggagcgccaggcggccttccgcttcggacagacgctgcccaagtacctgctctttaccagcccccaggagaacccctggggccacaagcgcagctaccgcctgcagatccactccatggccgaccaggtgctgcccccaggctggcaggaggagcaggccatcacctgggcaaggtaccccctggcagtgaccaagtaccgggagtcggagctgtgcagcagcagcatctaccaccagaacgacccctggcacccgcccgtggtctttgagcagtttcttcacaacaacgagaacattgaaaatgaggacctggtggcctgggtgacggtgggcttcctgcacatcccccactcagaggacattcccaacacagccacacctgggaactccgtgggcttcctgctccggccattcaacttcttcccagaggacccctccctggcatccagagacactgtgatcgtgtggcctcgggacaacggccccaactacgtccagcgctggatccctgaggacagggactgctcgatgcctcccccttttagctacaatgggacctatagacctgtgtga

SEQ ID NO: 24 - DNA, 2256 bp, Artificial Sequence
  hDAO-Hepmut7
atgccggccctgggctgggccgtggctgccatcctgatgctgcagacggccatggcggagccctccccggggactctgcccaggaaggcaggggtgttttcagacctaagcaaccaagagctgaaggcagtgcacagcttcctctggtccaagaaggagctgaggctgcagccctccagtaccaccaccatggccaagaacaccgtgtttctcatcgagatgctgctgcccaagaagtaccatgtgctgaggtttctggataaaggtgaaaggcatcctgtgcgggaagcccgtgccgtcatcttctttggtgaccaggagcatcccaatgtcaccgagtttgctgtggggcccctgccagggccctgctacatgcgagcactgtcccccaggcctgggtaccagtcctcctgggcatcgaggcccatctccacagcagagtatgccctcctctaccacaccctgcaggaagccaccaagcccctgcatcagttcttcctcaataccacaggcttctcattccaagactgccatgacagatgcctggccttcaccgatgtggccccccggggtgtggcttctggccagcgccgcagttggcttatcatacagcgctatgtagaaggctactttctgcaccccactgggctggagctcctcgtggatcatgggagcacagatgctgggcactgggccgtggagcaggtgtggtacaacgggaagttctatgggagcccagaggaactggctcggaagtatgcagatggagaggtggacgtggtggtcctggaggacccgctgcctgggggcaaggggcatgacagcacagaggagccgcccctcttctcctcccacaagccccgcggggacttccccagccccatccatgtgagcggcccccgcttggtccagccccacggccctcgcttcaggctggagggcaacgctgtgctctacggcggctggagctttgccttccggctgcgctcctcctccgggctgcaggtcctgaacgtgcacttcggcggagagcgcattgcctatgaggtcagcgtgcaagaggcagtggcgctgtatggaggacacacacctgcaggcatgcagaccaagtacctcgatgtcggctggggcctgggcagcgtcactcatgagttagcccccggcatcgactgcccggagaccgccaccttcctggacactttccactactatgatgccgatgacccggtccattatccccgagccctctgcctctttgaaatgcccacaggggtgccccttcggcggcactttaattccaactttaaaggtggcttcaacttctatgcggggctgaagggccaggtgctggtgctgcggacaacttcaactgtctacaattatgattacatttgggactttatcttctaccccaacggggtgatggaggccaagatgcatgccactggctacgtccacgccaccttctacacccccgaggggctgcgccacggcactcgcctgcacacccacctgattggcaacatacacactcacttggtgcactaccgcgtagacctggatgtggcaggcaccaagaacagcttccagacactgcagatgaagctagaaaacatcaccaacccctggagcccaagacaccgcgtggtccagccaactctggagcagacgcagtactcctgggagcgccaggcggccttcagcttcaaaaggaagctgcccacgtacctgctctttaccagcccccaggagaacccctggggccacaagcgcagctaccgcctgcagatccactccatggccgaccaggtgctgcccccaggctggcaggaggagcaggccatcacctgggcaaggtaccccctggcagtgaccaagtaccgggagtcggagctgtgcagcagcagcatctaccaccagaacgacccctggcacccgcccgtggtctttgagcagtttcttcacaacaacgagaacattgaaaatgaggacctggtggcctgggtgacggtgggcttcctgcacatcccccactcagaggacattcccaacacagccacacctgggaactccgtgggcttcctgctccggccattcaacttcttcccagaggacccctccctggcatccagagacactgtgatcgtgtggcctcgggacaacggccccaactacgtccagcgctggatccctgaggacagggactgctcgatgcctcccccttttagctacaatgggacctatagacctgtgtga

SEQ ID NO: 25 - DNA, 2256 bp, Artificial Sequence
  hDAO-Cysmut
atgccggccctgggctgggccgtggctgccatcctgatgctgcagacggccatggcggagccctccccggggactctgcccaggaaggcaggggtgttttcagacctaagcaaccaagagctgaaggcagtgcacagcttcctctggtccaagaaggagctgaggctgcagccctccagtaccaccaccatggccaagaacaccgtgtttctcatcgagatgctgctgcccaagaagtaccatgtgctgaggtttctggataaaggtgaaaggcatcctgtgcgggaagcccgtgccgtcatcttctttggtgaccaggagcatcccaatgtcaccgagtttgctgtggggcccctgccagggcccgcctacatgcgagcactgtcccccaggcctgggtaccagtcctcctgggcatcgaggcccatctccacagcagagtatgccctcctctaccacaccctgcaggaagccaccaagcccctgcatcagttcttcctcaataccacaggcttctcattccaagactgccatgacagatgcctggccttcaccgatgtggccccccggggtgtggcttctggccagcgccgcagttggcttatcatacagcgctatgtagaaggctactttctgcaccccactgggctggagctcctcgtggatcatgggagcacagatgctgggcactgggccgtggagcaggtgtggtacaacgggaagttctatgggagcccagaggaactggctcggaagtatgcagatggagaggtggacgtggtggtcctggaggacccgctgcctgggggcaaggggcatgacagcacagaggagccgcccctcttctcctcccacaagccccgcggggacttccccagccccatccatgtgagcggcccccgcttggtccagccccacggccctcgcttcaggctggagggcaacgctgtgctctacggcggctggagctttgccttccggctgcgctcctcctccgggctgcaggtcctgaacgtgcacttcggcggagagcgcattgcctatgaggtcagcgtgcaagaggcagtggcgctgtatggaggacacacacctgcaggcatgcagaccaagtacctcgatgtcggctggggcctgggcagcgtcactcatgagttagcccccggcatcgactgcccggagaccgccaccttcctggacactttccactactatgatgccgatgacccggtccattatccccgagccctctgcctctttgaaatgcccacaggggtgccccttcggcggcactttaattccaactttaaaggtggcttcaacttctatgcggggctgaagggccaggtgctggtgctgcggacaacttcaactgtctacaattatgattacatttgggactttatcttctaccccaacggggtgatggaggccaagatgcatgccactggctacgtccacgccaccttctacacccccgaggggctgcgccacggcactcgcctgcacacccacctgattggcaacatacacactcacttggtgcactaccgcgtagacctggatgtggcaggcaccaagaacagcttccagacactgcagatgaagctagaaaacatcaccaacccctggagcccaagacaccgcgtggtccagccaactctggagcagacgcagtactcctgggagcgccaggcggccttccgcttcaaaaggaagctgcccaagtacctgctctttaccagcccccaggagaacccctggggccacaagcgcagctaccgcctgcagatccactccatggccgaccaggtgctgcccccaggctggcaggaggagcaggccatcacctgggcaaggtaccccctggcagtgaccaagtaccgggagtcggagctgtgcagcagcagcatctaccaccagaacgacccctggcacccgcccgtggtctttgagcagtttcttcacaacaacgagaacattgaaaatgaggacctggtggcctgggtgacggtgggcttcctgcacatcccccactcagaggacattcccaacacagccacacctgggaactccgtgggcttcctgctccggccattcaacttcttcccagaggacccctccctggcatccagagacactgtgatcgtgtggcctcgggacaacggccccaactacgtccagcgctggatccctgaggacagggactgctcgatgcctcccccttttagctacaatgggacctatagacctgtgtga

SEQ ID NO: 26 - DNA, 2256 bp, Artificial Sequence
  hDAO-Hepmut1-Cysmut
atgccggccctgggctgggccgtggctgccatcctgatgctgcagacggccatggcggagccctccccggggactctgcccaggaaggcaggggtgttttcagacctaagcaaccaagagctgaaggcagtgcacagcttcctctggtccaagaaggagctgaggctgcagccctccagtaccaccaccatggccaagaacaccgtgtttctcatcgagatgctgctgcccaagaagtaccatgtgctgaggtttctggataaaggtgaaaggcatcctgtgcgggaagcccgtgccgtcatcttctttggtgaccaggagcatcccaatgtcaccgagtttgctgtggggcccctgccagggcccgcctacatgcgagcactgtcccccaggcctgggtaccagtcctcctgggcatcgaggcccatctccacagcagagtatgccctcctctaccacaccctgcaggaagccaccaagcccctgcatcagttcttcctcaataccacaggcttctcattccaagactgccatgacagatgcctggccttcaccgatgtggccccccggggtgtggcttctggccagcgccgcagttggcttatcatacagcgctatgtagaaggctactttctgcaccccactgggctggagctcctcgtggatcatgggagcacagatgctgggcactgggccgtggagcaggtgtggtacaacgggaagttctatgggagcccagaggaactggctcggaagtatgcagatggagaggtggacgtggtggtcctggaggacccgctgcctgggggcaaggggcatgacagcacagaggagccgcccctcttctcctcccacaagccccgcggggacttccccagccccatccatgtgagcggcccccgcttggtccagccccacggccctcgcttcaggctggagggcaacgctgtgctctacggcggctggagctttgccttccggctgcgctcctcctccgggctgcaggtcctgaacgtgcacttcggcggagagcgcattgcctatgaggtcagcgtgcaagaggcagtggcgctgtatggaggacacacacctgcaggcatgcagaccaagtacctcgatgtcggctggggcctgggcagcgtcactcatgagttagcccccggcatcgactgcccggagaccgccaccttcctggacactttccactactatgatgccgatgacccggtccattatccccgagccctctgcctctttgaaatgcccacaggggtgccccttcggcggcactttaattccaactttaaaggtggcttcaacttctatgcggggctgaagggccaggtgctggtgctgcggacaacttcaactgtctacaattatgattacatttgggactttatcttctaccccaacggggtgatggaggccaagatgcatgccactggctacgtccacgccaccttctacacccccgaggggctgcgccacggcactcgcctgcacacccacctgattggcaacatacacactcacttggtgcactaccgcgtagacctggatgtggcaggcaccaagaacagcttccagacactgcagatgaagctagaaaacatcaccaacccctggagcccaagacaccgcgtggtccagccaactctggagcagacgcagtactcctgggagcgccaggcggccttcagcttcaaaaggaagctgcccaagtacctgctctttaccagcccccaggagaacccctggggccacaagcgcagctaccgcctgcagatccactccatggccgaccaggtgctgcccccaggctggcaggaggagcaggccatcacctgggcaaggtaccccctggcagtgaccaagtaccgggagtcggagctgtgcagcagcagcatctaccaccagaacgacccctggcacccgcccgtggtctttgagcagtttcttcacaacaacgagaacattgaaaatgaggacctggtggcctgggtgacggtgggcttcctgcacatcccccactcagaggacattcccaacacagccacacctgggaactccgtgggcttcctgctccggccattcaacttcttcccagaggacccctccctggcatccagagacactgtgatcgtgtggcctcgggacaacggccccaactacgtccagcgctggatccctgaggacagggactgctcgatgcctcccccttttagctacaatgggacctatagacctgtgtga

SEQ ID NO: 27 - DNA, 2256 bp, Artificial Sequence
  hDAO-Hepmut2-Cysmut
atgccggccctgggctgggccgtggctgccatcctgatgctgcagacggccatggcggagccctccccggggactctgcccaggaaggcaggggtgttttcagacctaagcaaccaagagctgaaggcagtgcacagcttcctctggtccaagaaggagctgaggctgcagccctccagtaccaccaccatggccaagaacaccgtgtttctcatcgagatgctgctgcccaagaagtaccatgtgctgaggtttctggataaaggtgaaaggcatcctgtgcgggaagcccgtgccgtcatcttctttggtgaccaggagcatcccaatgtcaccgagtttgctgtggggcccctgccagggcccgcctacatgcgagcactgtcccccaggcctgggtaccagtcctcctgggcatcgaggcccatctccacagcagagtatgccctcctctaccacaccctgcaggaagccaccaagcccctgcatcagttcttcctcaataccacaggcttctcattccaagactgccatgacagatgcctggccttcaccgatgtggccccccggggtgtggcttctggccagcgccgcagttggcttatcatacagcgctatgtagaaggctactttctgcaccccactgggctggagctcctcgtggatcatgggagcacagatgctgggcactgggccgtggagcaggtgtggtacaacgggaagttctatgggagcccagaggaactggctcggaagtatgcagatggagaggtggacgtggtggtcctggaggacccgctgcctgggggcaaggggcatgacagcacagaggagccgcccctcttctcctcccacaagccccgcggggacttccccagccccatccatgtgagcggcccccgcttggtccagccccacggccctcgcttcaggctggagggcaacgctgtgctctacggcggctggagctttgccttccggctgcgctcctcctccgggctgcaggtcctgaacgtgcacttcggcggagagcgcattgcctatgaggtcagcgtgcaagaggcagtggcgctgtatggaggacacacacctgcaggcatgcagaccaagtacctcgatgtcggctggggcctgggcagcgtcactcatgagttagcccccggcatcgactgcccggagaccgccaccttcctggacactttccactactatgatgccgatgacccggtccattatccccgagccctctgcctctttgaaatgcccacaggggtgccccttcggcggcactttaattccaactttaaaggtggcttcaacttctatgcggggctgaagggccaggtgctggtgctgcggacaacttcaactgtctacaattatgattacatttgggactttatcttctaccccaacggggtgatggaggccaagatgcatgccactggctacgtccacgccaccttctacacccccgaggggctgcgccacggcactcgcctgcacacccacctgattggcaacatacacactcacttggtgcactaccgcgtagacctggatgtggcaggcaccaagaacagcttccagacactgcagatgaagctagaaaacatcaccaacccctggagcccaagacaccgcgtggtccagccaactctggagcagacgcagtactcctgggagcgccaggcggccttccgcttcaaaaggaagctgcccacgtacctgctctttaccagcccccaggagaacccctggggccacaagcgcagctaccgcctgcagatccactccatggccgaccaggtgctgcccccaggctggcaggaggagcaggccatcacctgggcaaggtaccccctggcagtgaccaagtaccgggagtcggagctgtgcagcagcagcatctaccaccagaacgacccctggcacccgcccgtggtctttgagcagtttcttcacaacaacgagaacattgaaaatgaggacctggtggcctgggtgacggtgggcttcctgcacatcccccactcagaggacattcccaacacagccacacctgggaactccgtgggcttcctgctccggccattcaacttcttcccagaggacccctccctggcatccagagacactgtgatcgtgtggcctcgggacaacggccccaactacgtccagcgctggatccctgaggacagggactgctcgatgcctcccccttttagctacaatgggacctatagacctgtgtga

SEQ ID NO: 28 - DNA, 2256 bp, Artificial Sequence
  hDAO-Hepmut3-Cysmut
atgccggccctgggctgggccgtggctgccatcctgatgctgcagacggccatggcggagccctccccggggactctgcccaggaaggcaggggtgttttcagacctaagcaaccaagagctgaaggcagtgcacagcttcctctggtccaagaaggagctgaggctgcagccctccagtaccaccaccatggccaagaacaccgtgtttctcatcgagatgctgctgcccaagaagtaccatgtgctgaggtttctggataaaggtgaaaggcatcctgtgcgggaagcccgtgccgtcatcttctttggtgaccaggagcatcccaatgtcaccgagtttgctgtggggcccctgccagggcccgcctacatgcgagcactgtcccccaggcctgggtaccagtcctcctgggcatcgaggcccatctccacagcagagtatgccctcctctaccacaccctgcaggaagccaccaagcccctgcatcagttcttcctcaataccacaggcttctcattccaagactgccatgacagatgcctggccttcaccgatgtggccccccggggtgtggcttctggccagcgccgcagttggcttatcatacagcgctatgtagaaggctactttctgcaccccactgggctggagctcctcgtggatcatgggagcacagatgctgggcactgggccgtggagcaggtgtggtacaacgggaagttctatgggagcccagaggaactggctcggaagtatgcagatggagaggtggacgtggtggtcctggaggacccgctgcctgggggcaaggggcatgacagcacagaggagccgcccctcttctcctcccacaagccccgcggggacttccccagccccatccatgtgagcggcccccgcttggtccagccccacggccctcgcttcaggctggagggcaacgctgtgctctacggcggctggagctttgccttccggctgcgctcctcctccgggctgcaggtcctgaacgtgcacttcggcggagagcgcattgcctatgaggtcagcgtgcaagaggcagtggcgctgtatggaggacacacacctgcaggcatgcagaccaagtacctcgatgtcggctggggcctgggcagcgtcactcatgagttagcccccggcatcgactgcccggagaccgccaccttcctggacactttccactactatgatgccgatgacccggtccattatccccgagccctctgcctctttgaaatgcccacaggggtgccccttcggcggcactttaattccaactttaaaggtggcttcaacttctatgcggggctgaagggccaggtgctggtgctgcggacaacttcaactgtctacaattatgattacatttgggactttatcttctaccccaacggggtgatggaggccaagatgcatgccactggctacgtccacgccaccttctacacccccgaggggctgcgccacggcactcgcctgcacacccacctgattggcaacatacacactcacttggtgcactaccgcgtagacctggatgtggcaggcaccaagaacagcttccagacactgcagatgaagctagaaaacatcaccaacccctggagcccaagacaccgcgtggtccagccaactctggagcagacgcagtactcctgggagcgccaggcggccttccgcttcaaaacgaagctgcccaagtacctgctctttaccagcccccaggagaacccctggggccacaagcgcagctaccgcctgcagatccactccatggccgaccaggtgctgcccccaggctggcaggaggagcaggccatcacctgggcaaggtaccccctggcagtgaccaagtaccgggagtcggagctgtgcagcagcagcatctaccaccagaacgacccctggcacccgcccgtggtctttgagcagtttcttcacaacaacgagaacattgaaaatgaggacctggtggcctgggtgacggtgggcttcctgcacatcccccactcagaggacattcccaacacagccacacctgggaactccgtgggcttcctgctccggccattcaacttcttcccagaggacccctccctggcatccagagacactgtgatcgtgtggcctcgggacaacggccccaactacgtccagcgctggatccctgaggacagggactgctcgatgcctcccccttttagctacaatgggacctatagacctgtgtga

SEQ ID NO: 29 - DNA, 2256 bp, Artificial Sequence
  hDAO-Hepmut4-Cysmut
atgccggccctgggctgggccgtggctgccatcctgatgctgcagacggccatggcggagccctccccggggactctgcccaggaaggcaggggtgttttcagacctaagcaaccaagagctgaaggcagtgcacagcttcctctggtccaagaaggagctgaggctgcagccctccagtaccaccaccatggccaagaacaccgtgtttctcatcgagatgctgctgcccaagaagtaccatgtgctgaggtttctggataaaggtgaaaggcatcctgtgcgggaagcccgtgccgtcatcttctttggtgaccaggagcatcccaatgtcaccgagtttgctgtggggcccctgccagggcccgcctacatgcgagcactgtcccccaggcctgggtaccagtcctcctgggcatcgaggcccatctccacagcagagtatgccctcctctaccacaccctgcaggaagccaccaagcccctgcatcagttcttcctcaataccacaggcttctcattccaagactgccatgacagatgcctggccttcaccgatgtggccccccggggtgtggcttctggccagcgccgcagttggcttatcatacagcgctatgtagaaggctactttctgcaccccactgggctggagctcctcgtggatcatgggagcacagatgctgggcactgggccgtggagcaggtgtggtacaacgggaagttctatgggagcccagaggaactggctcggaagtatgcagatggagaggtggacgtggtggtcctggaggacccgctgcctgggggcaaggggcatgacagcacagaggagccgcccctcttctcctcccacaagccccgcggggacttccccagccccatccatgtgagcggcccccgcttggtccagccccacggccctcgcttcaggctggagggcaacgctgtgctctacggcggctggagctttgccttccggctgcgctcctcctccgggctgcaggtcctgaacgtgcacttcggcggagagcgcattgcctatgaggtcagcgtgcaagaggcagtggcgctgtatggaggacacacacctgcaggcatgcagaccaagtacctcgatgtcggctggggcctgggcagcgtcactcatgagttagcccccggcatcgactgcccggagaccgccaccttcctggacactttccactactatgatgccgatgacccggtccattatccccgagccctctgcctctttgaaatgcccacaggggtgccccttcggcggcactttaattccaactttaaaggtggcttcaacttctatgcggggctgaagggccaggtgctggtgctgcggacaacttcaactgtctacaattatgattacatttgggactttatcttctaccccaacggggtgatggaggccaagatgcatgccactggctacgtccacgccaccttctacacccccgaggggctgcgccacggcactcgcctgcacacccacctgattggcaacatacacactcacttggtgcactaccgcgtagacctggatgtggcaggcaccaagaacagcttccagacactgcagatgaagctagaaaacatcaccaacccctggagcccaagacaccgcgtggtccagccaactctggagcagacgcagtactcctgggagcgccaggcggccttcagcttcaaaacgaagctgcccaagtacctgctctttaccagcccccaggagaacccctggggccacaagcgcagctaccgcctgcagatccactccatggccgaccaggtgctgcccccaggctggcaggaggagcaggccatcacctgggcaaggtaccccctggcagtgaccaagtaccgggagtcggagctgtgcagcagcagcatctaccaccagaacgacccctggcacccgcccgtggtctttgagcagtttcttcacaacaacgagaacattgaaaatgaggacctggtggcctgggtgacggtgggcttcctgcacatcccccactcagaggacattcccaacacagccacacctgggaactccgtgggcttcctgctccggccattcaacttcttcccagaggacccctccctggcatccagagacactgtgatcgtgtggcctcgggacaacggccccaactacgtccagcgctggatccctgaggacagggactgctcgatgcctcccccttttagctacaatgggacctatagacctgtgtga

SEQ ID NO: 30 - DNA, 2256 bp, Artificial Sequence
  hDAO-Hepmut5-Cysmut
atgccggccctgggctgggccgtggctgccatcctgatgctgcagacggccatggcggagccctccccggggactctgcccaggaaggcaggggtgttttcagacctaagcaaccaagagctgaaggcagtgcacagcttcctctggtccaagaaggagctgaggctgcagccctccagtaccaccaccatggccaagaacaccgtgtttctcatcgagatgctgctgcccaagaagtaccatgtgctgaggtttctggataaaggtgaaaggcatcctgtgcgggaagcccgtgccgtcatcttctttggtgaccaggagcatcccaatgtcaccgagtttgctgtggggcccctgccagggcccgcctacatgcgagcactgtcccccaggcctgggtaccagtcctcctgggcatcgaggcccatctccacagcagagtatgccctcctctaccacaccctgcaggaagccaccaagcccctgcatcagttcttcctcaataccacaggcttctcattccaagactgccatgacagatgcctggccttcaccgatgtggccccccggggtgtggcttctggccagcgccgcagttggcttatcatacagcgctatgtagaaggctactttctgcaccccactgggctggagctcctcgtggatcatgggagcacagatgctgggcactgggccgtggagcaggtgtggtacaacgggaagttctatgggagcccagaggaactggctcggaagtatgcagatggagaggtggacgtggtggtcctggaggacccgctgcctgggggcaaggggcatgacagcacagaggagccgcccctcttctcctcccacaagccccgcggggacttccccagccccatccatgtgagcggcccccgcttggtccagccccacggccctcgcttcaggctggagggcaacgctgtgctctacggcggctggagctttgccttccggctgcgctcctcctccgggctgcaggtcctgaacgtgcacttcggcggagagcgcattgcctatgaggtcagcgtgcaagaggcagtggcgctgtatggaggacacacacctgcaggcatgcagaccaagtacctcgatgtcggctggggcctgggcagcgtcactcatgagttagcccccggcatcgactgcccggagaccgccaccttcctggacactttccactactatgatgccgatgacccggtccattatccccgagccctctgcctctttgaaatgcccacaggggtgccccttcggcggcactttaattccaactttaaaggtggcttcaacttctatgcggggctgaagggccaggtgctggtgctgcggacaacttcaactgtctacaattatgattacatttgggactttatcttctaccccaacggggtgatggaggccaagatgcatgccactggctacgtccacgccaccttctacacccccgaggggctgcgccacggcactcgcctgcacacccacctgattggcaacatacacactcacttggtgcactaccgcgtagacctggatgtggcaggcaccaagaacagcttccagacactgcagatgaagctagaaaacatcaccaacccctggagcccaagacaccgcgtggtccagccaactctggagcagacgcagtactcctgggagcgccaggcggccttccgcttcaaaacgaagctgcccacgtacctgctctttaccagcccccaggagaacccctggggccacaagcgcagctaccgcctgcagatccactccatggccgaccaggtgctgcccccaggctggcaggaggagcaggccatcacctgggcaaggtaccccctggcagtgaccaagtaccgggagtcggagctgtgcagcagcagcatctaccaccagaacgacccctggcacccgcccgtggtctttgagcagtttcttcacaacaacgagaacattgaaaatgaggacctggtggcctgggtgacggtgggcttcctgcacatcccccactcagaggacattcccaacacagccacacctgggaactccgtgggcttcctgctccggccattcaacttcttcccagaggacccctccctggcatccagagacactgtgatcgtgtggcctcgggacaacggccccaactacgtccagcgctggatccctgaggacagggactgctcgatgcctcccccttttagctacaatgggacctatagacctgtgtga

SEQ ID NO: 31 - DNA, 2256 bp, Artificial Sequence
  hDAO-Hepmut6-Cysmut
atgccggccctgggctgggccgtggctgccatcctgatgctgcagacggccatggcggagccctccccggggactctgcccaggaaggcaggggtgttttcagacctaagcaaccaagagctgaaggcagtgcacagcttcctctggtccaagaaggagctgaggctgcagccctccagtaccaccaccatggccaagaacaccgtgtttctcatcgagatgctgctgcccaagaagtaccatgtgctgaggtttctggataaaggtgaaaggcatcctgtgcgggaagcccgtgccgtcatcttctttggtgaccaggagcatcccaatgtcaccgagtttgctgtggggcccctgccagggcccgcctacatgcgagcactgtcccccaggcctgggtaccagtcctcctgggcatcgaggcccatctccacagcagagtatgccctcctctaccacaccctgcaggaagccaccaagcccctgcatcagttcttcctcaataccacaggcttctcattccaagactgccatgacagatgcctggccttcaccgatgtggccccccggggtgtggcttctggccagcgccgcagttggcttatcatacagcgctatgtagaaggctactttctgcaccccactgggctggagctcctcgtggatcatgggagcacagatgctgggcactgggccgtggagcaggtgtggtacaacgggaagttctatgggagcccagaggaactggctcggaagtatgcagatggagaggtggacgtggtggtcctggaggacccgctgcctgggggcaaggggcatgacagcacagaggagccgcccctcttctcctcccacaagccccgcggggacttccccagccccatccatgtgagcggcccccgcttggtccagccccacggccctcgcttcaggctggagggcaacgctgtgctctacggcggctggagctttgccttccggctgcgctcctcctccgggctgcaggtcctgaacgtgcacttcggcggagagcgcattgcctatgaggtcagcgtgcaagaggcagtggcgctgtatggaggacacacacctgcaggcatgcagaccaagtacctcgatgtcggctggggcctgggcagcgtcactcatgagttagcccccggcatcgactgcccggagaccgccaccttcctggacactttccactactatgatgccgatgacccggtccattatccccgagccctctgcctctttgaaatgcccacaggggtgccccttcggcggcactttaattccaactttaaaggtggcttcaacttctatgcggggctgaagggccaggtgctggtgctgcggacaacttcaactgtctacaattatgattacatttgggactttatcttctaccccaacggggtgatggaggccaagatgcatgccactggctacgtccacgccaccttctacacccccgaggggctgcgccacggcactcgcctgcacacccacctgattggcaacatacacactcacttggtgcactaccgcgtagacctggatgtggcaggcaccaagaacagcttccagacactgcagatgaagctagaaaacatcaccaacccctggagcccaagacaccgcgtggtccagccaactctggagcagacgcagtactcctgggagcgccaggcggccttccgcttcggacagacgctgcccaagtacctgctctttaccagcccccaggagaacccctggggccacaagcgcagctaccgcctgcagatccactccatggccgaccaggtgctgcccccaggctggcaggaggagcaggccatcacctgggcaaggtaccccctggcagtgaccaagtaccgggagtcggagctgtgcagcagcagcatctaccaccagaacgacccctggcacccgcccgtggtctttgagcagtttcttcacaacaacgagaacattgaaaatgaggacctggtggcctgggtgacggtgggcttcctgcacatcccccactcagaggacattcccaacacagccacacctgggaactccgtgggcttcctgctccggccattcaacttcttcccagaggacccctccctggcatccagagacactgtgatcgtgtggcctcgggacaacggccccaactacgtccagcgctggatccctgaggacagggactgctcgatgcctcccccttttagctacaatgggacctatagacctgtgtga

SEQ ID NO: 32 - DNA, 2256 bp, Artificial Sequence
  hDAO-Hepmut7-Cysmut
atgccggccctgggctgggccgtggctgccatcctgatgctgcagacggccatggcggagccctccccggggactctgcccaggaaggcaggggtgttttcagacctaagcaaccaagagctgaaggcagtgcacagcttcctctggtccaagaaggagctgaggctgcagccctccagtaccaccaccatggccaagaacaccgtgtttctcatcgagatgctgctgcccaagaagtaccatgtgctgaggtttctggataaaggtgaaaggcatcctgtgcgggaagcccgtgccgtcatcttctttggtgaccaggagcatcccaatgtcaccgagtttgctgtggggcccctgccagggcccgcctacatgcgagcactgtcccccaggcctgggtaccagtcctcctgggcatcgaggcccatctccacagcagagtatgccctcctctaccacaccctgcaggaagccaccaagcccctgcatcagttcttcctcaataccacaggcttctcattccaagactgccatgacagatgcctggccttcaccgatgtggccccccggggtgtggcttctggccagcgccgcagttggcttatcatacagcgctatgtagaaggctactttctgcaccccactgggctggagctcctcgtggatcatgggagcacagatgctgggcactgggccgtggagcaggtgtggtacaacgggaagttctatgggagcccagaggaactggctcggaagtatgcagatggagaggtggacgtggtggtcctggaggacccgctgcctgggggcaaggggcatgacagcacagaggagccgcccctcttctcctcccacaagccccgcggggacttccccagccccatccatgtgagcggcccccgcttggtccagccccacggccctcgcttcaggctggagggcaacgctgtgctctacggcggctggagctttgccttccggctgcgctcctcctccgggctgcaggtcctgaacgtgcacttcggcggagagcgcattgcctatgaggtcagcgtgcaagaggcagtggcgctgtatggaggacacacacctgcaggcatgcagaccaagtacctcgatgtcggctggggcctgggcagcgtcactcatgagttagcccccggcatcgactgcccggagaccgccaccttcctggacactttccactactatgatgccgatgacccggtccattatccccgagccctctgcctctttgaaatgcccacaggggtgccccttcggcggcactttaattccaactttaaaggtggcttcaacttctatgcggggctgaagggccaggtgctggtgctgcggacaacttcaactgtctacaattatgattacatttgggactttatcttctaccccaacggggtgatggaggccaagatgcatgccactggctacgtccacgccaccttctacacccccgaggggctgcgccacggcactcgcctgcacacccacctgattggcaacatacacactcacttggtgcactaccgcgtagacctggatgtggcaggcaccaagaacagcttccagacactgcagatgaagctagaaaacatcaccaacccctggagcccaagacaccgcgtggtccagccaactctggagcagacgcagtactcctgggagcgccaggcggccttcagcttcaaaaggaagctgcccacgtacctgctctttaccagcccccaggagaacccctggggccacaagcgcagctaccgcctgcagatccactccatggccgaccaggtgctgcccccaggctggcaggaggagcaggccatcacctgggcaaggtaccccctggcagtgaccaagtaccgggagtcggagctgtgcagcagcagcatctaccaccagaacgacccctggcacccgcccgtggtctttgagcagtttcttcacaacaacgagaacattgaaaatgaggacctggtggcctgggtgacggtgggcttcctgcacatcccccactcagaggacattcccaacacagccacacctgggaactccgtgggcttcctgctccggccattcaacttcttcccagaggacccctccctggcatccagagacactgtgatcgtgtggcctcgggacaacggccccaactacgtccagcgctggatccctgaggacagggactgctcgatgcctcccccttttagctacaatgggacctatagacctgtgtga

SEQ ID NO: 33 - protein, 8 aa, Artificial Sequence
  DAO polypeptide
SFKAKLPK

SEQ ID NO: 34 - protein, 8 aa, Artificial Sequence
  DAO polypeptide
AFKAKLPT

SEQ ID NO: 35 - protein, 8 aa, Artificial Sequence
  DAO polypeptide
AFKTKLPK

SEQ ID NO: 36 - protein, 8 aa, Artificial Sequence
  DAO polypeptide
SFKTKLPK

SEQ ID NO: 37 - protein, 8 aa, Artificial Sequence
  DAO polypeptide
AFKTKLPT

SEQ ID NO: 38 - protein, 8 aa, Artificial Sequence
  DAO polypeptide
SFKAKLPK

SEQ ID NO: 39 - protein, 983 aa, Artificial Sequence
  Fc-hDAO
MPALGWAVAAILMLQTAMAECPPCPAPPVAGPSVFLFPPKPKDTLMISRTPEVTCVVVDVSHEDPEVKFNWYVDGVEVHNAKTKPREEQYNSTYRVVSVLTVLHQDWLNGKEYKCKVSNKGLPSSIEKTISKAKGQPREPQVYTLPPSREEMTKNQVSLTCLVKGFYPSDIAVEWESNGQPENNYKTTPPVLDSDGSFFLYSKLTVDKSRWQQGNVFSCSVMHEALHNHYTQKSLSLSPGKEPKSADKTHTEPSPGTLPRKAGVFSDLSNQELKAVHSFLWSKKELRLQPSSTTTMAKNTVFLIEMLLPKKYHVLRFLDKGERHPVREARAVIFFGDQEHPNVTEFAVGPLPGPCYMRALSPRPGYQSSWASRPISTAEYALLYHTLQEATKPLHQFFLNTTGFSFQDCHDRCLAFTDVAPRGVASGQRRSWLIIQRYVEGYFLHPTGLELLVDHGSTDAGHWAVEQVWYNGKFYGSPEELARKYADGEVDVVVLEDPLPGGKGHDSTEEPPLFSSHKPRGDFPSPIHVSGPRLVQPHGPRFRLEGNAVLYGGWSFAFRLRSSSGLQVLNVHFGGERIAYEVSVQEAVALYGGHTPAGMQTKYLDVGWGLGSVTHELAPGIDCPETATFLDTFHYYDADDPVHYPRALCLFEMPTGVPLRRHFNSNFKGGFNFYAGLKGQVLVLRTTSTVYNYDYIWDFIFYPNGVMEAKMHATGYVHATFYTPEGLRHGTRLHTHLIGNIHTHLVHYRVDLDVAGTKNSFQTLQMKLENITNPWSPRHRVVQPTLEQTQYSWERQAAFRFKRKLPKYLLFTSPQENPWGHKRSYRLQIHSMADQVLPPGWQEEQAITWARYPLAVTKYRESELCSSSIYHQNDPWHPPVVFEQFLHNNENIENEDLVAWVTVGFLHIPHSEDIPNTATPGNSVGFLLRPFNFFPEDPSLASRDTVIVWPRDNGPNYVQRWIPEDRDCSMPPPFSYNGTYRPV

SEQ ID NO: 40 - protein, 983 aa, Artificial Sequence
  Fc-hDAO-Hepmut1
MPALGWAVAAILMLQTAMAECPPCPAPPVAGPSVFLFPPKPKDTLMISRTPEVTCVVVDVSHEDPEVKFNWYVDGVEVHNAKTKPREEQYNSTYRVVSVLTVLHQDWLNGKEYKCKVSNKGLPSSIEKTISKAKGQPREPQVYTLPPSREEMTKNQVSLTCLVKGFYPSDIAVEWESNGQPENNYKTTPPVLDSDGSFFLYSKLTVDKSRWQQGNVFSCSVMHEALHNHYTQKSLSLSPGKEPKSADKTHTEPSPGTLPRKAGVFSDLSNQELKAVHSFLWSKKELRLQPSSTTTMAKNTVFLIEMLLPKKYHVLRFLDKGERHPVREARAVIFFGDQEHPNVTEFAVGPLPGPCYMRALSPRPGYQSSWASRPISTAEYALLYHTLQEATKPLHQFFLNTTGFSFQDCHDRCLAFTDVAPRGVASGQRRSWLIIQRYVEGYFLHPTGLELLVDHGSTDAGHWAVEQVWYNGKFYGSPEELARKYADGEVDVVVLEDPLPGGKGHDSTEEPPLFSSHKPRGDFPSPIHVSGPRLVQPHGPRFRLEGNAVLYGGWSFAFRLRSSSGLQVLNVHFGGERIAYEVSVQEAVALYGGHTPAGMQTKYLDVGWGLGSVTHELAPGIDCPETATFLDTFHYYDADDPVHYPRALCLFEMPTGVPLRRHFNSNFKGGFNFYAGLKGQVLVLRTTSTVYNYDYIWDFIFYPNGVMEAKMHATGYVHATFYTPEGLRHGTRLHTHLIGNIHTHLVHYRVDLDVAGTKNSFQTLQMKLENITNPWSPRHRVVQPTLEQTQYSWERQAAFSFKRKLPKYLLFTSPQENPWGHKRSYRLQIHSMADQVLPPGWQEEQAITWARYPLAVTKYRESELCSSSIYHQNDPWHPPVVFEQFLHNNENIENEDLVAWVTVGFLHIPHSEDIPNTATPGNSVGFLLRPFNFFPEDPSLASRDTVIVWPRDNGPNYVQRWIPEDRDCSMPPPFSYNGTYRPV

SEQ ID NO: 41 - protein, 983 aa, Artificial Sequence
  Fc-hDAO-Hepmut2
MPALGWAVAAILMLQTAMAECPPCPAPPVAGPSVFLFPPKPKDTLMISRTPEVTCVVVDVSHEDPEVKFNWYVDGVEVHNAKTKPREEQYNSTYRVVSVLTVLHQDWLNGKEYKCKVSNKGLPSSIEKTISKAKGQPREPQVYTLPPSREEMTKNQVSLTCLVKGFYPSDIAVEWESNGQPENNYKTTPPVLDSDGSFFLYSKLTVDKSRWQQGNVFSCSVMHEALHNHYTQKSLSLSPGKEPKSADKTHTEPSPGTLPRKAGVFSDLSNQELKAVHSFLWSKKELRLQPSSTTTMAKNTVFLIEMLLPKKYHVLRFLDKGERHPVREARAVIFFGDQEHPNVTEFAVGPLPGPCYMRALSPRPGYQSSWASRPISTAEYALLYHTLQEATKPLHQFFLNTTGFSFQDCHDRCLAFTDVAPRGVASGQRRSWLIIQRYVEGYFLHPTGLELLVDHGSTDAGHWAVEQVWYNGKFYGSPEELARKYADGEVDVVVLEDPLPGGKGHDSTEEPPLFSSHKPRGDFPSPIHVSGPRLVQPHGPRFRLEGNAVLYGGWSFAFRLRSSSGLQVLNVHFGGERIAYEVSVQEAVALYGGHTPAGMQTKYLDVGWGLGSVTHELAPGIDCPETATFLDTFHYYDADDPVHYPRALCLFEMPTGVPLRRHFNSNFKGGFNFYAGLKGQVLVLRTTSTVYNYDYIWDFIFYPNGVMEAKMHATGYVHATFYTPEGLRHGTRLHTHLIGNIHTHLVHYRVDLDVAGTKNSFQTLQMKLENITNPWSPRHRVVQPTLEQTQYSWERQAAFRFKRKLPTYLLFTSPQENPWGHKRSYRLQIHSMADQVLPPGWQEEQAITWARYPLAVTKYRESELCSSSIYHQNDPWHPPVVFEQFLHNNENIENEDLVAWVTVGFLHIPHSEDIPNTATPGNSVGFLLRPFNFFPEDPSLASRDTVIVWPRDNGPNYVQRWIPEDRDCSMPPPFSYNGTYRPV

SEQ ID NO: 42 - protein, 983 aa, Artificial Sequence
  Fc-hDAO-Hepmut3
MPALGWAVAAILMLQTAMAECPPCPAPPVAGPSVFLFPPKPKDTLMISRTPEVTCVVVDVSHEDPEVKFNWYVDGVEVHNAKTKPREEQYNSTYRVVSVLTVLHQDWLNGKEYKCKVSNKGLPSSIEKTISKAKGQPREPQVYTLPPSREEMTKNQVSLTCLVKGFYPSDIAVEWESNGQPENNYKTTPPVLDSDGSFFLYSKLTVDKSRWQQGNVFSCSVMHEALHNHYTQKSLSLSPGKEPKSADKTHTEPSPGTLPRKAGVFSDLSNQELKAVHSFLWSKKELRLQPSSTTTMAKNTVFLIEMLLPKKYHVLRFLDKGERHPVREARAVIFFGDQEHPNVTEFAVGPLPGPCYMRALSPRPGYQSSWASRPISTAEYALLYHTLQEATKPLHQFFLNTTGFSFQDCHDRCLAFTDVAPRGVASGQRRSWLIIQRYVEGYFLHPTGLELLVDHGSTDAGHWAVEQVWYNGKFYGSPEELARKYADGEVDVVVLEDPLPGGKGHDSTEEPPLFSSHKPRGDFPSPIHVSGPRLVQPHGPRFRLEGNAVLYGGWSFAFRLRSSSGLQVLNVHFGGERIAYEVSVQEAVALYGGHTPAGMQTKYLDVGWGLGSVTHELAPGIDCPETATFLDTFHYYDADDPVHYPRALCLFEMPTGVPLRRHFNSNFKGGFNFYAGLKGQVLVLRTTSTVYNYDYIWDFIFYPNGVMEAKMHATGYVHATFYTPEGLRHGTRLHTHLIGNIHTHLVHYRVDLDVAGTKNSFQTLQMKLENITNPWSPRHRVVQPTLEQTQYSWERQAAFRFKTKLPKYLLFTSPQENPWGHKRSYRLQIHSMADQVLPPGWQEEQAITWARYPLAVTKYRESELCSSSIYHQNDPWHPPVVFEQFLHNNENIENEDLVAWVTVGFLHIPHSEDIPNTATPGNSVGFLLRPFNFFPEDPSLASRDTVIVWPRDNGPNYVQRWIPEDRDCSMPPPFSYNGTYRPV

SEQ ID NO: 43 - protein, 983 aa, Artificial Sequence
  Fc-hDAO-Hepmut4
MPALGWAVAAILMLQTAMAECPPCPAPPVAGPSVFLFPPKPKDTLMISRTPEVTCVVVDVSHEDPEVKFNWYVDGVEVHNAKTKPREEQYNSTYRVVSVLTVLHQDWLNGKEYKCKVSNKGLPSSIEKTISKAKGQPREPQVYTLPPSREEMTKNQVSLTCLVKGFYPSDIAVEWESNGQPENNYKTTPPVLDSDGSFFLYSKLTVDKSRWQQGNVFSCSVMHEALHNHYTQKSLSLSPGKEPKSADKTHTEPSPGTLPRKAGVFSDLSNQELKAVHSFLWSKKELRLQPSSTTTMAKNTVFLIEMLLPKKYHVLRFLDKGERHPVREARAVIFFGDQEHPNVTEFAVGPLPGPCYMRALSPRPGYQSSWASRPISTAEYALLYHTLQEATKPLHQFFLNTTGFSFQDCHDRCLAFTDVAPRGVASGQRRSWLIIQRYVEGYFLHPTGLELLVDHGSTDAGHWAVEQVWYNGKFYGSPEELARKYADGEVDVVVLEDPLPGGKGHDSTEEPPLFSSHKPRGDFPSPIHVSGPRLVQPHGPRFRLEGNAVLYGGWSFAFRLRSSSGLQVLNVHFGGERIAYEVSVQEAVALYGGHTPAGMQTKYLDVGWGLGSVTHELAPGIDCPETATFLDTFHYYDADDPVHYPRALCLFEMPTGVPLRRHFNSNFKGGFNFYAGLKGQVLVLRTTSTVYNYDYIWDFIFYPNGVMEAKMHATGYVHATFYTPEGLRHGTRLHTHLIGNIHTHLVHYRVDLDVAGTKNSFQTLQMKLENITNPWSPRHRVVQPTLEQTQYSWERQAAFSFKTKLPKYLLFTSPQENPWGHKRSYRLQIHSMADQVLPPGWQEEQAITWARYPLAVTKYRESELCSSSIYHQNDPWHPPVVFEQFLHNNENIENEDLVAWVTVGFLHIPHSEDIPNTATPGNSVGFLLRPFNFFPEDPSLASRDTVIVWPRDNGPNYVQRWIPEDRDCSMPPPFSYNGTYRPV

SEQ ID NO: 44 - protein, 983 aa, Artificial Sequence
  Fc-hDAO-Hepmut5
MPALGWAVAAILMLQTAMAECPPCPAPPVAGPSVFLFPPKPKDTLMISRTPEVTCVVVDVSHEDPEVKFNWYVDGVEVHNAKTKPREEQYNSTYRVVSVLTVLHQDWLNGKEYKCKVSNKGLPSSIEKTISKAKGQPREPQVYTLPPSREEMTKNQVSLTCLVKGFYPSDIAVEWESNGQPENNYKTTPPVLDSDGSFFLYSKLTVDKSRWQQGNVFSCSVMHEALHNHYTQKSLSLSPGKEPKSADKTHTEPSPGTLPRKAGVFSDLSNQELKAVHSFLWSKKELRLQPSSTTTMAKNTVFLIEMLLPKKYHVLRFLDKGERHPVREARAVIFFGDQEHPNVTEFAVGPLPGPCYMRALSPRPGYQSSWASRPISTAEYALLYHTLQEATKPLHQFFLNTTGFSFQDCHDRCLAFTDVAPRGVASGQRRSWLIIQRYVEGYFLHPTGLELLVDHGSTDAGHWAVEQVWYNGKFYGSPEELARKYADGEVDVVVLEDPLPGGKGHDSTEEPPLFSSHKPRGDFPSPIHVSGPRLVQPHGPRFRLEGNAVLYGGWSFAFRLRSSSGLQVLNVHFGGERIAYEVSVQEAVALYGGHTPAGMQTKYLDVGWGLGSVTHELAPGIDCPETATFLDTFHYYDADDPVHYPRALCLFEMPTGVPLRRHFNSNFKGGFNFYAGLKGQVLVLRTTSTVYNYDYIWDFIFYPNGVMEAKMHATGYVHATFYTPEGLRHGTRLHTHLIGNIHTHLVHYRVDLDVAGTKNSFQTLQMKLENITNPWSPRHRVVQPTLEQTQYSWERQAAFRFKTKLPTYLLFTSPQENPWGHKRSYRLQIHSMADQVLPPGWQEEQAITWARYPLAVTKYRESELCSSSIYHQNDPWHPPVVFEQFLHNNENIENEDLVAWVTVGFLHIPHSEDIPNTATPGNSVGFLLRPFNFFPEDPSLASRDTVIVWPRDNGPNYVQRWIPEDRDCSMPPPFSYNGTYRPV

SEQ ID NO: 45 - protein, 983 aa, Artificial Sequence
  Fc-hDAO-Hepmut6
MPALGWAVAAILMLQTAMAECPPCPAPPVAGPSVFLFPPKPKDTLMISRTPEVTCVVVDVSHEDPEVKFNWYVDGVEVHNAKTKPREEQYNSTYRVVSVLTVLHQDWLNGKEYKCKVSNKGLPSSIEKTISKAKGQPREPQVYTLPPSREEMTKNQVSLTCLVKGFYPSDIAVEWESNGQPENNYKTTPPVLDSDGSFFLYSKLTVDKSRWQQGNVFSCSVMHEALHNHYTQKSLSLSPGKEPKSADKTHTEPSPGTLPRKAGVFSDLSNQELKAVHSFLWSKKELRLQPSSTTTMAKNTVFLIEMLLPKKYHVLRFLDKGERHPVREARAVIFFGDQEHPNVTEFAVGPLPGPCYMRALSPRPGYQSSWASRPISTAEYALLYHTLQEATKPLHQFFLNTTGFSFQDCHDRCLAFTDVAPRGVASGQRRSWLIIQRYVEGYFLHPTGLELLVDHGSTDAGHWAVEQVWYNGKFYGSPEELARKYADGEVDVVVLEDPLPGGKGHDSTEEPPLFSSHKPRGDFPSPIHVSGPRLVQPHGPRFRLEGNAVLYGGWSFAFRLRSSSGLQVLNVHFGGERIAYEVSVQEAVALYGGHTPAGMQTKYLDVGWGLGSVTHELAPGIDCPETATFLDTFHYYDADDPVHYPRALCLFEMPTGVPLRRHFNSNFKGGFNFYAGLKGQVLVLRTTSTVYNYDYIWDFIFYPNGVMEAKMHATGYVHATFYTPEGLRHGTRLHTHLIGNIHTHLVHYRVDLDVAGTKNSFQTLQMKLENITNPWSPRHRVVQPTLEQTQYSWERQAAFRFGQTLPKYLLFTSPQENPWGHKRSYRLQIHSMADQVLPPGWQEEQAITWARYPLAVTKYRESELCSSSIYHQNDPWHPPVVFEQFLHNNENIENEDLVAWVTVGFLHIPHSEDIPNTATPGNSVGFLLRPFNFFPEDPSLASRDTVIVWPRDNGPNYVQRWIPEDRDCSMPPPFSYNGTYRPV

SEQ ID NO: 46 - protein, 983 aa, Artificial Sequence
  Fc-hDAO-Hepmut7
MPALGWAVAAILMLQTAMAECPPCPAPPVAGPSVFLFPPKPKDTLMISRTPEVTCVVVDVSHEDPEVKFNWYVDGVEVHNAKTKPREEQYNSTYRVVSVLTVLHQDWLNGKEYKCKVSNKGLPSSIEKTISKAKGQPREPQVYTLPPSREEMTKNQVSLTCLVKGFYPSDIAVEWESNGQPENNYKTTPPVLDSDGSFFLYSKLTVDKSRWQQGNVFSCSVMHEALHNHYTQKSLSLSPGKEPKSADKTHTEPSPGTLPRKAGVFSDLSNQELKAVHSFLWSKKELRLQPSSTTTMAKNTVFLIEMLLPKKYHVLRFLDKGERHPVREARAVIFFGDQEHPNVTEFAVGPLPGPCYMRALSPRPGYQSSWASRPISTAEYALLYHTLQEATKPLHQFFLNTTGFSFQDCHDRCLAFTDVAPRGVASGQRRSWLIIQRYVEGYFLHPTGLELLVDHGSTDAGHWAVEQVWYNGKFYGSPEELARKYADGEVDVVVLEDPLPGGKGHDSTEEPPLFSSHKPRGDFPSPIHVSGPRLVQPHGPRFRLEGNAVLYGGWSFAFRLRSSSGLQVLNVHFGGERIAYEVSVQEAVALYGGHTPAGMQTKYLDVGWGLGSVTHELAPGIDCPETATFLDTFHYYDADDPVHYPRALCLFEMPTGVPLRRHFNSNFKGGFNFYAGLKGQVLVLRTTSTVYNYDYIWDFIFYPNGVMEAKMHATGYVHATFYTPEGLRHGTRLHTHLIGNIHTHLVHYRVDLDVAGTKNSFQTLQMKLENITNPWSPRHRVVQPTLEQTQYSWERQAAFSFKRKLPTYLLFTSPQENPWGHKRSYRLQIHSMADQVLPPGWQEEQAITWARYPLAVTKYRESELCSSSIYHQNDPWHPPVVFEQFLHNNENIENEDLVAWVTVGFLHIPHSEDIPNTATPGNSVGFLLRPFNFFPEDPSLASRDTVIVWPRDNGPNYVQRWIPEDRDCSMPPPFSYNGTYRPV

SEQ ID NO: 47 - protein, 983 aa, Artificial Sequence
  Fc-hDAO-Cysmut
MPALGWAVAAILMLQTAMAECPPCPAPPVAGPSVFLFPPKPKDTLMISRTPEVTCVVVDVSHEDPEVKFNWYVDGVEVHNAKTKPREEQYNSTYRVVSVLTVLHQDWLNGKEYKCKVSNKGLPSSIEKTISKAKGQPREPQVYTLPPSREEMTKNQVSLTCLVKGFYPSDIAVEWESNGQPENNYKTTPPVLDSDGSFFLYSKLTVDKSRWQQGNVFSCSVMHEALHNHYTQKSLSLSPGKEPKSADKTHTEPSPGTLPRKAGVFSDLSNQELKAVHSFLWSKKELRLQPSSTTTMAKNTVFLIEMLLPKKYHVLRFLDKGERHPVREARAVIFFGDQEHPNVTEFAVGPLPGPAYMRALSPRPGYQSSWASRPISTAEYALLYHTLQEATKPLHQFFLNTTGFSFQDCHDRCLAFTDVAPRGVASGQRRSWLIIQRYVEGYFLHPTGLELLVDHGSTDAGHWAVEQVWYNGKFYGSPEELARKYADGEVDVVVLEDPLPGGKGHDSTEEPPLFSSHKPRGDFPSPIHVSGPRLVQPHGPRFRLEGNAVLYGGWSFAFRLRSSSGLQVLNVHFGGERIAYEVSVQEAVALYGGHTPAGMQTKYLDVGWGLGSVTHELAPGIDCPETATFLDTFHYYDADDPVHYPRALCLFEMPTGVPLRRHFNSNFKGGFNFYAGLKGQVLVLRTTSTVYNYDYIWDFIFYPNGVMEAKMHATGYVHATFYTPEGLRHGTRLHTHLIGNIHTHLVHYRVDLDVAGTKNSFQTLQMKLENITNPWSPRHRVVQPTLEQTQYSWERQAAFRFKRKLPKYLLFTSPQENPWGHKRSYRLQIHSMADQVLPPGWQEEQAITWARYPLAVTKYRESELCSSSIYHQNDPWHPPVVFEQFLHNNENIENEDLVAWVTVGFLHIPHSEDIPNTATPGNSVGFLLRPFNFFPEDPSLASRDTVIVWPRDNGPNYVQRWIPEDRDCSMPPPFSYNGTYRPV

SEQ ID NO: 48 - protein, 983 aa, Artificial Sequence
  Fc-hDAO-Hepmut1-Cysmut
MPALGWAVAAILMLQTAMAECPPCPAPPVAGPSVFLFPPKPKDTLMISRTPEVTCVVVDVSHEDPEVKFNWYVDGVEVHNAKTKPREEQYNSTYRVVSVLTVLHQDWLNGKEYKCKVSNKGLPSSIEKTISKAKGQPREPQVYTLPPSREEMTKNQVSLTCLVKGFYPSDIAVEWESNGQPENNYKTTPPVLDSDGSFFLYSKLTVDKSRWQQGNVFSCSVMHEALHNHYTQKSLSLSPGKEPKSADKTHTEPSPGTLPRKAGVFSDLSNQELKAVHSFLWSKKELRLQPSSTTTMAKNTVFLIEMLLPKKYHVLRFLDKGERHPVREARAVIFFGDQEHPNVTEFAVGPLPGPAYMRALSPRPGYQSSWASRPISTAEYALLYHTLQEATKPLHQFFLNTTGFSFQDCHDRCLAFTDVAPRGVASGQRRSWLIIQRYVEGYFLHPTGLELLVDHGSTDAGHWAVEQVWYNGKFYGSPEELARKYADGEVDVVVLEDPLPGGKGHDSTEEPPLFSSHKPRGDFPSPIHVSGPRLVQPHGPRFRLEGNAVLYGGWSFAFRLRSSSGLQVLNVHFGGERIAYEVSVQEAVALYGGHTPAGMQTKYLDVGWGLGSVTHELAPGIDCPETATFLDTFHYYDADDPVHYPRALCLFEMPTGVPLRRHFNSNFKGGFNFYAGLKGQVLVLRTTSTVYNYDYIWDFIFYPNGVMEAKMHATGYVHATFYTPEGLRHGTRLHTHLIGNIHTHLVHYRVDLDVAGTKNSFQTLQMKLENITNPWSPRHRVVQPTLEQTQYSWERQAAFSFKRKLPKYLLFTSPQENPWGHKRSYRLQIHSMADQVLPPGWQEEQAITWARYPLAVTKYRESELCSSSIYHQNDPWHPPVVFEQFLHNNENIENEDLVAWVTVGFLHIPHSEDIPNTATPGNSVGFLLRPFNFFPEDPSLASRDTVIVWPRDNGPNYVQRWIPEDRDCSMPPPFSYNGTYRPV

SEQ ID NO: 49 - protein, 983 aa, Artificial Sequence
  Fc-hDAO-Hepmut2-Cysmut
MPALGWAVAAILMLQTAMAECPPCPAPPVAGPSVFLFPPKPKDTLMISRTPEVTCVVVDVSHEDPEVKFNWYVDGVEVHNAKTKPREEQYNSTYRVVSVLTVLHQDWLNGKEYKCKVSNKGLPSSIEKTISKAKGQPREPQVYTLPPSREEMTKNQVSLTCLVKGFYPSDIAVEWESNGQPENNYKTTPPVLDSDGSFFLYSKLTVDKSRWQQGNVFSCSVMHEALHNHYTQKSLSLSPGKEPKSADKTHTEPSPGTLPRKAGVFSDLSNQELKAVHSFLWSKKELRLQPSSTTTMAKNTVFLIEMLLPKKYHVLRFLDKGERHPVREARAVIFFGDQEHPNVTEFAVGPLPGPAYMRALSPRPGYQSSWASRPISTAEYALLYHTLQEATKPLHQFFLNTTGFSFQDCHDRCLAFTDVAPRGVASGQRRSWLIIQRYVEGYFLHPTGLELLVDHGSTDAGHWAVEQVWYNGKFYGSPEELARKYADGEVDVVVLEDPLPGGKGHDSTEEPPLFSSHKPRGDFPSPIHVSGPRLVQPHGPRFRLEGNAVLYGGWSFAFRLRSSSGLQVLNVHFGGERIAYEVSVQEAVALYGGHTPAGMQTKYLDVGWGLGSVTHELAPGIDCPETATFLDTFHYYDADDPVHYPRALCLFEMPTGVPLRRHFNSNFKGGFNFYAGLKGQVLVLRTTSTVYNYDYIWDFIFYPNGVMEAKMHATGYVHATFYTPEGLRHGTRLHTHLIGNIHTHLVHYRVDLDVAGTKNSFQTLQMKLENITNPWSPRHRVVQPTLEQTQYSWERQAAFRFKRKLPTYLLFTSPQENPWGHKRSYRLQIHSMADQVLPPGWQEEQAITWARYPLAVTKYRESELCSSSIYHQNDPWHPPVVFEQFLHNNENIENEDLVAWVTVGFLHIPHSEDIPNTATPGNSVGFLLRPFNFFPEDPSLASRDTVIVWPRDNGPNYVQRWIPEDRDCSMPPPFSYNGTYRPV

SEQ ID NO: 50 - protein, 983 aa, Artificial Sequence
  Fc-hDAO-Hepmut3-Cysmut
MPALGWAVAAILMLQTAMAECPPCPAPPVAGPSVFLFPPKPKDTLMISRTPEVTCVVVDVSHEDPEVKFNWYVDGVEVHNAKTKPREEQYNSTYRVVSVLTVLHQDWLNGKEYKCKVSNKGLPSSIEKTISKAKGQPREPQVYTLPPSREEMTKNQVSLTCLVKGFYPSDIAVEWESNGQPENNYKTTPPVLDSDGSFFLYSKLTVDKSRWQQGNVFSCSVMHEALHNHYTQKSLSLSPGKEPKSADKTHTEPSPGTLPRKAGVFSDLSNQELKAVHSFLWSKKELRLQPSSTTTMAKNTVFLIEMLLPKKYHVLRFLDKGERHPVREARAVIFFGDQEHPNVTEFAVGPLPGPAYMRALSPRPGYQSSWASRPISTAEYALLYHTLQEATKPLHQFFLNTTGFSFQDCHDRCLAFTDVAPRGVASGQRRSWLIIQRYVEGYFLHPTGLELLVDHGSTDAGHWAVEQVWYNGKFYGSPEELARKYADGEVDVVVLEDPLPGGKGHDSTEEPPLFSSHKPRGDFPSPIHVSGPRLVQPHGPRFRLEGNAVLYGGWSFAFRLRSSSGLQVLNVHFGGERIAYEVSVQEAVALYGGHTPAGMQTKYLDVGWGLGSVTHELAPGIDCPETATFLDTFHYYDADDPVHYPRALCLFEMPTGVPLRRHFNSNFKGGFNFYAGLKGQVLVLRTTSTVYNYDYIWDFIFYPNGVMEAKMHATGYVHATFYTPEGLRHGTRLHTHLIGNIHTHLVHYRVDLDVAGTKNSFQTLQMKLENITNPWSPRHRVVQPTLEQTQYSWERQAAFRFKTKLPKYLLFTSPQENPWGHKRSYRLQIHSMADQVLPPGWQEEQAITWARYPLAVTKYRESELCSSSIYHQNDPWHPPVVFEQFLHNNENIENEDLVAWVTVGFLHIPHSEDIPNTATPGNSVGFLLRPFNFFPEDPSLASRDTVIVWPRDNGPNYVQRWIPEDRDCSMPPPFSYNGTYRPV

SEQ ID NO: 51 - protein, 983 aa, Artificial Sequence
  Fc-hDAO-Hepmut4-Cysmut
MPALGWAVAAILMLQTAMAECPPCPAPPVAGPSVFLFPPKPKDTLMISRTPEVTCVVVDVSHEDPEVKFNWYVDGVEVHNAKTKPREEQYNSTYRVVSVLTVLHQDWLNGKEYKCKVSNKGLPSSIEKTISKAKGQPREPQVYTLPPSREEMTKNQVSLTCLVKGFYPSDIAVEWESNGQPENNYKTTPPVLDSDGSFFLYSKLTVDKSRWQQGNVFSCSVMHEALHNHYTQKSLSLSPGKEPKSADKTHTEPSPGTLPRKAGVFSDLSNQELKAVHSFLWSKKELRLQPSSTTTMAKNTVFLIEMLLPKKYHVLRFLDKGERHPVREARAVIFFGDQEHPNVTEFAVGPLPGPAYMRALSPRPGYQSSWASRPISTAEYALLYHTLQEATKPLHQFFLNTTGFSFQDCHDRCLAFTDVAPRGVASGQRRSWLIIQRYVEGYFLHPTGLELLVDHGSTDAGHWAVEQVWYNGKFYGSPEELARKYADGEVDVVVLEDPLPGGKGHDSTEEPPLFSSHKPRGDFPSPIHVSGPRLVQPHGPRFRLEGNAVLYGGWSFAFRLRSSSGLQVLNVHFGGERIAYEVSVQEAVALYGGHTPAGMQTKYLDVGWGLGSVTHELAPGIDCPETATFLDTFHYYDADDPVHYPRALCLFEMPTGVPLRRHFNSNFKGGFNFYAGLKGQVLVLRTTSTVYNYDYIWDFIFYPNGVMEAKMHATGYVHATFYTPEGLRHGTRLHTHLIGNIHTHLVHYRVDLDVAGTKNSFQTLQMKLENITNPWSPRHRVVQPTLEQTQYSWERQAAFSFKTKLPKYLLFTSPQENPWGHKRSYRLQIHSMADQVLPPGWQEEQAITWARYPLAVTKYRESELCSSSIYHQNDPWHPPVVFEQFLHNNENIENEDLVAWVTVGFLHIPHSEDIPNTATPGNSVGFLLRPFNFFPEDPSLASRDTVIVWPRDNGPNYVQRWIPEDRDCSMPPPFSYNGTYRPV

SEQ ID NO: 52 - protein, 983 aa, Artificial Sequence
  Fc-hDAO-Hepmut5-Cysmut
MPALGWAVAAILMLQTAMAECPPCPAPPVAGPSVFLFPPKPKDTLMISRTPEVTCVVVDVSHEDPEVKFNWYVDGVEVHNAKTKPREEQYNSTYRVVSVLTVLHQDWLNGKEYKCKVSNKGLPSSIEKTISKAKGQPREPQVYTLPPSREEMTKNQVSLTCLVKGFYPSDIAVEWESNGQPENNYKTTPPVLDSDGSFFLYSKLTVDKSRWQQGNVFSCSVMHEALHNHYTQKSLSLSPGKEPKSADKTHTEPSPGTLPRKAGVFSDLSNQELKAVHSFLWSKKELRLQPSSTTTMAKNTVFLIEMLLPKKYHVLRFLDKGERHPVREARAVIFFGDQEHPNVTEFAVGPLPGPAYMRALSPRPGYQSSWASRPISTAEYALLYHTLQEATKPLHQFFLNTTGFSFQDCHDRCLAFTDVAPRGVASGQRRSWLIIQRYVEGYFLHPTGLELLVDHGSTDAGHWAVEQVWYNGKFYGSPEELARKYADGEVDVVVLEDPLPGGKGHDSTEEPPLFSSHKPRGDFPSPIHVSGPRLVQPHGPRFRLEGNAVLYGGWSFAFRLRSSSGLQVLNVHFGGERIAYEVSVQEAVALYGGHTPAGMQTKYLDVGWGLGSVTHELAPGIDCPETATFLDTFHYYDADDPVHYPRALCLFEMPTGVPLRRHFNSNFKGGFNFYAGLKGQVLVLRTTSTVYNYDYIWDFIFYPNGVMEAKMHATGYVHATFYTPEGLRHGTRLHTHLIGNIHTHLVHYRVDLDVAGTKNSFQTLQMKLENITNPWSPRHRVVQPTLEQTQYSWERQAAFRFKTKLPTYLLFTSPQENPWGHKRSYRLQIHSMADQVLPPGWQEEQAITWARYPLAVTKYRESELCSSSIYHQNDPWHPPVVFEQFLHNNENIENEDLVAWVTVGFLHIPHSEDIPNTATPGNSVGFLLRPFNFFPEDPSLASRDTVIVWPRDNGPNYVQRWIPEDRDCSMPPPFSYNGTYRPV

SEQ ID NO: 53 - protein, 983 aa, Artificial Sequence
  Fc-hDAO-Hepmut6-Cysmut
MPALGWAVAAILMLQTAMAECPPCPAPPVAGPSVFLFPPKPKDTLMISRTPEVTCVVVDVSHEDPEVKFNWYVDGVEVHNAKTKPREEQYNSTYRVVSVLTVLHQDWLNGKEYKCKVSNKGLPSSIEKTISKAKGQPREPQVYTLPPSREEMTKNQVSLTCLVKGFYPSDIAVEWESNGQPENNYKTTPPVLDSDGSFFLYSKLTVDKSRWQQGNVFSCSVMHEALHNHYTQKSLSLSPGKEPKSADKTHTEPSPGTLPRKAGVFSDLSNQELKAVHSFLWSKKELRLQPSSTTTMAKNTVFLIEMLLPKKYHVLRFLDKGERHPVREARAVIFFGDQEHPNVTEFAVGPLPGPAYMRALSPRPGYQSSWASRPISTAEYALLYHTLQEATKPLHQFFLNTTGFSFQDCHDRCLAFTDVAPRGVASGQRRSWLIIQRYVEGYFLHPTGLELLVDHGSTDAGHWAVEQVWYNGKFYGSPEELARKYADGEVDVVVLEDPLPGGKGHDSTEEPPLFSSHKPRGDFPSPIHVSGPRLVQPHGPRFRLEGNAVLYGGWSFAFRLRSSSGLQVLNVHFGGERIAYEVSVQEAVALYGGHTPAGMQTKYLDVGWGLGSVTHELAPGIDCPETATFLDTFHYYDADDPVHYPRALCLFEMPTGVPLRRHFNSNFKGGFNFYAGLKGQVLVLRTTSTVYNYDYIWDFIFYPNGVMEAKMHATGYVHATFYTPEGLRHGTRLHTHLIGNIHTHLVHYRVDLDVAGTKNSFQTLQMKLENITNPWSPRHRVVQPTLEQTQYSWERQAAFRFGQTLPKYLLFTSPQENPWGHKRSYRLQIHSMADQVLPPGWQEEQAITWARYPLAVTKYRESELCSSSIYHQNDPWHPPVVFEQFLHNNENIENEDLVAWVTVGFLHIPHSEDIPNTATPGNSVGFLLRPFNFFPEDPSLASRDTVIVWPRDNGPNYVQRWIPEDRDCSMPPPFSYNGTYRPV

SEQ ID NO: 54 - protein, 983 aa, Artificial Sequence
  Fc-hDAO-Hepmut7-Cysmut
MPALGWAVAAILMLQTAMAECPPCPAPPVAGPSVFLFPPKPKDTLMISRTPEVTCVVVDVSHEDPEVKFNWYVDGVEVHNAKTKPREEQYNSTYRVVSVLTVLHQDWLNGKEYKCKVSNKGLPSSIEKTISKAKGQPREPQVYTLPPSREEMTKNQVSLTCLVKGFYPSDIAVEWESNGQPENNYKTTPPVLDSDGSFFLYSKLTVDKSRWQQGNVFSCSVMHEALHNHYTQKSLSLSPGKEPKSADKTHTEPSPGTLPRKAGVFSDLSNQELKAVHSFLWSKKELRLQPSSTTTMAKNTVFLIEMLLPKKYHVLRFLDKGERHPVREARAVIFFGDQEHPNVTEFAVGPLPGPAYMRALSPRPGYQSSWASRPISTAEYALLYHTLQEATKPLHQFFLNTTGFSFQDCHDRCLAFTDVAPRGVASGQRRSWLIIQRYVEGYFLHPTGLELLVDHGSTDAGHWAVEQVWYNGKFYGSPEELARKYADGEVDVVVLEDPLPGGKGHDSTEEPPLFSSHKPRGDFPSPIHVSGPRLVQPHGPRFRLEGNAVLYGGWSFAFRLRSSSGLQVLNVHFGGERIAYEVSVQEAVALYGGHTPAGMQTKYLDVGWGLGSVTHELAPGIDCPETATFLDTFHYYDADDPVHYPRALCLFEMPTGVPLRRHFNSNFKGGFNFYAGLKGQVLVLRTTSTVYNYDYIWDFIFYPNGVMEAKMHATGYVHATFYTPEGLRHGTRLHTHLIGNIHTHLVHYRVDLDVAGTKNSFQTLQMKLENITNPWSPRHRVVQPTLEQTQYSWERQAAFSFKRKLPTYLLFTSPQENPWGHKRSYRLQIHSMADQVLPPGWQEEQAITWARYPLAVTKYRESELCSSSIYHQNDPWHPPVVFEQFLHNNENIENEDLVAWVTVGFLHIPHSEDIPNTATPGNSVGFLLRPFNFFPEDPSLASRDTVIVWPRDNGPNYVQRWIPEDRDCSMPPPFSYNGTYRPV

SEQ ID NO: 55 - protein, 982 aa, Artificial Sequence
  hDAO-Fc
MPALGWAVAAILMLQTAMAEPSPGTLPRKAGVFSDLSNQELKAVHSFLWSKKELRLQPSSTTTMAKNTVFLIEMLLPKKYHVLRFLDKGERHPVREARAVIFFGDQEHPNVTEFAVGPLPGPCYMRALSPRPGYQSSWASRPISTAEYALLYHTLQEATKPLHQFFLNTTGFSFQDCHDRCLAFTDVAPRGVASGQRRSWLIIQRYVEGYFLHPTGLELLVDHGSTDAGHWAVEQVWYNGKFYGSPEELARKYADGEVDVVVLEDPLPGGKGHDSTEEPPLFSSHKPRGDFPSPIHVSGPRLVQPHGPRFRLEGNAVLYGGWSFAFRLRSSSGLQVLNVHFGGERIAYEVSVQEAVALYGGHTPAGMQTKYLDVGWGLGSVTHELAPGIDCPETATFLDTFHYYDADDPVHYPRALCLFEMPTGVPLRRHFNSNFKGGFNFYAGLKGQVLVLRTTSTVYNYDYIWDFIFYPNGVMEAKMHATGYVHATFYTPEGLRHGTRLHTHLIGNIHTHLVHYRVDLDVAGTKNSFQTLQMKLENITNPWSPRHRVVQPTLEQTQYSWERQAAFRFKRKLPKYLLFTSPQENPWGHKRSYRLQIHSMADQVLPPGWQEEQAITWARYPLAVTKYRESELCSSSIYHQNDPWHPPVVFEQFLHNNENIENEDLVAWVTVGFLHIPHSEDIPNTATPGNSVGFLLRPFNFFPEDPSLASRDTVIVWPRDNGPNYVQRWIPEDRDCSMPPPFSYNGTYRPVEPKSADKTHTCPPCPAPPVAGPSVFLFPPKPKDTLMISRTPEVTCVVVDVSHEDPEVKFNWYVDGVEVHNAKTKPREEQYNSTYRVVSVLTVLHQDWLNGKEYKCKVSNKGLPSSIEKTISKAKGQPREPQVYTLPPSREEMTKNQVSLTCLVKGFYPSDIAVEWESNGQPENNYKTTPPVLDSDGSFFLYSKLTVDKSRWQQGNVFSCSVMHEALHNHYTQKSLSLSPGK

SEQ ID NO: 56 - protein, 982 aa, Artificial Sequence
  hDAO-Fc-Hepmut1
MPALGWAVAAILMLQTAMAEPSPGTLPRKAGVFSDLSNQELKAVHSFLWSKKELRLQPSSTTTMAKNTVFLIEMLLPKKYHVLRFLDKGERHPVREARAVIFFGDQEHPNVTEFAVGPLPGPCYMRALSPRPGYQSSWASRPISTAEYALLYHTLQEATKPLHQFFLNTTGFSFQDCHDRCLAFTDVAPRGVASGQRRSWLIIQRYVEGYFLHPTGLELLVDHGSTDAGHWAVEQVWYNGKFYGSPEELARKYADGEVDVVVLEDPLPGGKGHDSTEEPPLFSSHKPRGDFPSPIHVSGPRLVQPHGPRFRLEGNAVLYGGWSFAFRLRSSSGLQVLNVHFGGERIAYEVSVQEAVALYGGHTPAGMQTKYLDVGWGLGSVTHELAPGIDCPETATFLDTFHYYDADDPVHYPRALCLFEMPTGVPLRRHFNSNFKGGFNFYAGLKGQVLVLRTTSTVYNYDYIWDFIFYPNGVMEAKMHATGYVHATFYTPEGLRHGTRLHTHLIGNIHTHLVHYRVDLDVAGTKNSFQTLQMKLENITNPWSPRHRVVQPTLEQTQYSWERQAAFSFKRKLPKYLLFTSPQENPWGHKRSYRLQIHSMADQVLPPGWQEEQAITWARYPLAVTKYRESELCSSSIYHQNDPWHPPVVFEQFLHNNENIENEDLVAWVTVGFLHIPHSEDIPNTATPGNSVGFLLRPFNFFPEDPSLASRDTVIVWPRDNGPNYVQRWIPEDRDCSMPPPFSYNGTYRPVEPKSADKTHTCPPCPAPPVAGPSVFLFPPKPKDTLMISRTPEVTCVVVDVSHEDPEVKFNWYVDGVEVHNAKTKPREEQYNSTYRVVSVLTVLHQDWLNGKEYKCKVSNKGLPSSIEKTISKAKGQPREPQVYTLPPSREEMTKNQVSLTCLVKGFYPSDIAVEWESNGQPENNYKTTPPVLDSDGSFFLYSKLTVDKSRWQQGNVFSCSVMHEALHNHYTQKSLSLSPGK

SEQ ID NO: 57 - protein, 982 aa, Artificial Sequence
  hDAO-Fc-Hepmut2
MPALGWAVAAILMLQTAMAEPSPGTLPRKAGVFSDLSNQELKAVHSFLWSKKELRLQPSSTTTMAKNTVFLIEMLLPKKYHVLRFLDKGERHPVREARAVIFFGDQEHPNVTEFAVGPLPGPCYMRALSPRPGYQSSWASRPISTAEYALLYHTLQEATKPLHQFFLNTTGFSFQDCHDRCLAFTDVAPRGVASGQRRSWLIIQRYVEGYFLHPTGLELLVDHGSTDAGHWAVEQVWYNGKFYGSPEELARKYADGEVDVVVLEDPLPGGKGHDSTEEPPLFSSHKPRGDFPSPIHVSGPRLVQPHGPRFRLEGNAVLYGGWSFAFRLRSSSGLQVLNVHFGGERIAYEVSVQEAVALYGGHTPAGMQTKYLDVGWGLGSVTHELAPGIDCPETATFLDTFHYYDADDPVHYPRALCLFEMPTGVPLRRHFNSNFKGGFNFYAGLKGQVLVLRTTSTVYNYDYIWDFIFYPNGVMEAKMHATGYVHATFYTPEGLRHGTRLHTHLIGNIHTHLVHYRVDLDVAGTKNSFQTLQMKLENITNPWSPRHRVVQPTLEQTQYSWERQAAFRFKRKLPTYLLFTSPQENPWGHKRSYRLQIHSMADQVLPPGWQEEQAITWARYPLAVTKYRESELCSSSIYHQNDPWHPPVVFEQFLHNNENIENEDLVAWVTVGFLHIPHSEDIPNTATPGNSVGFLLRPFNFFPEDPSLASRDTVIVWPRDNGPNYVQRWIPEDRDCSMPPPFSYNGTYRPVEPKSADKTHTCPPCPAPPVAGPSVFLFPPKPKDTLMISRTPEVTCVVVDVSHEDPEVKFNWYVDGVEVHNAKTKPREEQYNSTYRVVSVLTVLHQDWLNGKEYKCKVSNKGLPSSIEKTISKAKGQPREPQVYTLPPSREEMTKNQVSLTCLVKGFYPSDIAVEWESNGQPENNYKTTPPVLDSDGSFFLYSKLTVDKSRWQQGNVFSCSVMHEALHNHYTQKSLSLSPGK

SEQ ID NO: 58 - protein, 982 aa, Artificial Sequence
  hDAO-Fc-Hepmut3
MPALGWAVAAILMLQTAMAEPSPGTLPRKAGVFSDLSNQELKAVHSFLWSKKELRLQPSSTTTMAKNTVFLIEMLLPKKYHVLRFLDKGERHPVREARAVIFFGDQEHPNVTEFAVGPLPGPCYMRALSPRPGYQSSWASRPISTAEYALLYHTLQEATKPLHQFFLNTTGFSFQDCHDRCLAFTDVAPRGVASGQRRSWLIIQRYVEGYFLHPTGLELLVDHGSTDAGHWAVEQVWYNGKFYGSPEELARKYADGEVDVVVLEDPLPGGKGHDSTEEPPLFSSHKPRGDFPSPIHVSGPRLVQPHGPRFRLEGNAVLYGGWSFAFRLRSSSGLQVLNVHFGGERIAYEVSVQEAVALYGGHTPAGMQTKYLDVGWGLGSVTHELAPGIDCPETATFLDTFHYYDADDPVHYPRALCLFEMPTGVPLRRHFNSNFKGGFNFYAGLKGQVLVLRTTSTVYNYDYIWDFIFYPNGVMEAKMHATGYVHATFYTPEGLRHGTRLHTHLIGNIHTHLVHYRVDLDVAGTKNSFQTLQMKLENITNPWSPRHRVVQPTLEQTQYSWERQAAFRFKTKLPKYLLFTSPQENPWGHKRSYRLQIHSMADQVLPPGWQEEQAITWARYPLAVTKYRESELCSSSIYHQNDPWHPPVVFEQFLHNNENIENEDLVAWVTVGFLHIPHSEDIPNTATPGNSVGFLLRPFNFFPEDPSLASRDTVIVWPRDNGPNYVQRWIPEDRDCSMPPPFSYNGTYRPVEPKSADKTHTCPPCPAPPVAGPSVFLFPPKPKDTLMISRTPEVTCVVVDVSHEDPEVKFNWYVDGVEVHNAKTKPREEQYNSTYRVVSVLTVLHQDWLNGKEYKCKVSNKGLPSSIEKTISKAKGQPREPQVYTLPPSREEMTKNQVSLTCLVKGFYPSDIAVEWESNGQPENNYKTTPPVLDSDGSFFLYSKLTVDKSRWQQGNVFSCSVMHEALHNHYTQKSLSLSPGK

SEQ ID NO: 59 - protein, 982 aa, Artificial Sequence
  hDAO-Fc-Hepmut4
MPALGWAVAAILMLQTAMAEPSPGTLPRKAGVFSDLSNQELKAVHSFLWSKKELRLQPSSTTTMAKNTVFLIEMLLPKKYHVLRFLDKGERHPVREARAVIFFGDQEHPNVTEFAVGPLPGPCYMRALSPRPGYQSSWASRPISTAEYALLYHTLQEATKPLHQFFLNTTGFSFQDCHDRCLAFTDVAPRGVASGQRRSWLIIQRYVEGYFLHPTGLELLVDHGSTDAGHWAVEQVWYNGKFYGSPEELARKYADGEVDVVVLEDPLPGGKGHDSTEEPPLFSSHKPRGDFPSPIHVSGPRLVQPHGPRFRLEGNAVLYGGWSFAFRLRSSSGLQVLNVHFGGERIAYEVSVQEAVALYGGHTPAGMQTKYLDVGWGLGSVTHELAPGIDCPETATFLDTFHYYDADDPVHYPRALCLFEMPTGVPLRRHFNSNFKGGFNFYAGLKGQVLVLRTTSTVYNYDYIWDFIFYPNGVMEAKMHATGYVHATFYTPEGLRHGTRLHTHLIGNIHTHLVHYRVDLDVAGTKNSFQTLQMKLENITNPWSPRHRVVQPTLEQTQYSWERQAAFSFKTKLPKYLLFTSPQENPWGHKRSYRLQIHSMADQVLPPGWQEEQAITWARYPLAVTKYRESELCSSSIYHQNDPWHPPVVFEQFLHNNENIENEDLVAWVTVGFLHIPHSEDIPNTATPGNSVGFLLRPFNFFPEDPSLASRDTVIVWPRDNGPNYVQRWIPEDRDCSMPPPFSYNGTYRPVEPKSADKTHTCPPCPAPPVAGPSVFLFPPKPKDTLMISRTPEVTCVVVDVSHEDPEVKFNWYVDGVEVHNAKTKPREEQYNSTYRVVSVLTVLHQDWLNGKEYKCKVSNKGLPSSIEKTISKAKGQPREPQVYTLPPSREEMTKNQVSLTCLVKGFYPSDIAVEWESNGQPENNYKTTPPVLDSDGSFFLYSKLTVDKSRWQQGNVFSCSVMHEALHNHYTQKSLSLSPGK

SEQ ID NO: 60 - protein, 982 aa, Artificial Sequence
  hDAO-Fc-Hepmut5
MPALGWAVAAILMLQTAMAEPSPGTLPRKAGVFSDLSNQELKAVHSFLWSKKELRLQPSSTTTMAKNTVFLIEMLLPKKYHVLRFLDKGERHPVREARAVIFFGDQEHPNVTEFAVGPLPGPCYMRALSPRPGYQSSWASRPISTAEYALLYHTLQEATKPLHQFFLNTTGFSFQDCHDRCLAFTDVAPRGVASGQRRSWLIIQRYVEGYFLHPTGLELLVDHGSTDAGHWAVEQVWYNGKFYGSPEELARKYADGEVDVVVLEDPLPGGKGHDSTEEPPLFSSHKPRGDFPSPIHVSGPRLVQPHGPRFRLEGNAVLYGGWSFAFRLRSSSGLQVLNVHFGGERIAYEVSVQEAVALYGGHTPAGMQTKYLDVGWGLGSVTHELAPGIDCPETATFLDTFHYYDADDPVHYPRALCLFEMPTGVPLRRHFNSNFKGGFNFYAGLKGQVLVLRTTSTVYNYDYIWDFIFYPNGVMEAKMHATGYVHATFYTPEGLRHGTRLHTHLIGNIHTHLVHYRVDLDVAGTKNSFQTLQMKLENITNPWSPRHRVVQPTLEQTQYSWERQAAFRFKTKLPTYLLFTSPQENPWGHKRSYRLQIHSMADQVLPPGWQEEQAITWARYPLAVTKYRESELCSSSIYHQNDPWHPPVVFEQFLHNNENIENEDLVAWVTVGFLHIPHSEDIPNTATPGNSVGFLLRPFNFFPEDPSLASRDTVIVWPRDNGPNYVQRWIPEDRDCSMPPPFSYNGTYRPVEPKSADKTHTCPPCPAPPVAGPSVFLFPPKPKDTLMISRTPEVTCVVVDVSHEDPEVKFNWYVDGVEVHNAKTKPREEQYNSTYRVVSVLTVLHQDWLNGKEYKCKVSNKGLPSSIEKTISKAKGQPREPQVYTLPPSREEMTKNQVSLTCLVKGFYPSDIAVEWESNGQPENNYKTTPPVLDSDGSFFLYSKLTVDKSRWQQGNVFSCSVMHEALHNHYTQKSLSLSPGK

SEQ ID NO: 61 - protein, 982 aa, Artificial Sequence
  hDAO-Fc-Hepmut6
MPALGWAVAAILMLQTAMAEPSPGTLPRKAGVFSDLSNQELKAVHSFLWSKKELRLQPSSTTTMAKNTVFLIEMLLPKKYHVLRFLDKGERHPVREARAVIFFGDQEHPNVTEFAVGPLPGPCYMRALSPRPGYQSSWASRPISTAEYALLYHTLQEATKPLHQFFLNTTGFSFQDCHDRCLAFTDVAPRGVASGQRRSWLIIQRYVEGYFLHPTGLELLVDHGSTDAGHWAVEQVWYNGKFYGSPEELARKYADGEVDVVVLEDPLPGGKGHDSTEEPPLFSSHKPRGDFPSPIHVSGPRLVQPHGPRFRLEGNAVLYGGWSFAFRLRSSSGLQVLNVHFGGERIAYEVSVQEAVALYGGHTPAGMQTKYLDVGWGLGSVTHELAPGIDCPETATFLDTFHYYDADDPVHYPRALCLFEMPTGVPLRRHFNSNFKGGFNFYAGLKGQVLVLRTTSTVYNYDYIWDFIFYPNGVMEAKMHATGYVHATFYTPEGLRHGTRLHTHLIGNIHTHLVHYRVDLDVAGTKNSFQTLQMKLENITNPWSPRHRVVQPTLEQTQYSWERQAAFRFGQTLPKYLLFTSPQENPWGHKRSYRLQIHSMADQVLPPGWQEEQAITWARYPLAVTKYRESELCSSSIYHQNDPWHPPVVFEQFLHNNENIENEDLVAWVTVGFLHIPHSEDIPNTATPGNSVGFLLRPFNFFPEDPSLASRDTVIVWPRDNGPNYVQRWIPEDRDCSMPPPFSYNGTYRPVEPKSADKTHTCPPCPAPPVAGPSVFLFPPKPKDTLMISRTPEVTCVVVDVSHEDPEVKFNWYVDGVEVHNAKTKPREEQYNSTYRVVSVLTVLHQDWLNGKEYKCKVSNKGLPSSIEKTISKAKGQPREPQVYTLPPSREEMTKNQVSLTCLVKGFYPSDIAVEWESNGQPENNYKTTPPVLDSDGSFFLYSKLTVDKSRWQQGNVFSCSVMHEALHNHYTQKSLSLSPGK

SEQ ID NO: 62 - protein, 982 aa, Artificial Sequence
  hDAO-Fc-Hepmut7
MPALGWAVAAILMLQTAMAEPSPGTLPRKAGVFSDLSNQELKAVHSFLWSKKELRLQPSSTTTMAKNTVFLIEMLLPKKYHVLRFLDKGERHPVREARAVIFFGDQEHPNVTEFAVGPLPGPCYMRALSPRPGYQSSWASRPISTAEYALLYHTLQEATKPLHQFFLNTTGFSFQDCHDRCLAFTDVAPRGVASGQRRSWLIIQRYVEGYFLHPTGLELLVDHGSTDAGHWAVEQVWYNGKFYGSPEELARKYADGEVDVVVLEDPLPGGKGHDSTEEPPLFSSHKPRGDFPSPIHVSGPRLVQPHGPRFRLEGNAVLYGGWSFAFRLRSSSGLQVLNVHFGGERIAYEVSVQEAVALYGGHTPAGMQTKYLDVGWGLGSVTHELAPGIDCPETATFLDTFHYYDADDPVHYPRALCLFEMPTGVPLRRHFNSNFKGGFNFYAGLKGQVLVLRTTSTVYNYDYIWDFIFYPNGVMEAKMHATGYVHATFYTPEGLRHGTRLHTHLIGNIHTHLVHYRVDLDVAGTKNSFQTLQMKLENITNPWSPRHRVVQPTLEQTQYSWERQAAFSFKRKLPTYLLFTSPQENPWGHKRSYRLQIHSMADQVLPPGWQEEQAITWARYPLAVTKYRESELCSSSIYHQNDPWHPPVVFEQFLHNNENIENEDLVAWVTVGFLHIPHSEDIPNTATPGNSVGFLLRPFNFFPEDPSLASRDTVIVWPRDNGPNYVQRWIPEDRDCSMPPPFSYNGTYRPVEPKSADKTHTCPPCPAPPVAGPSVFLFPPKPKDTLMISRTPEVTCVVVDVSHEDPEVKFNWYVDGVEVHNAKTKPREEQYNSTYRVVSVLTVLHQDWLNGKEYKCKVSNKGLPSSIEKTISKAKGQPREPQVYTLPPSREEMTKNQVSLTCLVKGFYPSDIAVEWESNGQPENNYKTTPPVLDSDGSFFLYSKLTVDKSRWQQGNVFSCSVMHEALHNHYTQKSLSLSPGK

SEQ ID NO: 63 - protein, 982 aa, Artificial Sequence
  hDAO-Fc-Cysmut
MPALGWAVAAILMLQTAMAEPSPGTLPRKAGVFSDLSNQELKAVHSFLWSKKELRLQPSSTTTMAKNTVFLIEMLLPKKYHVLRFLDKGERHPVREARAVIFFGDQEHPNVTEFAVGPLPGPAYMRALSPRPGYQSSWASRPISTAEYALLYHTLQEATKPLHQFFLNTTGFSFQDCHDRCLAFTDVAPRGVASGQRRSWLIIQRYVEGYFLHPTGLELLVDHGSTDAGHWAVEQVWYNGKFYGSPEELARKYADGEVDVVVLEDPLPGGKGHDSTEEPPLFSSHKPRGDFPSPIHVSGPRLVQPHGPRFRLEGNAVLYGGWSFAFRLRSSSGLQVLNVHFGGERIAYEVSVQEAVALYGGHTPAGMQTKYLDVGWGLGSVTHELAPGIDCPETATFLDTFHYYDADDPVHYPRALCLFEMPTGVPLRRHFNSNFKGGFNFYAGLKGQVLVLRTTSTVYNYDYIWDFIFYPNGVMEAKMHATGYVHATFYTPEGLRHGTRLHTHLIGNIHTHLVHYRVDLDVAGTKNSFQTLQMKLENITNPWSPRHRVVQPTLEQTQYSWERQAAFRFKRKLPKYLLFTSPQENPWGHKRSYRLQIHSMADQVLPPGWQEEQAITWARYPLAVTKYRESELCSSSIYHQNDPWHPPVVFEQFLHNNENIENEDLVAWVTVGFLHIPHSEDIPNTATPGNSVGFLLRPFNFFPEDPSLASRDTVIVWPRDNGPNYVQRWIPEDRDCSMPPPFSYNGTYRPVEPKSADKTHTCPPCPAPPVAGPSVFLFPPKPKDTLMISRTPEVTCVVVDVSHEDPEVKFNWYVDGVEVHNAKTKPREEQYNSTYRVVSVLTVLHQDWLNGKEYKCKVSNKGLPSSIEKTISKAKGQPREPQVYTLPPSREEMTKNQVSLTCLVKGFYPSDIAVEWESNGQPENNYKTTPPVLDSDGSFFLYSKLTVDKSRWQQGNVFSCSVMHEALHNHYTQKSLSLSPGK

SEQ ID NO: 64 - protein, 982 aa, Artificial Sequence
  hDAO-Fc-Hepmut1-Cysmut
MPALGWAVAAILMLQTAMAEPSPGTLPRKAGVFSDLSNQELKAVHSFLWSKKELRLQPSSTTTMAKNTVFLIEMLLPKKYHVLRFLDKGERHPVREARAVIFFGDQEHPNVTEFAVGPLPGPAYMRALSPRPGYQSSWASRPISTAEYALLYHTLQEATKPLHQFFLNTTGFSFQDCHDRCLAFTDVAPRGVASGQRRSWLIIQRYVEGYFLHPTGLELLVDHGSTDAGHWAVEQVWYNGKFYGSPEELARKYADGEVDVVVLEDPLPGGKGHDSTEEPPLFSSHKPRGDFPSPIHVSGPRLVQPHGPRFRLEGNAVLYGGWSFAFRLRSSSGLQVLNVHFGGERIAYEVSVQEAVALYGGHTPAGMQTKYLDVGWGLGSVTHELAPGIDCPETATFLDTFHYYDADDPVHYPRALCLFEMPTGVPLRRHFNSNFKGGFNFYAGLKGQVLVLRTTSTVYNYDYIWDFIFYPNGVMEAKMHATGYVHATFYTPEGLRHGTRLHTHLIGNIHTHLVHYRVDLDVAGTKNSFQTLQMKLENITNPWSPRHRVVQPTLEQTQYSWERQAAFSFKRKLPKYLLFTSPQENPWGHKRSYRLQIHSMADQVLPPGWQEEQAITWARYPLAVTKYRESELCSSSIYHQNDPWHPPVVFEQFLHNNENIENEDLVAWVTVGFLHIPHSEDIPNTATPGNSVGFLLRPFNFFPEDPSLASRDTVIVWPRDNGPNYVQRWIPEDRDCSMPPPFSYNGTYRPVEPKSADKTHTCPPCPAPPVAGPSVFLFPPKPKDTLMISRTPEVTCVVVDVSHEDPEVKFNWYVDGVEVHNAKTKPREEQYNSTYRVVSVLTVLHQDWLNGKEYKCKVSNKGLPSSIEKTISKAKGQPREPQVYTLPPSREEMTKNQVSLTCLVKGFYPSDIAVEWESNGQPENNYKTTPPVLDSDGSFFLYSKLTVDKSRWQQGNVFSCSVMHEALHNHYTQKSLSLSPGK

SEQ ID NO: 65 - protein, 982 aa, Artificial Sequence
  hDAO-Fc-Hepmut2-Cysmut
MPALGWAVAAILMLQTAMAEPSPGTLPRKAGVFSDLSNQELKAVHSFLWSKKELRLQPSSTTTMAKNTVFLIEMLLPKKYHVLRFLDKGERHPVREARAVIFFGDQEHPNVTEFAVGPLPGPAYMRALSPRPGYQSSWASRPISTAEYALLYHTLQEATKPLHQFFLNTTGFSFQDCHDRCLAFTDVAPRGVASGQRRSWLIIQRYVEGYFLHPTGLELLVDHGSTDAGHWAVEQVWYNGKFYGSPEELARKYADGEVDVVVLEDPLPGGKGHDSTEEPPLFSSHKPRGDFPSPIHVSGPRLVQPHGPRFRLEGNAVLYGGWSFAFRLRSSSGLQVLNVHFGGERIAYEVSVQEAVALYGGHTPAGMQTKYLDVGWGLGSVTHELAPGIDCPETATFLDTFHYYDADDPVHYPRALCLFEMPTGVPLRRHFNSNFKGGFNFYAGLKGQVLVLRTTSTVYNYDYIWDFIFYPNGVMEAKMHATGYVHATFYTPEGLRHGTRLHTHLIGNIHTHLVHYRVDLDVAGTKNSFQTLQMKLENITNPWSPRHRVVQPTLEQTQYSWERQAAFRFKRKLPTYLLFTSPQENPWGHKRSYRLQIHSMADQVLPPGWQEEQAITWARYPLAVTKYRESELCSSSIYHQNDPWHPPVVFEQFLHNNENIENEDLVAWVTVGFLHIPHSEDIPNTATPGNSVGFLLRPFNFFPEDPSLASRDTVIVWPRDNGPNYVQRWIPEDRDCSMPPPFSYNGTYRPVEPKSADKTHTCPPCPAPPVAGPSVFLFPPKPKDTLMISRTPEVTCVVVDVSHEDPEVKFNWYVDGVEVHNAKTKPREEQYNSTYRVVSVLTVLHQDWLNGKEYKCKVSNKGLPSSIEKTISKAKGQPREPQVYTLPPSREEMTKNQVSLTCLVKGFYPSDIAVEWESNGQPENNYKTTPPVLDSDGSFFLYSKLTVDKSRWQQGNVFSCSVMHEALHNHYTQKSLSLSPGK

SEQ ID NO: 66 - protein, 982 aa, Artificial Sequence
  hDAO-Fc-Hepmut3-Cysmut
MPALGWAVAAILMLQTAMAEPSPGTLPRKAGVFSDLSNQELKAVHSFLWSKKELRLQPSSTTTMAKNTVFLIEMLLPKKYHVLRFLDKGERHPVREARAVIFFGDQEHPNVTEFAVGPLPGPAYMRALSPRPGYQSSWASRPISTAEYALLYHTLQEATKPLHQFFLNTTGFSFQDCHDRCLAFTDVAPRGVASGQRRSWLIIQRYVEGYFLHPTGLELLVDHGSTDAGHWAVEQVWYNGKFYGSPEELARKYADGEVDVVVLEDPLPGGKGHDSTEEPPLFSSHKPRGDFPSPIHVSGPRLVQPHGPRFRLEGNAVLYGGWSFAFRLRSSSGLQVLNVHFGGERIAYEVSVQEAVALYGGHTPAGMQTKYLDVGWGLGSVTHELAPGIDCPETATFLDTFHYYDADDPVHYPRALCLFEMPTGVPLRRHFNSNFKGGFNFYAGLKGQVLVLRTTSTVYNYDYIWDFIFYPNGVMEAKMHATGYVHATFYTPEGLRHGTRLHTHLIGNIHTHLVHYRVDLDVAGTKNSFQTLQMKLENITNPWSPRHRVVQPTLEQTQYSWERQAAFRFKTKLPKYLLFTSPQENPWGHKRSYRLQIHSMADQVLPPGWQEEQAITWARYPLAVTKYRESELCSSSIYHQNDPWHPPVVFEQFLHNNENIENEDLVAWVTVGFLHIPHSEDIPNTATPGNSVGFLLRPFNFFPEDPSLASRDTVIVWPRDNGPNYVQRWIPEDRDCSMPPPFSYNGTYRPVEPKSADKTHTCPPCPAPPVAGPSVFLFPPKPKDTLMISRTPEVTCVVVDVSHEDPEVKFNWYVDGVEVHNAKTKPREEQYNSTYRVVSVLTVLHQDWLNGKEYKCKVSNKGLPSSIEKTISKAKGQPREPQVYTLPPSREEMTKNQVSLTCLVKGFYPSDIAVEWESNGQPENNYKTTPPVLDSDGSFFLYSKLTVDKSRWQQGNVFSCSVMHEALHNHYTQKSLSLSPGK

SEQ ID NO: 67 - protein, 982 aa, Artificial Sequence
  hDAO-Fc-Hepmut4-Cysmut
MPALGWAVAAILMLQTAMAEPSPGTLPRKAGVFSDLSNQELKAVHSFLWSKKELRLQPSSTTTMAKNTVFLIEMLLPKKYHVLRFLDKGERHPVREARAVIFFGDQEHPNVTEFAVGPLPGPAYMRALSPRPGYQSSWASRPISTAEYALLYHTLQEATKPLHQFFLNTTGFSFQDCHDRCLAFTDVAPRGVASGQRRSWLIIQRYVEGYFLHPTGLELLVDHGSTDAGHWAVEQVWYNGKFYGSPEELARKYADGEVDVVVLEDPLPGGKGHDSTEEPPLFSSHKPRGDFPSPIHVSGPRLVQPHGPRFRLEGNAVLYGGWSFAFRLRSSSGLQVLNVHFGGERIAYEVSVQEAVALYGGHTPAGMQTKYLDVGWGLGSVTHELAPGIDCPETATFLDTFHYYDADDPVHYPRALCLFEMPTGVPLRRHFNSNFKGGFNFYAGLKGQVLVLRTTSTVYNYDYIWDFIFYPNGVMEAKMHATGYVHATFYTPEGLRHGTRLHTHLIGNIHTHLVHYRVDLDVAGTKNSFQTLQMKLENITNPWSPRHRVVQPTLEQTQYSWERQAAFSFKTKLPKYLLFTSPQENPWGHKRSYRLQIHSMADQVLPPGWQEEQAITWARYPLAVTKYRESELCSSSIYHQNDPWHPPVVFEQFLHNNENIENEDLVAWVTVGFLHIPHSEDIPNTATPGNSVGFLLRPFNFFPEDPSLASRDTVIVWPRDNGPNYVQRWIPEDRDCSMPPPFSYNGTYRPVEPKSADKTHTCPPCPAPPVAGPSVFLFPPKPKDTLMISRTPEVTCVVVDVSHEDPEVKFNWYVDGVEVHNAKTKPREEQYNSTYRVVSVLTVLHQDWLNGKEYKCKVSNKGLPSSIEKTISKAKGQPREPQVYTLPPSREEMTKNQVSLTCLVKGFYPSDIAVEWESNGQPENNYKTTPPVLDSDGSFFLYSKLTVDKSRWQQGNVFSCSVMHEALHNHYTQKSLSLSPGK

SEQ ID NO: 68 - protein, 982 aa, Artificial Sequence
  hDAO-Fc-Hepmut5-Cysmut
MPALGWAVAAILMLQTAMAEPSPGTLPRKAGVFSDLSNQELKAVHSFLWSKKELRLQPSSTTTMAKNTVFLIEMLLPKKYHVLRFLDKGERHPVREARAVIFFGDQEHPNVTEFAVGPLPGPAYMRALSPRPGYQSSWASRPISTAEYALLYHTLQEATKPLHQFFLNTTGFSFQDCHDRCLAFTDVAPRGVASGQRRSWLIIQRYVEGYFLHPTGLELLVDHGSTDAGHWAVEQVWYNGKFYGSPEELARKYADGEVDVVVLEDPLPGGKGHDSTEEPPLFSSHKPRGDFPSPIHVSGPRLVQPHGPRFRLEGNAVLYGGWSFAFRLRSSSGLQVLNVHFGGERIAYEVSVQEAVALYGGHTPAGMQTKYLDVGWGLGSVTHELAPGIDCPETATFLDTFHYYDADDPVHYPRALCLFEMPTGVPLRRHFNSNFKGGFNFYAGLKGQVLVLRTTSTVYNYDYIWDFIFYPNGVMEAKMHATGYVHATFYTPEGLRHGTRLHTHLIGNIHTHLVHYRVDLDVAGTKNSFQTLQMKLENITNPWSPRHRVVQPTLEQTQYSWERQAAFRFKTKLPTYLLFTSPQENPWGHKRSYRLQIHSMADQVLPPGWQEEQAITWARYPLAVTKYRESELCSSSIYHQNDPWHPPVVFEQFLHNNENIENEDLVAWVTVGFLHIPHSEDIPNTATPGNSVGFLLRPFNFFPEDPSLASRDTVIVWPRDNGPNYVQRWIPEDRDCSMPPPFSYNGTYRPVEPKSADKTHTCPPCPAPPVAGPSVFLFPPKPKDTLMISRTPEVTCVVVDVSHEDPEVKFNWYVDGVEVHNAKTKPREEQYNSTYRVVSVLTVLHQDWLNGKEYKCKVSNKGLPSSIEKTISKAKGQPREPQVYTLPPSREEMTKNQVSLTCLVKGFYPSDIAVEWESNGQPENNYKTTPPVLDSDGSFFLYSKLTVDKSRWQQGNVFSCSVMHEALHNHYTQKSLSLSPGK

SEQ ID NO: 69 - protein, 982 aa, Artificial Sequence
  hDAO-Fc-Hepmut6-Cysmut
MPALGWAVAAILMLQTAMAEPSPGTLPRKAGVFSDLSNQELKAVHSFLWSKKELRLQPSSTTTMAKNTVFLIEMLLPKKYHVLRFLDKGERHPVREARAVIFFGDQEHPNVTEFAVGPLPGPAYMRALSPRPGYQSSWASRPISTAEYALLYHTLQEATKPLHQFFLNTTGFSFQDCHDRCLAFTDVAPRGVASGQRRSWLIIQRYVEGYFLHPTGLELLVDHGSTDAGHWAVEQVWYNGKFYGSPEELARKYADGEVDVVVLEDPLPGGKGHDSTEEPPLFSSHKPRGDFPSPIHVSGPRLVQPHGPRFRLEGNAVLYGGWSFAFRLRSSSGLQVLNVHFGGERIAYEVSVQEAVALYGGHTPAGMQTKYLDVGWGLGSVTHELAPGIDCPETATFLDTFHYYDADDPVHYPRALCLFEMPTGVPLRRHFNSNFKGGFNFYAGLKGQVLVLRTTSTVYNYDYIWDFIFYPNGVMEAKMHATGYVHATFYTPEGLRHGTRLHTHLIGNIHTHLVHYRVDLDVAGTKNSFQTLQMKLENITNPWSPRHRVVQPTLEQTQYSWERQAAFRFGQTLPKYLLFTSPQENPWGHKRSYRLQIHSMADQVLPPGWQEEQAITWARYPLAVTKYRESELCSSSIYHQNDPWHPPVVFEQFLHNNENIENEDLVAWVTVGFLHIPHSEDIPNTATPGNSVGFLLRPFNFFPEDPSLASRDTVIVWPRDNGPNYVQRWIPEDRDCSMPPPFSYNGTYRPVEPKSADKTHTCPPCPAPPVAGPSVFLFPPKPKDTLMISRTPEVTCVVVDVSHEDPEVKFNWYVDGVEVHNAKTKPREEQYNSTYRVVSVLTVLHQDWLNGKEYKCKVSNKGLPSSIEKTISKAKGQPREPQVYTLPPSREEMTKNQVSLTCLVKGFYPSDIAVEWESNGQPENNYKTTPPVLDSDGSFFLYSKLTVDKSRWQQGNVFSCSVMHEALHNHYTQKSLSLSPGK

SEQ ID NO: 70 - protein, 982 aa, Artificial Sequence
  hDAO-Fc-Hepmut7-Cysmut
MPALGWAVAAILMLQTAMAEPSPGTLPRKAGVFSDLSNQELKAVHSFLWSKKELRLQPSSTTTMAKNTVFLIEMLLPKKYHVLRFLDKGERHPVREARAVIFFGDQEHPNVTEFAVGPLPGPAYMRALSPRPGYQSSWASRPISTAEYALLYHTLQEATKPLHQFFLNTTGFSFQDCHDRCLAFTDVAPRGVASGQRRSWLIIQRYVEGYFLHPTGLELLVDHGSTDAGHWAVEQVWYNGKFYGSPEELARKYADGEVDVVVLEDPLPGGKGHDSTEEPPLFSSHKPRGDFPSPIHVSGPRLVQPHGPRFRLEGNAVLYGGWSFAFRLRSSSGLQVLNVHFGGERIAYEVSVQEAVALYGGHTPAGMQTKYLDVGWGLGSVTHELAPGIDCPETATFLDTFHYYDADDPVHYPRALCLFEMPTGVPLRRHFNSNFKGGFNFYAGLKGQVLVLRTTSTVYNYDYIWDFIFYPNGVMEAKMHATGYVHATFYTPEGLRHGTRLHTHLIGNIHTHLVHYRVDLDVAGTKNSFQTLQMKLENITNPWSPRHRVVQPTLEQTQYSWERQAAFSFKRKLPTYLLFTSPQENPWGHKRSYRLQIHSMADQVLPPGWQEEQAITWARYPLAVTKYRESELCSSSIYHQNDPWHPPVVFEQFLHNNENIENEDLVAWVTVGFLHIPHSEDIPNTATPGNSVGFLLRPFNFFPEDPSLASRDTVIVWPRDNGPNYVQRWIPEDRDCSMPPPFSYNGTYRPVEPKSADKTHTCPPCPAPPVAGPSVFLFPPKPKDTLMISRTPEVTCVVVDVSHEDPEVKFNWYVDGVEVHNAKTKPREEQYNSTYRVVSVLTVLHQDWLNGKEYKCKVSNKGLPSSIEKTISKAKGQPREPQVYTLPPSREEMTKNQVSLTCLVKGFYPSDIAVEWESNGQPENNYKTTPPVLDSDGSFFLYSKLTVDKSRWQQGNVFSCSVMHEALHNHYTQKSLSLSPGK

SEQ ID NO: 71 - DNA, 2952 bp, Artificial Sequence
  Fc-hDAO
atgccggccctgggctgggccgtggctgccatcctgatgctgcagacggccatggcggagtgccccccctgccccgccccccccgtggccggcccctccgtgttcctgttcccccccaagcccaaggacaccctgatgatctccaggacccccgaggtgacctgcgtggtggtggacgtgtcccacgaggaccccgaggtgaagttcaactggtacgtggacggcgtggaggtgcacaacgccaagaccaagcccagggaggagcagtacaactccacctacagggtggtgtccgtgctgaccgtgctgcaccaggactggctgaacggcaaggagtacaagtgcaaggtgtccaacaagggcctgccctcctccatcgagaagaccatctccaaggccaagggccagcccagggagccccaggtgtacaccctgcccccctccagggaggagatgaccaagaaccaggtgtccctgacctgcctggtgaagggcttctacccctccgacatcgccgtggagtgggagtccaacggccagcccgagaacaactacaagaccaccccccccgtgctggactccgacggctccttcttcctgtactccaagctgaccgtggacaagtccaggtggcagcagggcaacgtgttctcctgctccgtgatgcacgaggccctgcacaaccactacacccagaagtccctgtccctgtcccccggcaaggagcccaagtccgccgacaagacccacaccgagccctccccggggactctgcccaggaaggcaggggtgttttcagacctaagcaaccaagagctgaaggcagtgcacagcttcctctggtccaagaaggagctgaggctgcagccctccagtaccaccaccatggccaagaacaccgtgtttctcatcgagatgctgctgcccaagaagtaccatgtgctgaggtttctggataaaggtgaaaggcatcctgtgcgggaagcccgtgccgtcatcttctttggtgaccaggagcatcccaatgtcaccgagtttgctgtggggcccctgccaggcccctgctacatgcgagcactgtcccccaggcctgggtaccagtcctcctgggcatcgaggcccatctccacagcagagtatgccctcctctaccacaccctgcaggaagccaccaagcccctgcatcagttcttcctcaataccacaggcttctcattccaagactgccatgacagatgcctggccttcaccgatgtggccccccggggtgtggcttctggccagcgccgcagttggcttatcatacagcgctatgtagaaggctactttctgcaccccactgggctggagctcctcgtggatcatgggagcacagatgctgggcactgggccgtggagcaggtgtggtacaacgggaagttctatgggagcccagaggaactggctcggaagtatgcagatggagaggtggacgtggtggtcctggaggacccgctgcctgggggcaaggggcatgacagcacagaggagccgcccctcttctcctcccacaagccccgcggggacttccccagccccatccatgtgagcggcccccgcttggtccagccccacggccctcgcttcaggctggagggcaacgctgtgctctacggcggctggagctttgccttccggctgcgctcctcctccgggctgcaggtcctgaacgtgcacttcggcggagagcgcattgcctatgaggtcagcgtgcaagaggcagtggcgctgtatggaggacacacacctgcaggcatgcagaccaagtacctcgatgtcggctggggcctgggcagcgtcactcatgagttagcccccggcatcgactgcccggagaccgccaccttcctggacactttccactactatgatgccgatgacccggtccattatccccgagccctctgcctctttgaaatgcccacaggggtgccccttcggcggcactttaattccaactttaaaggtggcttcaacttctatgcggggctgaagggccaggtgctggtgctgcggacaacttcaactgtctacaattatgattacatttgggactttatcttctaccccaacggggtgatggaggccaagatgcatgccactggctacgtccacgccaccttctacacccccgaggggctgcgccacggcactcgcctgcacacccacctgattggcaacatacacactcacttggtgcactaccgcgtagacctggatgtggcaggcaccaagaacagcttccagacactgcagatgaagctagaaaacatcaccaacccctggagcccaagacaccgcgtggtccagccaactctggagcagacgcagtactcctgggagcgccaggcggccttccgcttcaaaaggaagctgcccaagtacctgctctttaccagcccccaggagaacccctggggccacaagcgcagctaccgcctgcagatccactccatggccgaccaggtgctgcccccaggctggcaggaggagcaggccatcacctgggcaaggtaccccctggcagtgaccaagtaccgggagtcggagctgtgcagcagcagcatctaccaccagaacgacccctggcacccgcccgtggtctttgagcagtttcttcacaacaacgagaacattgaaaatgaggacctggtggcctgggtgacggtgggcttcctgcacatcccccactcagaggacattcccaacacagccacacctgggaactccgtgggcttcctgctccggccattcaacttcttcccagaggacccctccctggcatccagagacactgtgatcgtgtggcctcgggacaacggccccaactacgtccagcgctggatccctgaggacagggactgctcgatgcctcccccttttagctacaatgggacctatagacctgtgtga

SEQ ID NO: 72 - DNA, 2952 bp, Artificial Sequence
  Fc-hDAO-Hepmut1
atgccggccctgggctgggccgtggctgccatcctgatgctgcagacggccatggcggagtgccccccctgccccgccccccccgtggccggcccctccgtgttcctgttcccccccaagcccaaggacaccctgatgatctccaggacccccgaggtgacctgcgtggtggtggacgtgtcccacgaggaccccgaggtgaagttcaactggtacgtggacggcgtggaggtgcacaacgccaagaccaagcccagggaggagcagtacaactccacctacagggtggtgtccgtgctgaccgtgctgcaccaggactggctgaacggcaaggagtacaagtgcaaggtgtccaacaagggcctgccctcctccatcgagaagaccatctccaaggccaagggccagcccagggagccccaggtgtacaccctgcccccctccagggaggagatgaccaagaaccaggtgtccctgacctgcctggtgaagggcttctacccctccgacatcgccgtggagtgggagtccaacggccagcccgagaacaactacaagaccaccccccccgtgctggactccgacggctccttcttcctgtactccaagctgaccgtggacaagtccaggtggcagcagggcaacgtgttctcctgctccgtgatgcacgaggccctgcacaaccactacacccagaagtccctgtccctgtcccccggcaaggagcccaagtccgccgacaagacccacaccgagccctccccggggactctgcccaggaaggcaggggtgttttcagacctaagcaaccaagagctgaaggcagtgcacagcttcctctggtccaagaaggagctgaggctgcagccctccagtaccaccaccatggccaagaacaccgtgtttctcatcgagatgctgctgcccaagaagtaccatgtgctgaggtttctggataaaggtgaaaggcatcctgtgcgggaagcccgtgccgtcatcttctttggtgaccaggagcatcccaatgtcaccgagtttgctgtggggcccctgccaggcccctgctacatgcgagcactgtcccccaggcctgggtaccagtcctcctgggcatcgaggcccatctccacagcagagtatgccctcctctaccacaccctgcaggaagccaccaagcccctgcatcagttcttcctcaataccacaggcttctcattccaagactgccatgacagatgcctggccttcaccgatgtggccccccggggtgtggcttctggccagcgccgcagttggcttatcatacagcgctatgtagaaggctactttctgcaccccactgggctggagctcctcgtggatcatgggagcacagatgctgggcactgggccgtggagcaggtgtggtacaacgggaagttctatgggagcccagaggaactggctcggaagtatgcagatggagaggtggacgtggtggtcctggaggacccgctgcctgggggcaaggggcatgacagcacagaggagccgcccctcttctcctcccacaagccccgcggggacttccccagccccatccatgtgagcggcccccgcttggtccagccccacggccctcgcttcaggctggagggcaacgctgtgctctacggcggctggagctttgccttccggctgcgctcctcctccgggctgcaggtcctgaacgtgcacttcggcggagagcgcattgcctatgaggtcagcgtgcaagaggcagtggcgctgtatggaggacacacacctgcaggcatgcagaccaagtacctcgatgtcggctggggcctgggcagcgtcactcatgagttagcccccggcatcgactgcccggagaccgccaccttcctggacactttccactactatgatgccgatgacccggtccattatccccgagccctctgcctctttgaaatgcccacaggggtgccccttcggcggcactttaattccaactttaaaggtggcttcaacttctatgcggggctgaagggccaggtgctggtgctgcggacaacttcaactgtctacaattatgattacatttgggactttatcttctaccccaacggggtgatggaggccaagatgcatgccactggctacgtccacgccaccttctacacccccgaggggctgcgccacggcactcgcctgcacacccacctgattggcaacatacacactcacttggtgcactaccgcgtagacctggatgtggcaggcaccaagaacagcttccagacactgcagatgaagctagaaaacatcaccaacccctggagcccaagacaccgcgtggtccagccaactctggagcagacgcagtactcctgggagcgccaggcggccttcagcttcaaaaggaagctgcccaagtacctgctctttaccagcccccaggagaacccctggggccacaagcgcagctaccgcctgcagatccactccatggccgaccaggtgctgcccccaggctggcaggaggagcaggccatcacctgggcaaggtaccccctggcagtgaccaagtaccgggagtcggagctgtgcagcagcagcatctaccaccagaacgacccctggcacccgcccgtggtctttgagcagtttcttcacaacaacgagaacattgaaaatgaggacctggtggcctgggtgacggtgggcttcctgcacatcccccactcagaggacattcccaacacagccacacctgggaactccgtgggcttcctgctccggccattcaacttcttcccagaggacccctccctggcatccagagacactgtgatcgtgtggcctcgggacaacggccccaactacgtccagcgctggatccctgaggacagggactgctcgatgcctcccccttttagctacaatgggacctatagacctgtgtga

SEQ ID NO: 73 - DNA, 2952 bp, Artificial Sequence
  Fc-hDAO-Hepmut2
atgccggccctgggctgggccgtggctgccatcctgatgctgcagacggccatggcggagtgccccccctgccccgccccccccgtggccggcccctccgtgttcctgttcccccccaagcccaaggacaccctgatgatctccaggacccccgaggtgacctgcgtggtggtggacgtgtcccacgaggaccccgaggtgaagttcaactggtacgtggacggcgtggaggtgcacaacgccaagaccaagcccagggaggagcagtacaactccacctacagggtggtgtccgtgctgaccgtgctgcaccaggactggctgaacggcaaggagtacaagtgcaaggtgtccaacaagggcctgccctcctccatcgagaagaccatctccaaggccaagggccagcccagggagccccaggtgtacaccctgcccccctccagggaggagatgaccaagaaccaggtgtccctgacctgcctggtgaagggcttctacccctccgacatcgccgtggagtgggagtccaacggccagcccgagaacaactacaagaccaccccccccgtgctggactccgacggctccttcttcctgtactccaagctgaccgtggacaagtccaggtggcagcagggcaacgtgttctcctgctccgtgatgcacgaggccctgcacaaccactacacccagaagtccctgtccctgtcccccggcaaggagcccaagtccgccgacaagacccacaccgagccctccccggggactctgcccaggaaggcaggggtgttttcagacctaagcaaccaagagctgaaggcagtgcacagcttcctctggtccaagaaggagctgaggctgcagccctccagtaccaccaccatggccaagaacaccgtgtttctcatcgagatgctgctgcccaagaagtaccatgtgctgaggtttctggataaaggtgaaaggcatcctgtgcgggaagcccgtgccgtcatcttctttggtgaccaggagcatcccaatgtcaccgagtttgctgtggggcccctgccaggcccctgctacatgcgagcactgtcccccaggcctgggtaccagtcctcctgggcatcgaggcccatctccacagcagagtatgccctcctctaccacaccctgcaggaagccaccaagcccctgcatcagttcttcctcaataccacaggcttctcattccaagactgccatgacagatgcctggccttcaccgatgtggccccccggggtgtggcttctggccagcgccgcagttggcttatcatacagcgctatgtagaaggctactttctgcaccccactgggctggagctcctcgtggatcatgggagcacagatgctgggcactgggccgtggagcaggtgtggtacaacgggaagttctatgggagcccagaggaactggctcggaagtatgcagatggagaggtggacgtggtggtcctggaggacccgctgcctgggggcaaggggcatgacagcacagaggagccgcccctcttctcctcccacaagccccgcggggacttccccagccccatccatgtgagcggcccccgcttggtccagccccacggccctcgcttcaggctggagggcaacgctgtgctctacggcggctggagctttgccttccggctgcgctcctcctccgggctgcaggtcctgaacgtgcacttcggcggagagcgcattgcctatgaggtcagcgtgcaagaggcagtggcgctgtatggaggacacacacctgcaggcatgcagaccaagtacctcgatgtcggctggggcctgggcagcgtcactcatgagttagcccccggcatcgactgcccggagaccgccaccttcctggacactttccactactatgatgccgatgacccggtccattatccccgagccctctgcctctttgaaatgcccacaggggtgccccttcggcggcactttaattccaactttaaaggtggcttcaacttctatgcggggctgaagggccaggtgctggtgctgcggacaacttcaactgtctacaattatgattacatttgggactttatcttctaccccaacggggtgatggaggccaagatgcatgccactggctacgtccacgccaccttctacacccccgaggggctgcgccacggcactcgcctgcacacccacctgattggcaacatacacactcacttggtgcactaccgcgtagacctggatgtggcaggcaccaagaacagcttccagacactgcagatgaagctagaaaacatcaccaacccctggagcccaagacaccgcgtggtccagccaactctggagcagacgcagtactcctgggagcgccaggcggccttccgcttcaaaaggaagctgcccacgtacctgctctttaccagcccccaggagaacccctggggccacaagcgcagctaccgcctgcagatccactccatggccgaccaggtgctgcccccaggctggcaggaggagcaggccatcacctgggcaaggtaccccctggcagtgaccaagtaccgggagtcggagctgtgcagcagcagcatctaccaccagaacgacccctggcacccgcccgtggtctttgagcagtttcttcacaacaacgagaacattgaaaatgaggacctggtggcctgggtgacggtgggcttcctgcacatcccccactcagaggacattcccaacacagccacacctgggaactccgtgggcttcctgctccggccattcaacttcttcccagaggacccctccctggcatccagagacactgtgatcgtgtggcctcgggacaacggccccaactacgtccagcgctggatccctgaggacagggactgctcgatgcctcccccttttagctacaatgggacctatagacctgtgtga

SEQ ID NO: 74 - DNA, 2952 bp, Artificial Sequence
  Fc-hDAO-Hepmut3
atgccggccctgggctgggccgtggctgccatcctgatgctgcagacggccatggcggagtgccccccctgccccgccccccccgtggccggcccctccgtgttcctgttcccccccaagcccaaggacaccctgatgatctccaggacccccgaggtgacctgcgtggtggtggacgtgtcccacgaggaccccgaggtgaagttcaactggtacgtggacggcgtggaggtgcacaacgccaagaccaagcccagggaggagcagtacaactccacctacagggtggtgtccgtgctgaccgtgctgcaccaggactggctgaacggcaaggagtacaagtgcaaggtgtccaacaagggcctgccctcctccatcgagaagaccatctccaaggccaagggccagcccagggagccccaggtgtacaccctgcccccctccagggaggagatgaccaagaaccaggtgtccctgacctgcctggtgaagggcttctacccctccgacatcgccgtggagtgggagtccaacggccagcccgagaacaactacaagaccaccccccccgtgctggactccgacggctccttcttcctgtactccaagctgaccgtggacaagtccaggtggcagcagggcaacgtgttctcctgctccgtgatgcacgaggccctgcacaaccactacacccagaagtccctgtccctgtcccccggcaaggagcccaagtccgccgacaagacccacaccgagccctccccggggactctgcccaggaaggcaggggtgttttcagacctaagcaaccaagagctgaaggcagtgcacagcttcctctggtccaagaaggagctgaggctgcagccctccagtaccaccaccatggccaagaacaccgtgtttctcatcgagatgctgctgcccaagaagtaccatgtgctgaggtttctggataaaggtgaaaggcatcctgtgcgggaagcccgtgccgtcatcttctttggtgaccaggagcatcccaatgtcaccgagtttgctgtggggcccctgccaggcccctgctacatgcgagcactgtcccccaggcctgggtaccagtcctcctgggcatcgaggcccatctccacagcagagtatgccctcctctaccacaccctgcaggaagccaccaagcccctgcatcagttcttcctcaataccacaggcttctcattccaagactgccatgacagatgcctggccttcaccgatgtggccccccggggtgtggcttctggccagcgccgcagttggcttatcatacagcgctatgtagaaggctactttctgcaccccactgggctggagctcctcgtggatcatgggagcacagatgctgggcactgggccgtggagcaggtgtggtacaacgggaagttctatgggagcccagaggaactggctcggaagtatgcagatggagaggtggacgtggtggtcctggaggacccgctgcctgggggcaaggggcatgacagcacagaggagccgcccctcttctcctcccacaagccccgcggggacttccccagccccatccatgtgagcggcccccgcttggtccagccccacggccctcgcttcaggctggagggcaacgctgtgctctacggcggctggagctttgccttccggctgcgctcctcctccgggctgcaggtcctgaacgtgcacttcggcggagagcgcattgcctatgaggtcagcgtgcaagaggcagtggcgctgtatggaggacacacacctgcaggcatgcagaccaagtacctcgatgtcggctggggcctgggcagcgtcactcatgagttagcccccggcatcgactgcccggagaccgccaccttcctggacactttccactactatgatgccgatgacccggtccattatccccgagccctctgcctctttgaaatgcccacaggggtgccccttcggcggcactttaattccaactttaaaggtggcttcaacttctatgcggggctgaagggccaggtgctggtgctgcggacaacttcaactgtctacaattatgattacatttgggactttatcttctaccccaacggggtgatggaggccaagatgcatgccactggctacgtccacgccaccttctacacccccgaggggctgcgccacggcactcgcctgcacacccacctgattggcaacatacacactcacttggtgcactaccgcgtagacctggatgtggcaggcaccaagaacagcttccagacactgcagatgaagctagaaaacatcaccaacccctggagcccaagacaccgcgtggtccagccaactctggagcagacgcagtactcctgggagcgccaggcggccttccgcttcaaaacgaagctgcccaagtacctgctctttaccagcccccaggagaacccctggggccacaagcgcagctaccgcctgcagatccactccatggccgaccaggtgctgcccccaggctggcaggaggagcaggccatcacctgggcaaggtaccccctggcagtgaccaagtaccgggagtcggagctgtgcagcagcagcatctaccaccagaacgacccctggcacccgcccgtggtctttgagcagtttcttcacaacaacgagaacattgaaaatgaggacctggtggcctgggtgacggtgggcttcctgcacatcccccactcagaggacattcccaacacagccacacctgggaactccgtgggcttcctgctccggccattcaacttcttcccagaggacccctccctggcatccagagacactgtgatcgtgtggcctcgggacaacggccccaactacgtccagcgctggatccctgaggacagggactgctcgatgcctcccccttttagctacaatgggacctatagacctgtgtga

SEQ ID NO: 75 - DNA, 2952 bp, Artificial Sequence
  Fc-hDAO-Hepmut4
atgccggccctgggctgggccgtggctgccatcctgatgctgcagacggccatggcggagtgccccccctgccccgccccccccgtggccggcccctccgtgttcctgttcccccccaagcccaaggacaccctgatgatctccaggacccccgaggtgacctgcgtggtggtggacgtgtcccacgaggaccccgaggtgaagttcaactggtacgtggacggcgtggaggtgcacaacgccaagaccaagcccagggaggagcagtacaactccacctacagggtggtgtccgtgctgaccgtgctgcaccaggactggctgaacggcaaggagtacaagtgcaaggtgtccaacaagggcctgccctcctccatcgagaagaccatctccaaggccaagggccagcccagggagccccaggtgtacaccctgcccccctccagggaggagatgaccaagaaccaggtgtccctgacctgcctggtgaagggcttctacccctccgacatcgccgtggagtgggagtccaacggccagcccgagaacaactacaagaccaccccccccgtgctggactccgacggctccttcttcctgtactccaagctgaccgtggacaagtccaggtggcagcagggcaacgtgttctcctgctccgtgatgcacgaggccctgcacaaccactacacccagaagtccctgtccctgtcccccggcaaggagcccaagtccgccgacaagacccacaccgagccctccccggggactctgcccaggaaggcaggggtgttttcagacctaagcaaccaagagctgaaggcagtgcacagcttcctctggtccaagaaggagctgaggctgcagccctccagtaccaccaccatggccaagaacaccgtgtttctcatcgagatgctgctgcccaagaagtaccatgtgctgaggtttctggataaaggtgaaaggcatcctgtgcgggaagcccgtgccgtcatcttctttggtgaccaggagcatcccaatgtcaccgagtttgctgtggggcccctgccaggcccctgctacatgcgagcactgtcccccaggcctgggtaccagtcctcctgggcatcgaggcccatctccacagcagagtatgccctcctctaccacaccctgcaggaagccaccaagcccctgcatcagttcttcctcaataccacaggcttctcattccaagactgccatgacagatgcctggccttcaccgatgtggccccccggggtgtggcttctggccagcgccgcagttggcttatcatacagcgctatgtagaaggctactttctgcaccccactgggctggagctcctcgtggatcatgggagcacagatgctgggcactgggccgtggagcaggtgtggtacaacgggaagttctatgggagcccagaggaactggctcggaagtatgcagatggagaggtggacgtggtggtcctggaggacccgctgcctgggggcaaggggcatgacagcacagaggagccgcccctcttctcctcccacaagccccgcggggacttccccagccccatccatgtgagcggcccccgcttggtccagccccacggccctcgcttcaggctggagggcaacgctgtgctctacggcggctggagctttgccttccggctgcgctcctcctccgggctgcaggtcctgaacgtgcacttcggcggagagcgcattgcctatgaggtcagcgtgcaagaggcagtggcgctgtatggaggacacacacctgcaggcatgcagaccaagtacctcgatgtcggctggggcctgggcagcgtcactcatgagttagcccccggcatcgactgcccggagaccgccaccttcctggacactttccactactatgatgccgatgacccggtccattatccccgagccctctgcctctttgaaatgcccacaggggtgccccttcggcggcactttaattccaactttaaaggtggcttcaacttctatgcggggctgaagggccaggtgctggtgctgcggacaacttcaactgtctacaattatgattacatttgggactttatcttctaccccaacggggtgatggaggccaagatgcatgccactggctacgtccacgccaccttctacacccccgaggggctgcgccacggcactcgcctgcacacccacctgattggcaacatacacactcacttggtgcactaccgcgtagacctggatgtggcaggcaccaagaacagcttccagacactgcagatgaagctagaaaacatcaccaacccctggagcccaagacaccgcgtggtccagccaactctggagcagacgcagtactcctgggagcgccaggcggccttcagcttcaaaacgaagctgcccaagtacctgctctttaccagcccccaggagaacccctggggccacaagcgcagctaccgcctgcagatccactccatggccgaccaggtgctgcccccaggctggcaggaggagcaggccatcacctgggcaaggtaccccctggcagtgaccaagtaccgggagtcggagctgtgcagcagcagcatctaccaccagaacgacccctggcacccgcccgtggtctttgagcagtttcttcacaacaacgagaacattgaaaatgaggacctggtggcctgggtgacggtgggcttcctgcacatcccccactcagaggacattcccaacacagccacacctgggaactccgtgggcttcctgctccggccattcaacttcttcccagaggacccctccctggcatccagagacactgtgatcgtgtggcctcgggacaacggccccaactacgtccagcgctggatccctgaggacagggactgctcgatgcctcccccttttagctacaatgggacctatagacctgtgtga

SEQ ID NO: 76 - DNA, 2952 bp, Artificial Sequence
  Fc-hDAO-Hepmut5
atgccggccctgggctgggccgtggctgccatcctgatgctgcagacggccatggcggagtgccccccctgccccgccccccccgtggccggcccctccgtgttcctgttcccccccaagcccaaggacaccctgatgatctccaggacccccgaggtgacctgcgtggtggtggacgtgtcccacgaggaccccgaggtgaagttcaactggtacgtggacggcgtggaggtgcacaacgccaagaccaagcccagggaggagcagtacaactccacctacagggtggtgtccgtgctgaccgtgctgcaccaggactggctgaacggcaaggagtacaagtgcaaggtgtccaacaagggcctgccctcctccatcgagaagaccatctccaaggccaagggccagcccagggagccccaggtgtacaccctgcccccctccagggaggagatgaccaagaaccaggtgtccctgacctgcctggtgaagggcttctacccctccgacatcgccgtggagtgggagtccaacggccagcccgagaacaactacaagaccaccccccccgtgctggactccgacggctccttcttcctgtactccaagctgaccgtggacaagtccaggtggcagcagggcaacgtgttctcctgctccgtgatgcacgaggccctgcacaaccactacacccagaagtccctgtccctgtcccccggcaaggagcccaagtccgccgacaagacccacaccgagccctccccggggactctgcccaggaaggcaggggtgttttcagacctaagcaaccaagagctgaaggcagtgcacagcttcctctggtccaagaaggagctgaggctgcagccctccagtaccaccaccatggccaagaacaccgtgtttctcatcgagatgctgctgcccaagaagtaccatgtgctgaggtttctggataaaggtgaaaggcatcctgtgcgggaagcccgtgccgtcatcttctttggtgaccaggagcatcccaatgtcaccgagtttgctgtggggcccctgccaggcccctgctacatgcgagcactgtcccccaggcctgggtaccagtcctcctgggcatcgaggcccatctccacagcagagtatgccctcctctaccacaccctgcaggaagccaccaagcccctgcatcagttcttcctcaataccacaggcttctcattccaagactgccatgacagatgcctggccttcaccgatgtggccccccggggtgtggcttctggccagcgccgcagttggcttatcatacagcgctatgtagaaggctactttctgcaccccactgggctggagctcctcgtggatcatgggagcacagatgctgggcactgggccgtggagcaggtgtggtacaacgggaagttctatgggagcccagaggaactggctcggaagtatgcagatggagaggtggacgtggtggtcctggaggacccgctgcctgggggcaaggggcatgacagcacagaggagccgcccctcttctcctcccacaagccccgcggggacttccccagccccatccatgtgagcggcccccgcttggtccagccccacggccctcgcttcaggctggagggcaacgctgtgctctacggcggctggagctttgccttccggctgcgctcctcctccgggctgcaggtcctgaacgtgcacttcggcggagagcgcattgcctatgaggtcagcgtgcaagaggcagtggcgctgtatggaggacacacacctgcaggcatgcagaccaagtacctcgatgtcggctggggcctgggcagcgtcactcatgagttagcccccggcatcgactgcccggagaccgccaccttcctggacactttccactactatgatgccgatgacccggtccattatccccgagccctctgcctctttgaaatgcccacaggggtgccccttcggcggcactttaattccaactttaaaggtggcttcaacttctatgcggggctgaagggccaggtgctggtgctgcggacaacttcaactgtctacaattatgattacatttgggactttatcttctaccccaacggggtgatggaggccaagatgcatgccactggctacgtccacgccaccttctacacccccgaggggctgcgccacggcactcgcctgcacacccacctgattggcaacatacacactcacttggtgcactaccgcgtagacctggatgtggcaggcaccaagaacagcttccagacactgcagatgaagctagaaaacatcaccaacccctggagcccaagacaccgcgtggtccagccaactctggagcagacgcagtactcctgggagcgccaggcggccttccgcttcaaaacgaagctgcccacgtacctgctctttaccagcccccaggagaacccctggggccacaagcgcagctaccgcctgcagatccactccatggccgaccaggtgctgcccccaggctggcaggaggagcaggccatcacctgggcaaggtaccccctggcagtgaccaagtaccgggagtcggagctgtgcagcagcagcatctaccaccagaacgacccctggcacccgcccgtggtctttgagcagtttcttcacaacaacgagaacattgaaaatgaggacctggtggcctgggtgacggtgggcttcctgcacatcccccactcagaggacattcccaacacagccacacctgggaactccgtgggcttcctgctccggccattcaacttcttcccagaggacccctccctggcatccagagacactgtgatcgtgtggcctcgggacaacggccccaactacgtccagcgctggatccctgaggacagggactgctcgatgcctcccccttttagctacaatgggacctatagacctgtgtga

SEQ ID NO: 77 - DNA, 2952 bp, Artificial Sequence
  Fc-hDAO-Hepmut6
atgccggccctgggctgggccgtggctgccatcctgatgctgcagacggccatggcggagtgccccccctgccccgccccccccgtggccggcccctccgtgttcctgttcccccccaagcccaaggacaccctgatgatctccaggacccccgaggtgacctgcgtggtggtggacgtgtcccacgaggaccccgaggtgaagttcaactggtacgtggacggcgtggaggtgcacaacgccaagaccaagcccagggaggagcagtacaactccacctacagggtggtgtccgtgctgaccgtgctgcaccaggactggctgaacggcaaggagtacaagtgcaaggtgtccaacaagggcctgccctcctccatcgagaagaccatctccaaggccaagggccagcccagggagccccaggtgtacaccctgcccccctccagggaggagatgaccaagaaccaggtgtccctgacctgcctggtgaagggcttctacccctccgacatcgccgtggagtgggagtccaacggccagcccgagaacaactacaagaccaccccccccgtgctggactccgacggctccttcttcctgtactccaagctgaccgtggacaagtccaggtggcagcagggcaacgtgttctcctgctccgtgatgcacgaggccctgcacaaccactacacccagaagtccctgtccctgtcccccggcaaggagcccaagtccgccgacaagacccacaccgagccctccccggggactctgcccaggaaggcaggggtgttttcagacctaagcaaccaagagctgaaggcagtgcacagcttcctctggtccaagaaggagctgaggctgcagccctccagtaccaccaccatggccaagaacaccgtgtttctcatcgagatgctgctgcccaagaagtaccatgtgctgaggtttctggataaaggtgaaaggcatcctgtgcgggaagcccgtgccgtcatcttctttggtgaccaggagcatcccaatgtcaccgagtttgctgtggggcccctgccaggcccctgctacatgcgagcactgtcccccaggcctgggtaccagtcctcctgggcatcgaggcccatctccacagcagagtatgccctcctctaccacaccctgcaggaagccaccaagcccctgcatcagttcttcctcaataccacaggcttctcattccaagactgccatgacagatgcctggccttcaccgatgtggccccccggggtgtggcttctggccagcgccgcagttggcttatcatacagcgctatgtagaaggctactttctgcaccccactgggctggagctcctcgtggatcatgggagcacagatgctgggcactgggccgtggagcaggtgtggtacaacgggaagttctatgggagcccagaggaactggctcggaagtatgcagatggagaggtggacgtggtggtcctggaggacccgctgcctgggggcaaggggcatgacagcacagaggagccgcccctcttctcctcccacaagccccgcggggacttccccagccccatccatgtgagcggcccccgcttggtccagccccacggccctcgcttcaggctggagggcaacgctgtgctctacggcggctggagctttgccttccggctgcgctcctcctccgggctgcaggtcctgaacgtgcacttcggcggagagcgcattgcctatgaggtcagcgtgcaagaggcagtggcgctgtatggaggacacacacctgcaggcatgcagaccaagtacctcgatgtcggctggggcctgggcagcgtcactcatgagttagcccccggcatcgactgcccggagaccgccaccttcctggacactttccactactatgatgccgatgacccggtccattatccccgagccctctgcctctttgaaatgcccacaggggtgccccttcggcggcactttaattccaactttaaaggtggcttcaacttctatgcggggctgaagggccaggtgctggtgctgcggacaacttcaactgtctacaattatgattacatttgggactttatcttctaccccaacggggtgatggaggccaagatgcatgccactggctacgtccacgccaccttctacacccccgaggggctgcgccacggcactcgcctgcacacccacctgattggcaacatacacactcacttggtgcactaccgcgtagacctggatgtggcaggcaccaagaacagcttccagacactgcagatgaagctagaaaacatcaccaacccctggagcccaagacaccgcgtggtccagccaactctggagcagacgcagtactcctgggagcgccaggcggccttccgcttcggacagacgctgcccaagtacctgctctttaccagcccccaggagaacccctggggccacaagcgcagctaccgcctgcagatccactccatggccgaccaggtgctgcccccaggctggcaggaggagcaggccatcacctgggcaaggtaccccctggcagtgaccaagtaccgggagtcggagctgtgcagcagcagcatctaccaccagaacgacccctggcacccgcccgtggtctttgagcagtttcttcacaacaacgagaacattgaaaatgaggacctggtggcctgggtgacggtgggcttcctgcacatcccccactcagaggacattcccaacacagccacacctgggaactccgtgggcttcctgctccggccattcaacttcttcccagaggacccctccctggcatccagagacactgtgatcgtgtggcctcgggacaacggccccaactacgtccagcgctggatccctgaggacagggactgctcgatgcctcccccttttagctacaatgggacctatagacctgtgtga

SEQ ID NO: 78 - DNA, 2952 bp, Artificial Sequence
  Fc-hDAO-Hepmut7
atgccggccctgggctgggccgtggctgccatcctgatgctgcagacggccatggcggagtgccccccctgccccgccccccccgtggccggcccctccgtgttcctgttcccccccaagcccaaggacaccctgatgatctccaggacccccgaggtgacctgcgtggtggtggacgtgtcccacgaggaccccgaggtgaagttcaactggtacgtggacggcgtggaggtgcacaacgccaagaccaagcccagggaggagcagtacaactccacctacagggtggtgtccgtgctgaccgtgctgcaccaggactggctgaacggcaaggagtacaagtgcaaggtgtccaacaagggcctgccctcctccatcgagaagaccatctccaaggccaagggccagcccagggagccccaggtgtacaccctgcccccctccagggaggagatgaccaagaaccaggtgtccctgacctgcctggtgaagggcttctacccctccgacatcgccgtggagtgggagtccaacggccagcccgagaacaactacaagaccaccccccccgtgctggactccgacggctccttcttcctgtactccaagctgaccgtggacaagtccaggtggcagcagggcaacgtgttctcctgctccgtgatgcacgaggccctgcacaaccactacacccagaagtccctgtccctgtcccccggcaaggagcccaagtccgccgacaagacccacaccgagccctccccggggactctgcccaggaaggcaggggtgttttcagacctaagcaaccaagagctgaaggcagtgcacagcttcctctggtccaagaaggagctgaggctgcagccctccagtaccaccaccatggccaagaacaccgtgtttctcatcgagatgctgctgcccaagaagtaccatgtgctgaggtttctggataaaggtgaaaggcatcctgtgcgggaagcccgtgccgtcatcttctttggtgaccaggagcatcccaatgtcaccgagtttgctgtggggcccctgccaggcccctgctacatgcgagcactgtcccccaggcctgggtaccagtcctcctgggcatcgaggcccatctccacagcagagtatgccctcctctaccacaccctgcaggaagccaccaagcccctgcatcagttcttcctcaataccacaggcttctcattccaagactgccatgacagatgcctggccttcaccgatgtggccccccggggtgtggcttctggccagcgccgcagttggcttatcatacagcgctatgtagaaggctactttctgcaccccactgggctggagctcctcgtggatcatgggagcacagatgctgggcactgggccgtggagcaggtgtggtacaacgggaagttctatgggagcccagaggaactggctcggaagtatgcagatggagaggtggacgtggtggtcctggaggacccgctgcctgggggcaaggggcatgacagcacagaggagccgcccctcttctcctcccacaagccccgcggggacttccccagccccatccatgtgagcggcccccgcttggtccagccccacggccctcgcttcaggctggagggcaacgctgtgctctacggcggctggagctttgccttccggctgcgctcctcctccgggctgcaggtcctgaacgtgcacttcggcggagagcgcattgcctatgaggtcagcgtgcaagaggcagtggcgctgtatggaggacacacacctgcaggcatgcagaccaagtacctcgatgtcggctggggcctgggcagcgtcactcatgagttagcccccggcatcgactgcccggagaccgccaccttcctggacactttccactactatgatgccgatgacccggtccattatccccgagccctctgcctctttgaaatgcccacaggggtgccccttcggcggcactttaattccaactttaaaggtggcttcaacttctatgcggggctgaagggccaggtgctggtgctgcggacaacttcaactgtctacaattatgattacatttgggactttatcttctaccccaacggggtgatggaggccaagatgcatgccactggctacgtccacgccaccttctacacccccgaggggctgcgccacggcactcgcctgcacacccacctgattggcaacatacacactcacttggtgcactaccgcgtagacctggatgtggcaggcaccaagaacagcttccagacactgcagatgaagctagaaaacatcaccaacccctggagcccaagacaccgcgtggtccagccaactctggagcagacgcagtactcctgggagcgccaggcggccttcagcttcaaaaggaagctgcccacgtacctgctctttaccagcccccaggagaacccctggggccacaagcgcagctaccgcctgcagatccactccatggccgaccaggtgctgcccccaggctggcaggaggagcaggccatcacctgggcaaggtaccccctggcagtgaccaagtaccgggagtcggagctgtgcagcagcagcatctaccaccagaacgacccctggcacccgcccgtggtctttgagcagtttcttcacaacaacgagaacattgaaaatgaggacctggtggcctgggtgacggtgggcttcctgcacatcccccactcagaggacattcccaacacagccacacctgggaactccgtgggcttcctgctccggccattcaacttcttcccagaggacccctccctggcatccagagacactgtgatcgtgtggcctcgggacaacggccccaactacgtccagcgctggatccctgaggacagggactgctcgatgcctcccccttttagctacaatgggacctatagacctgtgtga

SEQ ID NO: 79 - DNA, 2952 bp, Artificial Sequence
  Fc-hDAO-Cysmut
atgccggccctgggctgggccgtggctgccatcctgatgctgcagacggccatggcggagtgccccccctgccccgccccccccgtggccggcccctccgtgttcctgttcccccccaagcccaaggacaccctgatgatctccaggacccccgaggtgacctgcgtggtggtggacgtgtcccacgaggaccccgaggtgaagttcaactggtacgtggacggcgtggaggtgcacaacgccaagaccaagcccagggaggagcagtacaactccacctacagggtggtgtccgtgctgaccgtgctgcaccaggactggctgaacggcaaggagtacaagtgcaaggtgtccaacaagggcctgccctcctccatcgagaagaccatctccaaggccaagggccagcccagggagccccaggtgtacaccctgcccccctccagggaggagatgaccaagaaccaggtgtccctgacctgcctggtgaagggcttctacccctccgacatcgccgtggagtgggagtccaacggccagcccgagaacaactacaagaccaccccccccgtgctggactccgacggctccttcttcctgtactccaagctgaccgtggacaagtccaggtggcagcagggcaacgtgttctcctgctccgtgatgcacgaggccctgcacaaccactacacccagaagtccctgtccctgtcccccggcaaggagcccaagtccgccgacaagacccacaccgagccctccccggggactctgcccaggaaggcaggggtgttttcagacctaagcaaccaagagctgaaggcagtgcacagcttcctctggtccaagaaggagctgaggctgcagccctccagtaccaccaccatggccaagaacaccgtgtttctcatcgagatgctgctgcccaagaagtaccatgtgctgaggtttctggataaaggtgaaaggcatcctgtgcgggaagcccgtgccgtcatcttctttggtgaccaggagcatcccaatgtcaccgagtttgctgtggggcccctgccaggccccgcctacatgcgagcactgtcccccaggcctgggtaccagtcctcctgggcatcgaggcccatctccacagcagagtatgccctcctctaccacaccctgcaggaagccaccaagcccctgcatcagttcttcctcaataccacaggcttctcattccaagactgccatgacagatgcctggccttcaccgatgtggccccccggggtgtggcttctggccagcgccgcagttggcttatcatacagcgctatgtagaaggctactttctgcaccccactgggctggagctcctcgtggatcatgggagcacagatgctgggcactgggccgtggagcaggtgtggtacaacgggaagttctatgggagcccagaggaactggctcggaagtatgcagatggagaggtggacgtggtggtcctggaggacccgctgcctgggggcaaggggcatgacagcacagaggagccgcccctcttctcctcccacaagccccgcggggacttccccagccccatccatgtgagcggcccccgcttggtccagccccacggccctcgcttcaggctggagggcaacgctgtgctctacggcggctggagctttgccttccggctgcgctcctcctccgggctgcaggtcctgaacgtgcacttcggcggagagcgcattgcctatgaggtcagcgtgcaagaggcagtggcgctgtatggaggacacacacctgcaggcatgcagaccaagtacctcgatgtcggctggggcctgggcagcgtcactcatgagttagcccccggcatcgactgcccggagaccgccaccttcctggacactttccactactatgatgccgatgacccggtccattatccccgagccctctgcctctttgaaatgcccacaggggtgccccttcggcggcactttaattccaactttaaaggtggcttcaacttctatgcggggctgaagggccaggtgctggtgctgcggacaacttcaactgtctacaattatgattacatttgggactttatcttctaccccaacggggtgatggaggccaagatgcatgccactggctacgtccacgccaccttctacacccccgaggggctgcgccacggcactcgcctgcacacccacctgattggcaacatacacactcacttggtgcactaccgcgtagacctggatgtggcaggcaccaagaacagcttccagacactgcagatgaagctagaaaacatcaccaacccctggagcccaagacaccgcgtggtccagccaactctggagcagacgcagtactcctgggagcgccaggcggccttccgcttcaaaaggaagctgcccaagtacctgctctttaccagcccccaggagaacccctggggccacaagcgcagctaccgcctgcagatccactccatggccgaccaggtgctgcccccaggctggcaggaggagcaggccatcacctgggcaaggtaccccctggcagtgaccaagtaccgggagtcggagctgtgcagcagcagcatctaccaccagaacgacccctggcacccgcccgtggtctttgagcagtttcttcacaacaacgagaacattgaaaatgaggacctggtggcctgggtgacggtgggcttcctgcacatcccccactcagaggacattcccaacacagccacacctgggaactccgtgggcttcctgctccggccattcaacttcttcccagaggacccctccctggcatccagagacactgtgatcgtgtggcctcgggacaacggccccaactacgtccagcgctggatccctgaggacagggactgctcgatgcctcccccttttagctacaatgggacctatagacctgtgtga

SEQ ID NO: 80 - DNA, 2952 bp, Artificial Sequence
  Fc-hDAO-Hepmut1-Cysmut
atgccggccctgggctgggccgtggctgccatcctgatgctgcagacggccatggcggagtgccccccctgccccgccccccccgtggccggcccctccgtgttcctgttcccccccaagcccaaggacaccctgatgatctccaggacccccgaggtgacctgcgtggtggtggacgtgtcccacgaggaccccgaggtgaagttcaactggtacgtggacggcgtggaggtgcacaacgccaagaccaagcccagggaggagcagtacaactccacctacagggtggtgtccgtgctgaccgtgctgcaccaggactggctgaacggcaaggagtacaagtgcaaggtgtccaacaagggcctgccctcctccatcgagaagaccatctccaaggccaagggccagcccagggagccccaggtgtacaccctgcccccctccagggaggagatgaccaagaaccaggtgtccctgacctgcctggtgaagggcttctacccctccgacatcgccgtggagtgggagtccaacggccagcccgagaacaactacaagaccaccccccccgtgctggactccgacggctccttcttcctgtactccaagctgaccgtggacaagtccaggtggcagcagggcaacgtgttctcctgctccgtgatgcacgaggccctgcacaaccactacacccagaagtccctgtccctgtcccccggcaaggagcccaagtccgccgacaagacccacaccgagccctccccggggactctgcccaggaaggcaggggtgttttcagacctaagcaaccaagagctgaaggcagtgcacagcttcctctggtccaagaaggagctgaggctgcagccctccagtaccaccaccatggccaagaacaccgtgtttctcatcgagatgctgctgcccaagaagtaccatgtgctgaggtttctggataaaggtgaaaggcatcctgtgcgggaagcccgtgccgtcatcttctttggtgaccaggagcatcccaatgtcaccgagtttgctgtggggcccctgccaggccccgcctacatgcgagcactgtcccccaggcctgggtaccagtcctcctgggcatcgaggcccatctccacagcagagtatgccctcctctaccacaccctgcaggaagccaccaagcccctgcatcagttcttcctcaataccacaggcttctcattccaagactgccatgacagatgcctggccttcaccgatgtggccccccggggtgtggcttctggccagcgccgcagttggcttatcatacagcgctatgtagaaggctactttctgcaccccactgggctggagctcctcgtggatcatgggagcacagatgctgggcactgggccgtggagcaggtgtggtacaacgggaagttctatgggagcccagaggaactggctcggaagtatgcagatggagaggtggacgtggtggtcctggaggacccgctgcctgggggcaaggggcatgacagcacagaggagccgcccctcttctcctcccacaagccccgcggggacttccccagccccatccatgtgagcggcccccgcttggtccagccccacggccctcgcttcaggctggagggcaacgctgtgctctacggcggctggagctttgccttccggctgcgctcctcctccgggctgcaggtcctgaacgtgcacttcggcggagagcgcattgcctatgaggtcagcgtgcaagaggcagtggcgctgtatggaggacacacacctgcaggcatgcagaccaagtacctcgatgtcggctggggcctgggcagcgtcactcatgagttagcccccggcatcgactgcccggagaccgccaccttcctggacactttccactactatgatgccgatgacccggtccattatccccgagccctctgcctctttgaaatgcccacaggggtgccccttcggcggcactttaattccaactttaaaggtggcttcaacttctatgcggggctgaagggccaggtgctggtgctgcggacaacttcaactgtctacaattatgattacatttgggactttatcttctaccccaacggggtgatggaggccaagatgcatgccactggctacgtccacgccaccttctacacccccgaggggctgcgccacggcactcgcctgcacacccacctgattggcaacatacacactcacttggtgcactaccgcgtagacctggatgtggcaggcaccaagaacagcttccagacactgcagatgaagctagaaaacatcaccaacccctggagcccaagacaccgcgtggtccagccaactctggagcagacgcagtactcctgggagcgccaggcggccttcagcttcaaaaggaagctgcccaagtacctgctctttaccagcccccaggagaacccctggggccacaagcgcagctaccgcctgcagatccactccatggccgaccaggtgctgcccccaggctggcaggaggagcaggccatcacctgggcaaggtaccccctggcagtgaccaagtaccgggagtcggagctgtgcagcagcagcatctaccaccagaacgacccctggcacccgcccgtggtctttgagcagtttcttcacaacaacgagaacattgaaaatgaggacctggtggcctgggtgacggtgggcttcctgcacatcccccactcagaggacattcccaacacagccacacctgggaactccgtgggcttcctgctccggccattcaacttcttcccagaggacccctccctggcatccagagacactgtgatcgtgtggcctcgggacaacggccccaactacgtccagcgctggatccctgaggacagggactgctcgatgcctcccccttttagctacaatgggacctatagacctgtgtga

SEQ ID NO: 81 - DNA, 2952 bp, Artificial Sequence
  Fc-hDAO-Hepmut2-Cysmut
atgccggccctgggctgggccgtggctgccatcctgatgctgcagacggccatggcggagtgccccccctgccccgccccccccgtggccggcccctccgtgttcctgttcccccccaagcccaaggacaccctgatgatctccaggacccccgaggtgacctgcgtggtggtggacgtgtcccacgaggaccccgaggtgaagttcaactggtacgtggacggcgtggaggtgcacaacgccaagaccaagcccagggaggagcagtacaactccacctacagggtggtgtccgtgctgaccgtgctgcaccaggactggctgaacggcaaggagtacaagtgcaaggtgtccaacaagggcctgccctcctccatcgagaagaccatctccaaggccaagggccagcccagggagccccaggtgtacaccctgcccccctccagggaggagatgaccaagaaccaggtgtccctgacctgcctggtgaagggcttctacccctccgacatcgccgtggagtgggagtccaacggccagcccgagaacaactacaagaccaccccccccgtgctggactccgacggctccttcttcctgtactccaagctgaccgtggacaagtccaggtggcagcagggcaacgtgttctcctgctccgtgatgcacgaggccctgcacaaccactacacccagaagtccctgtccctgtcccccggcaaggagcccaagtccgccgacaagacccacaccgagccctccccggggactctgcccaggaaggcaggggtgttttcagacctaagcaaccaagagctgaaggcagtgcacagcttcctctggtccaagaaggagctgaggctgcagccctccagtaccaccaccatggccaagaacaccgtgtttctcatcgagatgctgctgcccaagaagtaccatgtgctgaggtttctggataaaggtgaaaggcatcctgtgcgggaagcccgtgccgtcatcttctttggtgaccaggagcatcccaatgtcaccgagtttgctgtggggcccctgccaggccccgcctacatgcgagcactgtcccccaggcctgggtaccagtcctcctgggcatcgaggcccatctccacagcagagtatgccctcctctaccacaccctgcaggaagccaccaagcccctgcatcagttcttcctcaataccacaggcttctcattccaagactgccatgacagatgcctggccttcaccgatgtggccccccggggtgtggcttctggccagcgccgcagttggcttatcatacagcgctatgtagaaggctactttctgcaccccactgggctggagctcctcgtggatcatgggagcacagatgctgggcactgggccgtggagcaggtgtggtacaacgggaagttctatgggagcccagaggaactggctcggaagtatgcagatggagaggtggacgtggtggtcctggaggacccgctgcctgggggcaaggggcatgacagcacagaggagccgcccctcttctcctcccacaagccccgcggggacttccccagccccatccatgtgagcggcccccgcttggtccagccccacggccctcgcttcaggctggagggcaacgctgtgctctacggcggctggagctttgccttccggctgcgctcctcctccgggctgcaggtcctgaacgtgcacttcggcggagagcgcattgcctatgaggtcagcgtgcaagaggcagtggcgctgtatggaggacacacacctgcaggcatgcagaccaagtacctcgatgtcggctggggcctgggcagcgtcactcatgagttagcccccggcatcgactgcccggagaccgccaccttcctggacactttccactactatgatgccgatgacccggtccattatccccgagccctctgcctctttgaaatgcccacaggggtgccccttcggcggcactttaattccaactttaaaggtggcttcaacttctatgcggggctgaagggccaggtgctggtgctgcggacaacttcaactgtctacaattatgattacatttgggactttatcttctaccccaacggggtgatggaggccaagatgcatgccactggctacgtccacgccaccttctacacccccgaggggctgcgccacggcactcgcctgcacacccacctgattggcaacatacacactcacttggtgcactaccgcgtagacctggatgtggcaggcaccaagaacagcttccagacactgcagatgaagctagaaaacatcaccaacccctggagcccaagacaccgcgtggtccagccaactctggagcagacgcagtactcctgggagcgccaggcggccttccgcttcaaaaggaagctgcccacgtacctgctctttaccagcccccaggagaacccctggggccacaagcgcagctaccgcctgcagatccactccatggccgaccaggtgctgcccccaggctggcaggaggagcaggccatcacctgggcaaggtaccccctggcagtgaccaagtaccgggagtcggagctgtgcagcagcagcatctaccaccagaacgacccctggcacccgcccgtggtctttgagcagtttcttcacaacaacgagaacattgaaaatgaggacctggtggcctgggtgacggtgggcttcctgcacatcccccactcagaggacattcccaacacagccacacctgggaactccgtgggcttcctgctccggccattcaacttcttcccagaggacccctccctggcatccagagacactgtgatcgtgtggcctcgggacaacggccccaactacgtccagcgctggatccctgaggacagggactgctcgatgcctcccccttttagctacaatgggacctatagacctgtgtga

SEQ ID NO: 82 - DNA, 2952 bp, Artificial Sequence
  Fc-hDAO-Hepmut3-Cysmut
atgccggccctgggctgggccgtggctgccatcctgatgctgcagacggccatggcggagtgccccccctgccccgccccccccgtggccggcccctccgtgttcctgttcccccccaagcccaaggacaccctgatgatctccaggacccccgaggtgacctgcgtggtggtggacgtgtcccacgaggaccccgaggtgaagttcaactggtacgtggacggcgtggaggtgcacaacgccaagaccaagcccagggaggagcagtacaactccacctacagggtggtgtccgtgctgaccgtgctgcaccaggactggctgaacggcaaggagtacaagtgcaaggtgtccaacaagggcctgccctcctccatcgagaagaccatctccaaggccaagggccagcccagggagccccaggtgtacaccctgcccccctccagggaggagatgaccaagaaccaggtgtccctgacctgcctggtgaagggcttctacccctccgacatcgccgtggagtgggagtccaacggccagcccgagaacaactacaagaccaccccccccgtgctggactccgacggctccttcttcctgtactccaagctgaccgtggacaagtccaggtggcagcagggcaacgtgttctcctgctccgtgatgcacgaggccctgcacaaccactacacccagaagtccctgtccctgtcccccggcaaggagcccaagtccgccgacaagacccacaccgagccctccccggggactctgcccaggaaggcaggggtgttttcagacctaagcaaccaagagctgaaggcagtgcacagcttcctctggtccaagaaggagctgaggctgcagccctccagtaccaccaccatggccaagaacaccgtgtttctcatcgagatgctgctgcccaagaagtaccatgtgctgaggtttctggataaaggtgaaaggcatcctgtgcgggaagcccgtgccgtcatcttctttggtgaccaggagcatcccaatgtcaccgagtttgctgtggggcccctgccaggccccgcctacatgcgagcactgtcccccaggcctgggtaccagtcctcctgggcatcgaggcccatctccacagcagagtatgccctcctctaccacaccctgcaggaagccaccaagcccctgcatcagttcttcctcaataccacaggcttctcattccaagactgccatgacagatgcctggccttcaccgatgtggccccccggggtgtggcttctggccagcgccgcagttggcttatcatacagcgctatgtagaaggctactttctgcaccccactgggctggagctcctcgtggatcatgggagcacagatgctgggcactgggccgtggagcaggtgtggtacaacgggaagttctatgggagcccagaggaactggctcggaagtatgcagatggagaggtggacgtggtggtcctggaggacccgctgcctgggggcaaggggcatgacagcacagaggagccgcccctcttctcctcccacaagccccgcggggacttccccagccccatccatgtgagcggcccccgcttggtccagccccacggccctcgcttcaggctggagggcaacgctgtgctctacggcggctggagctttgccttccggctgcgctcctcctccgggctgcaggtcctgaacgtgcacttcggcggagagcgcattgcctatgaggtcagcgtgcaagaggcagtggcgctgtatggaggacacacacctgcaggcatgcagaccaagtacctcgatgtcggctggggcctgggcagcgtcactcatgagttagcccccggcatcgactgcccggagaccgccaccttcctggacactttccactactatgatgccgatgacccggtccattatccccgagccctctgcctctttgaaatgcccacaggggtgccccttcggcggcactttaattccaactttaaaggtggcttcaacttctatgcggggctgaagggccaggtgctggtgctgcggacaacttcaactgtctacaattatgattacatttgggactttatcttctaccccaacggggtgatggaggccaagatgcatgccactggctacgtccacgccaccttctacacccccgaggggctgcgccacggcactcgcctgcacacccacctgattggcaacatacacactcacttggtgcactaccgcgtagacctggatgtggcaggcaccaagaacagcttccagacactgcagatgaagctagaaaacatcaccaacccctggagcccaagacaccgcgtggtccagccaactctggagcagacgcagtactcctgggagcgccaggcggccttccgcttcaaaacgaagctgcccaagtacctgctctttaccagcccccaggagaacccctggggccacaagcgcagctaccgcctgcagatccactccatggccgaccaggtgctgcccccaggctggcaggaggagcaggccatcacctgggcaaggtaccccctggcagtgaccaagtaccgggagtcggagctgtgcagcagcagcatctaccaccagaacgacccctggcacccgcccgtggtctttgagcagtttcttcacaacaacgagaacattgaaaatgaggacctggtggcctgggtgacggtgggcttcctgcacatcccccactcagaggacattcccaacacagccacacctgggaactccgtgggcttcctgctccggccattcaacttcttcccagaggacccctccctggcatccagagacactgtgatcgtgtggcctcgggacaacggccccaactacgtccagcgctggatccctgaggacagggactgctcgatgcctcccccttttagctacaatgggacctatagacctgtgtga

SEQ ID NO: 83 - DNA, 2952 bp, Artificial Sequence
  Fc-hDAO-Hepmut4-Cysmut
atgccggccctgggctgggccgtggctgccatcctgatgctgcagacggccatggcggagtgccccccctgccccgccccccccgtggccggcccctccgtgttcctgttcccccccaagcccaaggacaccctgatgatctccaggacccccgaggtgacctgcgtggtggtggacgtgtcccacgaggaccccgaggtgaagttcaactggtacgtggacggcgtggaggtgcacaacgccaagaccaagcccagggaggagcagtacaactccacctacagggtggtgtccgtgctgaccgtgctgcaccaggactggctgaacggcaaggagtacaagtgcaaggtgtccaacaagggcctgccctcctccatcgagaagaccatctccaaggccaagggccagcccagggagccccaggtgtacaccctgcccccctccagggaggagatgaccaagaaccaggtgtccctgacctgcctggtgaagggcttctacccctccgacatcgccgtggagtgggagtccaacggccagcccgagaacaactacaagaccaccccccccgtgctggactccgacggctccttcttcctgtactccaagctgaccgtggacaagtccaggtggcagcagggcaacgtgttctcctgctccgtgatgcacgaggccctgcacaaccactacacccagaagtccctgtccctgtcccccggcaaggagcccaagtccgccgacaagacccacaccgagccctccccggggactctgcccaggaaggcaggggtgttttcagacctaagcaaccaagagctgaaggcagtgcacagcttcctctggtccaagaaggagctgaggctgcagccctccagtaccaccaccatggccaagaacaccgtgtttctcatcgagatgctgctgcccaagaagtaccatgtgctgaggtttctggataaaggtgaaaggcatcctgtgcgggaagcccgtgccgtcatcttctttggtgaccaggagcatcccaatgtcaccgagtttgctgtggggcccctgccaggccccgcctacatgcgagcactgtcccccaggcctgggtaccagtcctcctgggcatcgaggcccatctccacagcagagtatgccctcctctaccacaccctgcaggaagccaccaagcccctgcatcagttcttcctcaataccacaggcttctcattccaagactgccatgacagatgcctggccttcaccgatgtggccccccggggtgtggcttctggccagcgccgcagttggcttatcatacagcgctatgtagaaggctactttctgcaccccactgggctggagctcctcgtggatcatgggagcacagatgctgggcactgggccgtggagcaggtgtggtacaacgggaagttctatgggagcccagaggaactggctcggaagtatgcagatggagaggtggacgtggtggtcctggaggacccgctgcctgggggcaaggggcatgacagcacagaggagccgcccctcttctcctcccacaagccccgcggggacttccccagccccatccatgtgagcggcccccgcttggtccagccccacggccctcgcttcaggctggagggcaacgctgtgctctacggcggctggagctttgccttccggctgcgctcctcctccgggctgcaggtcctgaacgtgcacttcggcggagagcgcattgcctatgaggtcagcgtgcaagaggcagtggcgctgtatggaggacacacacctgcaggcatgcagaccaagtacctcgatgtcggctggggcctgggcagcgtcactcatgagttagcccccggcatcgactgcccggagaccgccaccttcctggacactttccactactatgatgccgatgacccggtccattatccccgagccctctgcctctttgaaatgcccacaggggtgccccttcggcggcactttaattccaactttaaaggtggcttcaacttctatgcggggctgaagggccaggtgctggtgctgcggacaacttcaactgtctacaattatgattacatttgggactttatcttctaccccaacggggtgatggaggccaagatgcatgccactggctacgtccacgccaccttctacacccccgaggggctgcgccacggcactcgcctgcacacccacctgattggcaacatacacactcacttggtgcactaccgcgtagacctggatgtggcaggcaccaagaacagcttccagacactgcagatgaagctagaaaacatcaccaacccctggagcccaagacaccgcgtggtccagccaactctggagcagacgcagtactcctgggagcgccaggcggccttcagcttcaaaacgaagctgcccaagtacctgctctttaccagcccccaggagaacccctggggccacaagcgcagctaccgcctgcagatccactccatggccgaccaggtgctgcccccaggctggcaggaggagcaggccatcacctgggcaaggtaccccctggcagtgaccaagtaccgggagtcggagctgtgcagcagcagcatctaccaccagaacgacccctggcacccgcccgtggtctttgagcagtttcttcacaacaacgagaacattgaaaatgaggacctggtggcctgggtgacggtgggcttcctgcacatcccccactcagaggacattcccaacacagccacacctgggaactccgtgggcttcctgctccggccattcaacttcttcccagaggacccctccctggcatccagagacactgtgatcgtgtggcctcgggacaacggccccaactacgtccagcgctggatccctgaggacagggactgctcgatgcctcccccttttagctacaatgggacctatagacctgtgtga

SEQ ID NO: 84 - DNA, 2952 bp, Artificial Sequence
  Fc-hDAO-Hepmut5-Cysmut
atgccggccctgggctgggccgtggctgccatcctgatgctgcagacggccatggcggagtgccccccctgccccgccccccccgtggccggcccctccgtgttcctgttcccccccaagcccaaggacaccctgatgatctccaggacccccgaggtgacctgcgtggtggtggacgtgtcccacgaggaccccgaggtgaagttcaactggtacgtggacggcgtggaggtgcacaacgccaagaccaagcccagggaggagcagtacaactccacctacagggtggtgtccgtgctgaccgtgctgcaccaggactggctgaacggcaaggagtacaagtgcaaggtgtccaacaagggcctgccctcctccatcgagaagaccatctccaaggccaagggccagcccagggagccccaggtgtacaccctgcccccctccagggaggagatgaccaagaaccaggtgtccctgacctgcctggtgaagggcttctacccctccgacatcgccgtggagtgggagtccaacggccagcccgagaacaactacaagaccaccccccccgtgctggactccgacggctccttcttcctgtactccaagctgaccgtggacaagtccaggtggcagcagggcaacgtgttctcctgctccgtgatgcacgaggccctgcacaaccactacacccagaagtccctgtccctgtcccccggcaaggagcccaagtccgccgacaagacccacaccgagccctccccggggactctgcccaggaaggcaggggtgttttcagacctaagcaaccaagagctgaaggcagtgcacagcttcctctggtccaagaaggagctgaggctgcagccctccagtaccaccaccatggccaagaacaccgtgtttctcatcgagatgctgctgcccaagaagtaccatgtgctgaggtttctggataaaggtgaaaggcatcctgtgcgggaagcccgtgccgtcatcttctttggtgaccaggagcatcccaatgtcaccgagtttgctgtggggcccctgccaggccccgcctacatgcgagcactgtcccccaggcctgggtaccagtcctcctgggcatcgaggcccatctccacagcagagtatgccctcctctaccacaccctgcaggaagccaccaagcccctgcatcagttcttcctcaataccacaggcttctcattccaagactgccatgacagatgcctggccttcaccgatgtggccccccggggtgtggcttctggccagcgccgcagttggcttatcatacagcgctatgtagaaggctactttctgcaccccactgggctggagctcctcgtggatcatgggagcacagatgctgggcactgggccgtggagcaggtgtggtacaacgggaagttctatgggagcccagaggaactggctcggaagtatgcagatggagaggtggacgtggtggtcctggaggacccgctgcctgggggcaaggggcatgacagcacagaggagccgcccctcttctcctcccacaagccccgcggggacttccccagccccatccatgtgagcggcccccgcttggtccagccccacggccctcgcttcaggctggagggcaacgctgtgctctacggcggctggagctttgccttccggctgcgctcctcctccgggctgcaggtcctgaacgtgcacttcggcggagagcgcattgcctatgaggtcagcgtgcaagaggcagtggcgctgtatggaggacacacacctgcaggcatgcagaccaagtacctcgatgtcggctggggcctgggcagcgtcactcatgagttagcccccggcatcgactgcccggagaccgccaccttcctggacactttccactactatgatgccgatgacccggtccattatccccgagccctctgcctctttgaaatgcccacaggggtgccccttcggcggcactttaattccaactttaaaggtggcttcaacttctatgcggggctgaagggccaggtgctggtgctgcggacaacttcaactgtctacaattatgattacatttgggactttatcttctaccccaacggggtgatggaggccaagatgcatgccactggctacgtccacgccaccttctacacccccgaggggctgcgccacggcactcgcctgcacacccacctgattggcaacatacacactcacttggtgcactaccgcgtagacctggatgtggcaggcaccaagaacagcttccagacactgcagatgaagctagaaaacatcaccaacccctggagcccaagacaccgcgtggtccagccaactctggagcagacgcagtactcctgggagcgccaggcggccttccgcttcaaaacgaagctgcccacgtacctgctctttaccagcccccaggagaacccctggggccacaagcgcagctaccgcctgcagatccactccatggccgaccaggtgctgcccccaggctggcaggaggagcaggccatcacctgggcaaggtaccccctggcagtgaccaagtaccgggagtcggagctgtgcagcagcagcatctaccaccagaacgacccctggcacccgcccgtggtctttgagcagtttcttcacaacaacgagaacattgaaaatgaggacctggtggcctgggtgacggtgggcttcctgcacatcccccactcagaggacattcccaacacagccacacctgggaactccgtgggcttcctgctccggccattcaacttcttcccagaggacccctccctggcatccagagacactgtgatcgtgtggcctcgggacaacggccccaactacgtccagcgctggatccctgaggacagggactgctcgatgcctcccccttttagctacaatgggacctatagacctgtgtga

SEQ ID NO: 85 - DNA, 2952 bp, Artificial Sequence
  Fc-hDAO-Hepmut6-Cysmut
atgccggccctgggctgggccgtggctgccatcctgatgctgcagacggccatggcggagtgccccccctgccccgccccccccgtggccggcccctccgtgttcctgttcccccccaagcccaaggacaccctgatgatctccaggacccccgaggtgacctgcgtggtggtggacgtgtcccacgaggaccccgaggtgaagttcaactggtacgtggacggcgtggaggtgcacaacgccaagaccaagcccagggaggagcagtacaactccacctacagggtggtgtccgtgctgaccgtgctgcaccaggactggctgaacggcaaggagtacaagtgcaaggtgtccaacaagggcctgccctcctccatcgagaagaccatctccaaggccaagggccagcccagggagccccaggtgtacaccctgcccccctccagggaggagatgaccaagaaccaggtgtccctgacctgcctggtgaagggcttctacccctccgacatcgccgtggagtgggagtccaacggccagcccgagaacaactacaagaccaccccccccgtgctggactccgacggctccttcttcctgtactccaagctgaccgtggacaagtccaggtggcagcagggcaacgtgttctcctgctccgtgatgcacgaggccctgcacaaccactacacccagaagtccctgtccctgtcccccggcaaggagcccaagtccgccgacaagacccacaccgagccctccccggggactctgcccaggaaggcaggggtgttttcagacctaagcaaccaagagctgaaggcagtgcacagcttcctctggtccaagaaggagctgaggctgcagccctccagtaccaccaccatggccaagaacaccgtgtttctcatcgagatgctgctgcccaagaagtaccatgtgctgaggtttctggataaaggtgaaaggcatcctgtgcgggaagcccgtgccgtcatcttctttggtgaccaggagcatcccaatgtcaccgagtttgctgtggggcccctgccaggccccgcctacatgcgagcactgtcccccaggcctgggtaccagtcctcctgggcatcgaggcccatctccacagcagagtatgccctcctctaccacaccctgcaggaagccaccaagcccctgcatcagttcttcctcaataccacaggcttctcattccaagactgccatgacagatgcctggccttcaccgatgtggccccccggggtgtggcttctggccagcgccgcagttggcttatcatacagcgctatgtagaaggctactttctgcaccccactgggctggagctcctcgtggatcatgggagcacagatgctgggcactgggccgtggagcaggtgtggtacaacgggaagttctatgggagcccagaggaactggctcggaagtatgcagatggagaggtggacgtggtggtcctggaggacccgctgcctgggggcaaggggcatgacagcacagaggagccgcccctcttctcctcccacaagccccgcggggacttccccagccccatccatgtgagcggcccccgcttggtccagccccacggccctcgcttcaggctggagggcaacgctgtgctctacggcggctggagctttgccttccggctgcgctcctcctccgggctgcaggtcctgaacgtgcacttcggcggagagcgcattgcctatgaggtcagcgtgcaagaggcagtggcgctgtatggaggacacacacctgcaggcatgcagaccaagtacctcgatgtcggctggggcctgggcagcgtcactcatgagttagcccccggcatcgactgcccggagaccgccaccttcctggacactttccactactatgatgccgatgacccggtccattatccccgagccctctgcctctttgaaatgcccacaggggtgccccttcggcggcactttaattccaactttaaaggtggcttcaacttctatgcggggctgaagggccaggtgctggtgctgcggacaacttcaactgtctacaattatgattacatttgggactttatcttctaccccaacggggtgatggaggccaagatgcatgccactggctacgtccacgccaccttctacacccccgaggggctgcgccacggcactcgcctgcacacccacctgattggcaacatacacactcacttggtgcactaccgcgtagacctggatgtggcaggcaccaagaacagcttccagacactgcagatgaagctagaaaacatcaccaacccctggagcccaagacaccgcgtggtccagccaactctggagcagacgcagtactcctgggagcgccaggcggccttccgcttcggacagacgctgcccaagtacctgctctttaccagcccccaggagaacccctggggccacaagcgcagctaccgcctgcagatccactccatggccgaccaggtgctgcccccaggctggcaggaggagcaggccatcacctgggcaaggtaccccctggcagtgaccaagtaccgggagtcggagctgtgcagcagcagcatctaccaccagaacgacccctggcacccgcccgtggtctttgagcagtttcttcacaacaacgagaacattgaaaatgaggacctggtggcctgggtgacggtgggcttcctgcacatcccccactcagaggacattcccaacacagccacacctgggaactccgtgggcttcctgctccggccattcaacttcttcccagaggacccctccctggcatccagagacactgtgatcgtgtggcctcgggacaacggccccaactacgtccagcgctggatccctgaggacagggactgctcgatgcctcccccttttagctacaatgggacctatagacctgtgtga

SEQ ID NO: 86 - DNA, 2952 bp, Artificial Sequence
  Fc-hDAO-Hepmut7-Cysmut
atgccggccctgggctgggccgtggctgccatcctgatgctgcagacggccatggcggagtgccccccctgccccgccccccccgtggccggcccctccgtgttcctgttcccccccaagcccaaggacaccctgatgatctccaggacccccgaggtgacctgcgtggtggtggacgtgtcccacgaggaccccgaggtgaagttcaactggtacgtggacggcgtggaggtgcacaacgccaagaccaagcccagggaggagcagtacaactccacctacagggtggtgtccgtgctgaccgtgctgcaccaggactggctgaacggcaaggagtacaagtgcaaggtgtccaacaagggcctgccctcctccatcgagaagaccatctccaaggccaagggccagcccagggagccccaggtgtacaccctgcccccctccagggaggagatgaccaagaaccaggtgtccctgacctgcctggtgaagggcttctacccctccgacatcgccgtggagtgggagtccaacggccagcccgagaacaactacaagaccaccccccccgtgctggactccgacggctccttcttcctgtactccaagctgaccgtggacaagtccaggtggcagcagggcaacgtgttctcctgctccgtgatgcacgaggccctgcacaaccactacacccagaagtccctgtccctgtcccccggcaaggagcccaagtccgccgacaagacccacaccgagccctccccggggactctgcccaggaaggcaggggtgttttcagacctaagcaaccaagagctgaaggcagtgcacagcttcctctggtccaagaaggagctgaggctgcagccctccagtaccaccaccatggccaagaacaccgtgtttctcatcgagatgctgctgcccaagaagtaccatgtgctgaggtttctggataaaggtgaaaggcatcctgtgcgggaagcccgtgccgtcatcttctttggtgaccaggagcatcccaatgtcaccgagtttgctgtggggcccctgccaggccccgcctacatgcgagcactgtcccccaggcctgggtaccagtcctcctgggcatcgaggcccatctccacagcagagtatgccctcctctaccacaccctgcaggaagccaccaagcccctgcatcagttcttcctcaataccacaggcttctcattccaagactgccatgacagatgcctggccttcaccgatgtggccccccggggtgtggcttctggccagcgccgcagttggcttatcatacagcgctatgtagaaggctactttctgcaccccactgggctggagctcctcgtggatcatgggagcacagatgctgggcactgggccgtggagcaggtgtggtacaacgggaagttctatgggagcccagaggaactggctcggaagtatgcagatggagaggtggacgtggtggtcctggaggacccgctgcctgggggcaaggggcatgacagcacagaggagccgcccctcttctcctcccacaagccccgcggggacttccccagccccatccatgtgagcggcccccgcttggtccagccccacggccctcgcttcaggctggagggcaacgctgtgctctacggcggctggagctttgccttccggctgcgctcctcctccgggctgcaggtcctgaacgtgcacttcggcggagagcgcattgcctatgaggtcagcgtgcaagaggcagtggcgctgtatggaggacacacacctgcaggcatgcagaccaagtacctcgatgtcggctggggcctgggcagcgtcactcatgagttagcccccggcatcgactgcccggagaccgccaccttcctggacactttccactactatgatgccgatgacccggtccattatccccgagccctctgcctctttgaaatgcccacaggggtgccccttcggcggcactttaattccaactttaaaggtggcttcaacttctatgcggggctgaagggccaggtgctggtgctgcggacaacttcaactgtctacaattatgattacatttgggactttatcttctaccccaacggggtgatggaggccaagatgcatgccactggctacgtccacgccaccttctacacccccgaggggctgcgccacggcactcgcctgcacacccacctgattggcaacatacacactcacttggtgcactaccgcgtagacctggatgtggcaggcaccaagaacagcttccagacactgcagatgaagctagaaaacatcaccaacccctggagcccaagacaccgcgtggtccagccaactctggagcagacgcagtactcctgggagcgccaggcggccttcagcttcaaaaggaagctgcccacgtacctgctctttaccagcccccaggagaacccctggggccacaagcgcagctaccgcctgcagatccactccatggccgaccaggtgctgcccccaggctggcaggaggagcaggccatcacctgggcaaggtaccccctggcagtgaccaagtaccgggagtcggagctgtgcagcagcagcatctaccaccagaacgacccctggcacccgcccgtggtctttgagcagtttcttcacaacaacgagaacattgaaaatgaggacctggtggcctgggtgacggtgggcttcctgcacatcccccactcagaggacattcccaacacagccacacctgggaactccgtgggcttcctgctccggccattcaacttcttcccagaggacccctccctggcatccagagacactgtgatcgtgtggcctcgggacaacggccccaactacgtccagcgctggatccctgaggacagggactgctcgatgcctcccccttttagctacaatgggacctatagacctgtgtga

SEQ ID NO: 87 - DNA, 2949 bp, Artificial Sequence
  hDAO-Fc
atgccggccctgggctgggccgtggctgccatcctgatgctgcagacggccatggcggagccctccccggggactctgcccaggaaggcaggggtgttttcagacctaagcaaccaagagctgaaggcagtgcacagcttcctctggtccaagaaggagctgaggctgcagccctccagtaccaccaccatggccaagaacaccgtgtttctcatcgagatgctgctgcccaagaagtaccatgtgctgaggtttctggataaaggtgaaaggcatcctgtgcgggaagcccgtgccgtcatcttctttggtgaccaggagcatcccaatgtcaccgagtttgctgtggggcccctgccagggccctgctacatgcgagcactgtcccccaggcctgggtaccagtcctcctgggcatcgaggcccatctccacagcagagtatgccctcctctaccacaccctgcaggaagccaccaagcccctgcatcagttcttcctcaataccacaggcttctcattccaagactgccatgacagatgcctggccttcaccgatgtggccccccggggtgtggcttctggccagcgccgcagttggcttatcatacagcgctatgtagaaggctactttctgcaccccactgggctggagctcctcgtggatcatgggagcacagatgctgggcactgggccgtggagcaggtgtggtacaacgggaagttctatgggagcccagaggaactggctcggaagtatgcagatggagaggtggacgtggtggtcctggaggacccgctgcctgggggcaaggggcatgacagcacagaggagccgcccctcttctcctcccacaagccccgcggggacttccccagccccatccatgtgagcggcccccgcttggtccagccccacggccctcgcttcaggctggagggcaacgctgtgctctacggcggctggagctttgccttccggctgcgctcctcctccgggctgcaggtcctgaacgtgcacttcggcggagagcgcattgcctatgaggtcagcgtgcaagaggcagtggcgctgtatggaggacacacacctgcaggcatgcagaccaagtacctcgatgtcggctggggcctgggcagcgtcactcatgagttagcccccggcatcgactgcccggagaccgccaccttcctggacactttccactactatgatgccgatgacccggtccattatccccgagccctctgcctctttgaaatgcccacaggggtgccccttcggcggcactttaattccaactttaaaggtggcttcaacttctatgcggggctgaagggccaggtgctggtgctgcggacaacttcaactgtctacaattatgattacatttgggactttatcttctaccccaacggggtgatggaggccaagatgcatgccactggctacgtccacgccaccttctacacccccgaggggctgcgccacggcactcgcctgcacacccacctgattggcaacatacacactcacttggtgcactaccgcgtagacctggatgtggcaggcaccaagaacagcttccagacactgcagatgaagctagaaaacatcaccaacccctggagcccaagacaccgcgtggtccagccaactctggagcagacgcagtactcctgggagcgccaggcggccttccgcttcaaaaggaagctgcccaagtacctgctctttaccagcccccaggagaacccctggggccacaagcgcagctaccgcctgcagatccactccatggccgaccaggtgctgcccccaggctggcaggaggagcaggccatcacctgggcaaggtaccccctggcagtgaccaagtaccgggagtcggagctgtgcagcagcagcatctaccaccagaacgacccctggcacccgcccgtggtctttgagcagtttcttcacaacaacgagaacattgaaaatgaggacctggtggcctgggtgacggtgggcttcctgcacatcccccactcagaggacattcccaacacagccacacctgggaactccgtgggcttcctgctccggccattcaacttcttcccagaggacccctccctggcatccagagacactgtgatcgtgtggcctcgggacaacggccccaactacgtccagcgctggatccctgaggacagggactgctcgatgcctcccccttttagctacaatgggacctatagacctgtggagcccaagtccgccgacaagacccacacctgccccccctgccccgccccccccgtggccggcccctccgtgttcctgttcccccccaagcccaaggacaccctgatgatctccaggacccccgaggtgacctgcgtggtggtggacgtgtcccacgaggaccccgaggtgaagttcaactggtacgtggacggcgtggaggtgcacaacgccaagaccaagcccagggaggagcagtacaactccacctacagggtggtgtccgtgctgaccgtgctgcaccaggactggctgaacggcaaggagtacaagtgcaaggtgtccaacaagggcctgccctcctccatcgagaagaccatctccaaggccaagggccagcccagggagccccaggtgtacaccctgcccccctccagggaggagatgaccaagaaccaggtgtccctgacctgcctggtgaagggcttctacccctccgacatcgccgtggagtgggagtccaacggccagcccgagaacaactacaagaccaccccccccgtgctggactccgacggctccttcttcctgtactccaagctgaccgtggacaagtccaggtggcagcagggcaacgtgttctcctgctccgtgatgcacgaggccctgcacaaccactacacccagaagtccctgtccctgtcccccggcaagtga

SEQ ID NO: 88 - DNA, 2949 bp, Artificial Sequence
  hDAO-Fc-Hepmut1
atgccggccctgggctgggccgtggctgccatcctgatgctgcagacggccatggcggagccctccccggggactctgcccaggaaggcaggggtgttttcagacctaagcaaccaagagctgaaggcagtgcacagcttcctctggtccaagaaggagctgaggctgcagccctccagtaccaccaccatggccaagaacaccgtgtttctcatcgagatgctgctgcccaagaagtaccatgtgctgaggtttctggataaaggtgaaaggcatcctgtgcgggaagcccgtgccgtcatcttctttggtgaccaggagcatcccaatgtcaccgagtttgctgtggggcccctgccagggccctgctacatgcgagcactgtcccccaggcctgggtaccagtcctcctgggcatcgaggcccatctccacagcagagtatgccctcctctaccacaccctgcaggaagccaccaagcccctgcatcagttcttcctcaataccacaggcttctcattccaagactgccatgacagatgcctggccttcaccgatgtggccccccggggtgtggcttctggccagcgccgcagttggcttatcatacagcgctatgtagaaggctactttctgcaccccactgggctggagctcctcgtggatcatgggagcacagatgctgggcactgggccgtggagcaggtgtggtacaacgggaagttctatgggagcccagaggaactggctcggaagtatgcagatggagaggtggacgtggtggtcctggaggacccgctgcctgggggcaaggggcatgacagcacagaggagccgcccctcttctcctcccacaagccccgcggggacttccccagccccatccatgtgagcggcccccgcttggtccagccccacggccctcgcttcaggctggagggcaacgctgtgctctacggcggctggagctttgccttccggctgcgctcctcctccgggctgcaggtcctgaacgtgcacttcggcggagagcgcattgcctatgaggtcagcgtgcaagaggcagtggcgctgtatggaggacacacacctgcaggcatgcagaccaagtacctcgatgtcggctggggcctgggcagcgtcactcatgagttagcccccggcatcgactgcccggagaccgccaccttcctggacactttccactactatgatgccgatgacccggtccattatccccgagccctctgcctctttgaaatgcccacaggggtgccccttcggcggcactttaattccaactttaaaggtggcttcaacttctatgcggggctgaagggccaggtgctggtgctgcggacaacttcaactgtctacaattatgattacatttgggactttatcttctaccccaacggggtgatggaggccaagatgcatgccactggctacgtccacgccaccttctacacccccgaggggctgcgccacggcactcgcctgcacacccacctgattggcaacatacacactcacttggtgcactaccgcgtagacctggatgtggcaggcaccaagaacagcttccagacactgcagatgaagctagaaaacatcaccaacccctggagcccaagacaccgcgtggtccagccaactctggagcagacgcagtactcctgggagcgccaggcggccttcagcttcaaaaggaagctgcccaagtacctgctctttaccagcccccaggagaacccctggggccacaagcgcagctaccgcctgcagatccactccatggccgaccaggtgctgcccccaggctggcaggaggagcaggccatcacctgggcaaggtaccccctggcagtgaccaagtaccgggagtcggagctgtgcagcagcagcatctaccaccagaacgacccctggcacccgcccgtggtctttgagcagtttcttcacaacaacgagaacattgaaaatgaggacctggtggcctgggtgacggtgggcttcctgcacatcccccactcagaggacattcccaacacagccacacctgggaactccgtgggcttcctgctccggccattcaacttcttcccagaggacccctccctggcatccagagacactgtgatcgtgtggcctcgggacaacggccccaactacgtccagcgctggatccctgaggacagggactgctcgatgcctcccccttttagctacaatgggacctatagacctgtggagcccaagtccgccgacaagacccacacctgccccccctgccccgccccccccgtggccggcccctccgtgttcctgttcccccccaagcccaaggacaccctgatgatctccaggacccccgaggtgacctgcgtggtggtggacgtgtcccacgaggaccccgaggtgaagttcaactggtacgtggacggcgtggaggtgcacaacgccaagaccaagcccagggaggagcagtacaactccacctacagggtggtgtccgtgctgaccgtgctgcaccaggactggctgaacggcaaggagtacaagtgcaaggtgtccaacaagggcctgccctcctccatcgagaagaccatctccaaggccaagggccagcccagggagccccaggtgtacaccctgcccccctccagggaggagatgaccaagaaccaggtgtccctgacctgcctggtgaagggcttctacccctccgacatcgccgtggagtgggagtccaacggccagcccgagaacaactacaagaccaccccccccgtgctggactccgacggctccttcttcctgtactccaagctgaccgtggacaagtccaggtggcagcagggcaacgtgttctcctgctccgtgatgcacgaggccctgcacaaccactacacccagaagtccctgtccctgtcccccggcaagtga

SEQ ID NO: 89 - DNA, 2949 bp, Artificial Sequence
  hDAO-Fc-Hepmut2
atgccggccctgggctgggccgtggctgccatcctgatgctgcagacggccatggcggagccctccccggggactctgcccaggaaggcaggggtgttttcagacctaagcaaccaagagctgaaggcagtgcacagcttcctctggtccaagaaggagctgaggctgcagccctccagtaccaccaccatggccaagaacaccgtgtttctcatcgagatgctgctgcccaagaagtaccatgtgctgaggtttctggataaaggtgaaaggcatcctgtgcgggaagcccgtgccgtcatcttctttggtgaccaggagcatcccaatgtcaccgagtttgctgtggggcccctgccagggccctgctacatgcgagcactgtcccccaggcctgggtaccagtcctcctgggcatcgaggcccatctccacagcagagtatgccctcctctaccacaccctgcaggaagccaccaagcccctgcatcagttcttcctcaataccacaggcttctcattccaagactgccatgacagatgcctggccttcaccgatgtggccccccggggtgtggcttctggccagcgccgcagttggcttatcatacagcgctatgtagaaggctactttctgcaccccactgggctggagctcctcgtggatcatgggagcacagatgctgggcactgggccgtggagcaggtgtggtacaacgggaagttctatgggagcccagaggaactggctcggaagtatgcagatggagaggtggacgtggtggtcctggaggacccgctgcctgggggcaaggggcatgacagcacagaggagccgcccctcttctcctcccacaagccccgcggggacttccccagccccatccatgtgagcggcccccgcttggtccagccccacggccctcgcttcaggctggagggcaacgctgtgctctacggcggctggagctttgccttccggctgcgctcctcctccgggctgcaggtcctgaacgtgcacttcggcggagagcgcattgcctatgaggtcagcgtgcaagaggcagtggcgctgtatggaggacacacacctgcaggcatgcagaccaagtacctcgatgtcggctggggcctgggcagcgtcactcatgagttagcccccggcatcgactgcccggagaccgccaccttcctggacactttccactactatgatgccgatgacccggtccattatccccgagccctctgcctctttgaaatgcccacaggggtgccccttcggcggcactttaattccaactttaaaggtggcttcaacttctatgcggggctgaagggccaggtgctggtgctgcggacaacttcaactgtctacaattatgattacatttgggactttatcttctaccccaacggggtgatggaggccaagatgcatgccactggctacgtccacgccaccttctacacccccgaggggctgcgccacggcactcgcctgcacacccacctgattggcaacatacacactcacttggtgcactaccgcgtagacctggatgtggcaggcaccaagaacagcttccagacactgcagatgaagctagaaaacatcaccaacccctggagcccaagacaccgcgtggtccagccaactctggagcagacgcagtactcctgggagcgccaggcggccttccgcttcaaaaggaagctgcccacgtacctgctctttaccagcccccaggagaacccctggggccacaagcgcagctaccgcctgcagatccactccatggccgaccaggtgctgcccccaggctggcaggaggagcaggccatcacctgggcaaggtaccccctggcagtgaccaagtaccgggagtcggagctgtgcagcagcagcatctaccaccagaacgacccctggcacccgcccgtggtctttgagcagtttcttcacaacaacgagaacattgaaaatgaggacctggtggcctgggtgacggtgggcttcctgcacatcccccactcagaggacattcccaacacagccacacctgggaactccgtgggcttcctgctccggccattcaacttcttcccagaggacccctccctggcatccagagacactgtgatcgtgtggcctcgggacaacggccccaactacgtccagcgctggatccctgaggacagggactgctcgatgcctcccccttttagctacaatgggacctatagacctgtggagcccaagtccgccgacaagacccacacctgccccccctgccccgccccccccgtggccggcccctccgtgttcctgttcccccccaagcccaaggacaccctgatgatctccaggacccccgaggtgacctgcgtggtggtggacgtgtcccacgaggaccccgaggtgaagttcaactggtacgtggacggcgtggaggtgcacaacgccaagaccaagcccagggaggagcagtacaactccacctacagggtggtgtccgtgctgaccgtgctgcaccaggactggctgaacggcaaggagtacaagtgcaaggtgtccaacaagggcctgccctcctccatcgagaagaccatctccaaggccaagggccagcccagggagccccaggtgtacaccctgcccccctccagggaggagatgaccaagaaccaggtgtccctgacctgcctggtgaagggcttctacccctccgacatcgccgtggagtgggagtccaacggccagcccgagaacaactacaagaccaccccccccgtgctggactccgacggctccttcttcctgtactccaagctgaccgtggacaagtccaggtggcagcagggcaacgtgttctcctgctccgtgatgcacgaggccctgcacaaccactacacccagaagtccctgtccctgtcccccggcaagtga

SEQ ID NO: 90 - DNA, 2949 bp, Artificial Sequence
  hDAO-Fc-Hepmut3
atgccggccctgggctgggccgtggctgccatcctgatgctgcagacggccatggcggagccctccccggggactctgcccaggaaggcaggggtgttttcagacctaagcaaccaagagctgaaggcagtgcacagcttcctctggtccaagaaggagctgaggctgcagccctccagtaccaccaccatggccaagaacaccgtgtttctcatcgagatgctgctgcccaagaagtaccatgtgctgaggtttctggataaaggtgaaaggcatcctgtgcgggaagcccgtgccgtcatcttctttggtgaccaggagcatcccaatgtcaccgagtttgctgtggggcccctgccagggccctgctacatgcgagcactgtcccccaggcctgggtaccagtcctcctgggcatcgaggcccatctccacagcagagtatgccctcctctaccacaccctgcaggaagccaccaagcccctgcatcagttcttcctcaataccacaggcttctcattccaagactgccatgacagatgcctggccttcaccgatgtggccccccggggtgtggcttctggccagcgccgcagttggcttatcatacagcgctatgtagaaggctactttctgcaccccactgggctggagctcctcgtggatcatgggagcacagatgctgggcactgggccgtggagcaggtgtggtacaacgggaagttctatgggagcccagaggaactggctcggaagtatgcagatggagaggtggacgtggtggtcctggaggacccgctgcctgggggcaaggggcatgacagcacagaggagccgcccctcttctcctcccacaagccccgcggggacttccccagccccatccatgtgagcggcccccgcttggtccagccccacggccctcgcttcaggctggagggcaacgctgtgctctacggcggctggagctttgccttccggctgcgctcctcctccgggctgcaggtcctgaacgtgcacttcggcggagagcgcattgcctatgaggtcagcgtgcaagaggcagtggcgctgtatggaggacacacacctgcaggcatgcagaccaagtacctcgatgtcggctggggcctgggcagcgtcactcatgagttagcccccggcatcgactgcccggagaccgccaccttcctggacactttccactactatgatgccgatgacccggtccattatccccgagccctctgcctctttgaaatgcccacaggggtgccccttcggcggcactttaattccaactttaaaggtggcttcaacttctatgcggggctgaagggccaggtgctggtgctgcggacaacttcaactgtctacaattatgattacatttgggactttatcttctaccccaacggggtgatggaggccaagatgcatgccactggctacgtccacgccaccttctacacccccgaggggctgcgccacggcactcgcctgcacacccacctgattggcaacatacacactcacttggtgcactaccgcgtagacctggatgtggcaggcaccaagaacagcttccagacactgcagatgaagctagaaaacatcaccaacccctggagcccaagacaccgcgtggtccagccaactctggagcagacgcagtactcctgggagcgccaggcggccttccgcttcaaaacgaagctgcccaagtacctgctctttaccagcccccaggagaacccctggggccacaagcgcagctaccgcctgcagatccactccatggccgaccaggtgctgcccccaggctggcaggaggagcaggccatcacctgggcaaggtaccccctggcagtgaccaagtaccgggagtcggagctgtgcagcagcagcatctaccaccagaacgacccctggcacccgcccgtggtctttgagcagtttcttcacaacaacgagaacattgaaaatgaggacctggtggcctgggtgacggtgggcttcctgcacatcccccactcagaggacattcccaacacagccacacctgggaactccgtgggcttcctgctccggccattcaacttcttcccagaggacccctccctggcatccagagacactgtgatcgtgtggcctcgggacaacggccccaactacgtccagcgctggatccctgaggacagggactgctcgatgcctcccccttttagctacaatgggacctatagacctgtggagcccaagtccgccgacaagacccacacctgccccccctgccccgccccccccgtggccggcccctccgtgttcctgttcccccccaagcccaaggacaccctgatgatctccaggacccccgaggtgacctgcgtggtggtggacgtgtcccacgaggaccccgaggtgaagttcaactggtacgtggacggcgtggaggtgcacaacgccaagaccaagcccagggaggagcagtacaactccacctacagggtggtgtccgtgctgaccgtgctgcaccaggactggctgaacggcaaggagtacaagtgcaaggtgtccaacaagggcctgccctcctccatcgagaagaccatctccaaggccaagggccagcccagggagccccaggtgtacaccctgcccccctccagggaggagatgaccaagaaccaggtgtccctgacctgcctggtgaagggcttctacccctccgacatcgccgtggagtgggagtccaacggccagcccgagaacaactacaagaccaccccccccgtgctggactccgacggctccttcttcctgtactccaagctgaccgtggacaagtccaggtggcagcagggcaacgtgttctcctgctccgtgatgcacgaggccctgcacaaccactacacccagaagtccctgtccctgtcccccggcaagtga

SEQ ID NO: 91 - DNA, 2949 bp, Artificial Sequence
  hDAO-Fc-Hepmut4
atgccggccctgggctgggccgtggctgccatcctgatgctgcagacggccatggcggagccctccccggggactctgcccaggaaggcaggggtgttttcagacctaagcaaccaagagctgaaggcagtgcacagcttcctctggtccaagaaggagctgaggctgcagccctccagtaccaccaccatggccaagaacaccgtgtttctcatcgagatgctgctgcccaagaagtaccatgtgctgaggtttctggataaaggtgaaaggcatcctgtgcgggaagcccgtgccgtcatcttctttggtgaccaggagcatcccaatgtcaccgagtttgctgtggggcccctgccagggccctgctacatgcgagcactgtcccccaggcctgggtaccagtcctcctgggcatcgaggcccatctccacagcagagtatgccctcctctaccacaccctgcaggaagccaccaagcccctgcatcagttcttcctcaataccacaggcttctcattccaagactgccatgacagatgcctggccttcaccgatgtggccccccggggtgtggcttctggccagcgccgcagttggcttatcatacagcgctatgtagaaggctactttctgcaccccactgggctggagctcctcgtggatcatgggagcacagatgctgggcactgggccgtggagcaggtgtggtacaacgggaagttctatgggagcccagaggaactggctcggaagtatgcagatggagaggtggacgtggtggtcctggaggacccgctgcctgggggcaaggggcatgacagcacagaggagccgcccctcttctcctcccacaagccccgcggggacttccccagccccatccatgtgagcggcccccgcttggtccagccccacggccctcgcttcaggctggagggcaacgctgtgctctacggcggctggagctttgccttccggctgcgctcctcctccgggctgcaggtcctgaacgtgcacttcggcggagagcgcattgcctatgaggtcagcgtgcaagaggcagtggcgctgtatggaggacacacacctgcaggcatgcagaccaagtacctcgatgtcggctggggcctgggcagcgtcactcatgagttagcccccggcatcgactgcccggagaccgccaccttcctggacactttccactactatgatgccgatgacccggtccattatccccgagccctctgcctctttgaaatgcccacaggggtgccccttcggcggcactttaattccaactttaaaggtggcttcaacttctatgcggggctgaagggccaggtgctggtgctgcggacaacttcaactgtctacaattatgattacatttgggactttatcttctaccccaacggggtgatggaggccaagatgcatgccactggctacgtccacgccaccttctacacccccgaggggctgcgccacggcactcgcctgcacacccacctgattggcaacatacacactcacttggtgcactaccgcgtagacctggatgtggcaggcaccaagaacagcttccagacactgcagatgaagctagaaaacatcaccaacccctggagcccaagacaccgcgtggtccagccaactctggagcagacgcagtactcctgggagcgccaggcggccttcagcttcaaaacgaagctgcccaagtacctgctctttaccagcccccaggagaacccctggggccacaagcgcagctaccgcctgcagatccactccatggccgaccaggtgctgcccccaggctggcaggaggagcaggccatcacctgggcaaggtaccccctggcagtgaccaagtaccgggagtcggagctgtgcagcagcagcatctaccaccagaacgacccctggcacccgcccgtggtctttgagcagtttcttcacaacaacgagaacattgaaaatgaggacctggtggcctgggtgacggtgggcttcctgcacatcccccactcagaggacattcccaacacagccacacctgggaactccgtgggcttcctgctccggccattcaacttcttcccagaggacccctccctggcatccagagacactgtgatcgtgtggcctcgggacaacggccccaactacgtccagcgctggatccctgaggacagggactgctcgatgcctcccccttttagctacaatgggacctatagacctgtggagcccaagtccgccgacaagacccacacctgccccccctgccccgccccccccgtggccggcccctccgtgttcctgttcccccccaagcccaaggacaccctgatgatctccaggacccccgaggtgacctgcgtggtggtggacgtgtcccacgaggaccccgaggtgaagttcaactggtacgtggacggcgtggaggtgcacaacgccaagaccaagcccagggaggagcagtacaactccacctacagggtggtgtccgtgctgaccgtgctgcaccaggactggctgaacggcaaggagtacaagtgcaaggtgtccaacaagggcctgccctcctccatcgagaagaccatctccaaggccaagggccagcccagggagccccaggtgtacaccctgcccccctccagggaggagatgaccaagaaccaggtgtccctgacctgcctggtgaagggcttctacccctccgacatcgccgtggagtgggagtccaacggccagcccgagaacaactacaagaccaccccccccgtgctggactccgacggctccttcttcctgtactccaagctgaccgtggacaagtccaggtggcagcagggcaacgtgttctcctgctccgtgatgcacgaggccctgcacaaccactacacccagaagtccctgtccctgtcccccggcaagtga

SEQ ID NO: 92 - DNA, 2949 bp, Artificial Sequence
  hDAO-Fc-Hepmut5
atgccggccctgggctgggccgtggctgccatcctgatgctgcagacggccatggcggagccctccccggggactctgcccaggaaggcaggggtgttttcagacctaagcaaccaagagctgaaggcagtgcacagcttcctctggtccaagaaggagctgaggctgcagccctccagtaccaccaccatggccaagaacaccgtgtttctcatcgagatgctgctgcccaagaagtaccatgtgctgaggtttctggataaaggtgaaaggcatcctgtgcgggaagcccgtgccgtcatcttctttggtgaccaggagcatcccaatgtcaccgagtttgctgtggggcccctgccagggccctgctacatgcgagcactgtcccccaggcctgggtaccagtcctcctgggcatcgaggcccatctccacagcagagtatgccctcctctaccacaccctgcaggaagccaccaagcccctgcatcagttcttcctcaataccacaggcttctcattccaagactgccatgacagatgcctggccttcaccgatgtggccccccggggtgtggcttctggccagcgccgcagttggcttatcatacagcgctatgtagaaggctactttctgcaccccactgggctggagctcctcgtggatcatgggagcacagatgctgggcactgggccgtggagcaggtgtggtacaacgggaagttctatgggagcccagaggaactggctcggaagtatgcagatggagaggtggacgtggtggtcctggaggacccgctgcctgggggcaaggggcatgacagcacagaggagccgcccctcttctcctcccacaagccccgcggggacttccccagccccatccatgtgagcggcccccgcttggtccagccccacggccctcgcttcaggctggagggcaacgctgtgctctacggcggctggagctttgccttccggctgcgctcctcctccgggctgcaggtcctgaacgtgcacttcggcggagagcgcattgcctatgaggtcagcgtgcaagaggcagtggcgctgtatggaggacacacacctgcaggcatgcagaccaagtacctcgatgtcggctggggcctgggcagcgtcactcatgagttagcccccggcatcgactgcccggagaccgccaccttcctggacactttccactactatgatgccgatgacccggtccattatccccgagccctctgcctctttgaaatgcccacaggggtgccccttcggcggcactttaattccaactttaaaggtggcttcaacttctatgcggggctgaagggccaggtgctggtgctgcggacaacttcaactgtctacaattatgattacatttgggactttatcttctaccccaacggggtgatggaggccaagatgcatgccactggctacgtccacgccaccttctacacccccgaggggctgcgccacggcactcgcctgcacacccacctgattggcaacatacacactcacttggtgcactaccgcgtagacctggatgtggcaggcaccaagaacagcttccagacactgcagatgaagctagaaaacatcaccaacccctggagcccaagacaccgcgtggtccagccaactctggagcagacgcagtactcctgggagcgccaggcggccttccgcttcaaaacgaagctgcccacgtacctgctctttaccagcccccaggagaacccctggggccacaagcgcagctaccgcctgcagatccactccatggccgaccaggtgctgcccccaggctggcaggaggagcaggccatcacctgggcaaggtaccccctggcagtgaccaagtaccgggagtcggagctgtgcagcagcagcatctaccaccagaacgacccctggcacccgcccgtggtctttgagcagtttcttcacaacaacgagaacattgaaaatgaggacctggtggcctgggtgacggtgggcttcctgcacatcccccactcagaggacattcccaacacagccacacctgggaactccgtgggcttcctgctccggccattcaacttcttcccagaggacccctccctggcatccagagacactgtgatcgtgtggcctcgggacaacggccccaactacgtccagcgctggatccctgaggacagggactgctcgatgcctcccccttttagctacaatgggacctatagacctgtggagcccaagtccgccgacaagacccacacctgccccccctgccccgccccccccgtggccggcccctccgtgttcctgttcccccccaagcccaaggacaccctgatgatctccaggacccccgaggtgacctgcgtggtggtggacgtgtcccacgaggaccccgaggtgaagttcaactggtacgtggacggcgtggaggtgcacaacgccaagaccaagcccagggaggagcagtacaactccacctacagggtggtgtccgtgctgaccgtgctgcaccaggactggctgaacggcaaggagtacaagtgcaaggtgtccaacaagggcctgccctcctccatcgagaagaccatctccaaggccaagggccagcccagggagccccaggtgtacaccctgcccccctccagggaggagatgaccaagaaccaggtgtccctgacctgcctggtgaagggcttctacccctccgacatcgccgtggagtgggagtccaacggccagcccgagaacaactacaagaccaccccccccgtgctggactccgacggctccttcttcctgtactccaagctgaccgtggacaagtccaggtggcagcagggcaacgtgttctcctgctccgtgatgcacgaggccctgcacaaccactacacccagaagtccctgtccctgtcccccggcaagtga

SEQ ID NO: 93 - DNA, 2949 bp, Artificial Sequence
  hDAO-Fc-Hepmut6
atgccggccctgggctgggccgtggctgccatcctgatgctgcagacggccatggcggagccctccccggggactctgcccaggaaggcaggggtgttttcagacctaagcaaccaagagctgaaggcagtgcacagcttcctctggtccaagaaggagctgaggctgcagccctccagtaccaccaccatggccaagaacaccgtgtttctcatcgagatgctgctgcccaagaagtaccatgtgctgaggtttctggataaaggtgaaaggcatcctgtgcgggaagcccgtgccgtcatcttctttggtgaccaggagcatcccaatgtcaccgagtttgctgtggggcccctgccagggccctgctacatgcgagcactgtcccccaggcctgggtaccagtcctcctgggcatcgaggcccatctccacagcagagtatgccctcctctaccacaccctgcaggaagccaccaagcccctgcatcagttcttcctcaataccacaggcttctcattccaagactgccatgacagatgcctggccttcaccgatgtggccccccggggtgtggcttctggccagcgccgcagttggcttatcatacagcgctatgtagaaggctactttctgcaccccactgggctggagctcctcgtggatcatgggagcacagatgctgggcactgggccgtggagcaggtgtggtacaacgggaagttctatgggagcccagaggaactggctcggaagtatgcagatggagaggtggacgtggtggtcctggaggacccgctgcctgggggcaaggggcatgacagcacagaggagccgcccctcttctcctcccacaagccccgcggggacttccccagccccatccatgtgagcggcccccgcttggtccagccccacggccctcgcttcaggctggagggcaacgctgtgctctacggcggctggagctttgccttccggctgcgctcctcctccgggctgcaggtcctgaacgtgcacttcggcggagagcgcattgcctatgaggtcagcgtgcaagaggcagtggcgctgtatggaggacacacacctgcaggcatgcagaccaagtacctcgatgtcggctggggcctgggcagcgtcactcatgagttagcccccggcatcgactgcccggagaccgccaccttcctggacactttccactactatgatgccgatgacccggtccattatccccgagccctctgcctctttgaaatgcccacaggggtgccccttcggcggcactttaattccaactttaaaggtggcttcaacttctatgcggggctgaagggccaggtgctggtgctgcggacaacttcaactgtctacaattatgattacatttgggactttatcttctaccccaacggggtgatggaggccaagatgcatgccactggctacgtccacgccaccttctacacccccgaggggctgcgccacggcactcgcctgcacacccacctgattggcaacatacacactcacttggtgcactaccgcgtagacctggatgtggcaggcaccaagaacagcttccagacactgcagatgaagctagaaaacatcaccaacccctggagcccaagacaccgcgtggtccagccaactctggagcagacgcagtactcctgggagcgccaggcggccttccgcttcggacagacgctgcccaagtacctgctctttaccagcccccaggagaacccctggggccacaagcgcagctaccgcctgcagatccactccatggccgaccaggtgctgcccccaggctggcaggaggagcaggccatcacctgggcaaggtaccccctggcagtgaccaagtaccgggagtcggagctgtgcagcagcagcatctaccaccagaacgacccctggcacccgcccgtggtctttgagcagtttcttcacaacaacgagaacattgaaaatgaggacctggtggcctgggtgacggtgggcttcctgcacatcccccactcagaggacattcccaacacagccacacctgggaactccgtgggcttcctgctccggccattcaacttcttcccagaggacccctccctggcatccagagacactgtgatcgtgtggcctcgggacaacggccccaactacgtccagcgctggatccctgaggacagggactgctcgatgcctcccccttttagctacaatgggacctatagacctgtggagcccaagtccgccgacaagacccacacctgccccccctgccccgccccccccgtggccggcccctccgtgttcctgttcccccccaagcccaaggacaccctgatgatctccaggacccccgaggtgacctgcgtggtggtggacgtgtcccacgaggaccccgaggtgaagttcaactggtacgtggacggcgtggaggtgcacaacgccaagaccaagcccagggaggagcagtacaactccacctacagggtggtgtccgtgctgaccgtgctgcaccaggactggctgaacggcaaggagtacaagtgcaaggtgtccaacaagggcctgccctcctccatcgagaagaccatctccaaggccaagggccagcccagggagccccaggtgtacaccctgcccccctccagggaggagatgaccaagaaccaggtgtccctgacctgcctggtgaagggcttctacccctccgacatcgccgtggagtgggagtccaacggccagcccgagaacaactacaagaccaccccccccgtgctggactccgacggctccttcttcctgtactccaagctgaccgtggacaagtccaggtggcagcagggcaacgtgttctcctgctccgtgatgcacgaggccctgcacaaccactacacccagaagtccctgtccctgtcccccggcaagtga

SEQ ID NO: 94 - DNA, 2949 bp, Artificial Sequence
  hDAO-Fc-Hepmut7
atgccggccctgggctgggccgtggctgccatcctgatgctgcagacggccatggcggagccctccccggggactctgcccaggaaggcaggggtgttttcagacctaagcaaccaagagctgaaggcagtgcacagcttcctctggtccaagaaggagctgaggctgcagccctccagtaccaccaccatggccaagaacaccgtgtttctcatcgagatgctgctgcccaagaagtaccatgtgctgaggtttctggataaaggtgaaaggcatcctgtgcgggaagcccgtgccgtcatcttctttggtgaccaggagcatcccaatgtcaccgagtttgctgtggggcccctgccagggccctgctacatgcgagcactgtcccccaggcctgggtaccagtcctcctgggcatcgaggcccatctccacagcagagtatgccctcctctaccacaccctgcaggaagccaccaagcccctgcatcagttcttcctcaataccacaggcttctcattccaagactgccatgacagatgcctggccttcaccgatgtggccccccggggtgtggcttctggccagcgccgcagttggcttatcatacagcgctatgtagaaggctactttctgcaccccactgggctggagctcctcgtggatcatgggagcacagatgctgggcactgggccgtggagcaggtgtggtacaacgggaagttctatgggagcccagaggaactggctcggaagtatgcagatggagaggtggacgtggtggtcctggaggacccgctgcctgggggcaaggggcatgacagcacagaggagccgcccctcttctcctcccacaagccccgcggggacttccccagccccatccatgtgagcggcccccgcttggtccagccccacggccctcgcttcaggctggagggcaacgctgtgctctacggcggctggagctttgccttccggctgcgctcctcctccgggctgcaggtcctgaacgtgcacttcggcggagagcgcattgcctatgaggtcagcgtgcaagaggcagtggcgctgtatggaggacacacacctgcaggcatgcagaccaagtacctcgatgtcggctggggcctgggcagcgtcactcatgagttagcccccggcatcgactgcccggagaccgccaccttcctggacactttccactactatgatgccgatgacccggtccattatccccgagccctctgcctctttgaaatgcccacaggggtgccccttcggcggcactttaattccaactttaaaggtggcttcaacttctatgcggggctgaagggccaggtgctggtgctgcggacaacttcaactgtctacaattatgattacatttgggactttatcttctaccccaacggggtgatggaggccaagatgcatgccactggctacgtccacgccaccttctacacccccgaggggctgcgccacggcactcgcctgcacacccacctgattggcaacatacacactcacttggtgcactaccgcgtagacctggatgtggcaggcaccaagaacagcttccagacactgcagatgaagctagaaaacatcaccaacccctggagcccaagacaccgcgtggtccagccaactctggagcagacgcagtactcctgggagcgccaggcggccttcagcttcaaaaggaagctgcccacgtacctgctctttaccagcccccaggagaacccctggggccacaagcgcagctaccgcctgcagatccactccatggccgaccaggtgctgcccccaggctggcaggaggagcaggccatcacctgggcaaggtaccccctggcagtgaccaagtaccgggagtcggagctgtgcagcagcagcatctaccaccagaacgacccctggcacccgcccgtggtctttgagcagtttcttcacaacaacgagaacattgaaaatgaggacctggtggcctgggtgacggtgggcttcctgcacatcccccactcagaggacattcccaacacagccacacctgggaactccgtgggcttcctgctccggccattcaacttcttcccagaggacccctccctggcatccagagacactgtgatcgtgtggcctcgggacaacggccccaactacgtccagcgctggatccctgaggacagggactgctcgatgcctcccccttttagctacaatgggacctatagacctgtggagcccaagtccgccgacaagacccacacctgccccccctgccccgccccccccgtggccggcccctccgtgttcctgttcccccccaagcccaaggacaccctgatgatctccaggacccccgaggtgacctgcgtggtggtggacgtgtcccacgaggaccccgaggtgaagttcaactggtacgtggacggcgtggaggtgcacaacgccaagaccaagcccagggaggagcagtacaactccacctacagggtggtgtccgtgctgaccgtgctgcaccaggactggctgaacggcaaggagtacaagtgcaaggtgtccaacaagggcctgccctcctccatcgagaagaccatctccaaggccaagggccagcccagggagccccaggtgtacaccctgcccccctccagggaggagatgaccaagaaccaggtgtccctgacctgcctggtgaagggcttctacccctccgacatcgccgtggagtgggagtccaacggccagcccgagaacaactacaagaccaccccccccgtgctggactccgacggctccttcttcctgtactccaagctgaccgtggacaagtccaggtggcagcagggcaacgtgttctcctgctccgtgatgcacgaggccctgcacaaccactacacccagaagtccctgtccctgtcccccggcaagtga

SEQ ID NO: 95 - DNA, 2949 bp, Artificial Sequence
  hDAO-Fc-Cysmut
atgccggccctgggctgggccgtggctgccatcctgatgctgcagacggccatggcggagccctccccggggactctgcccaggaaggcaggggtgttttcagacctaagcaaccaagagctgaaggcagtgcacagcttcctctggtccaagaaggagctgaggctgcagccctccagtaccaccaccatggccaagaacaccgtgtttctcatcgagatgctgctgcccaagaagtaccatgtgctgaggtttctggataaaggtgaaaggcatcctgtgcgggaagcccgtgccgtcatcttctttggtgaccaggagcatcccaatgtcaccgagtttgctgtggggcccctgccagggcccgcctacatgcgagcactgtcccccaggcctgggtaccagtcctcctgggcatcgaggcccatctccacagcagagtatgccctcctctaccacaccctgcaggaagccaccaagcccctgcatcagttcttcctcaataccacaggcttctcattccaagactgccatgacagatgcctggccttcaccgatgtggccccccggggtgtggcttctggccagcgccgcagttggcttatcatacagcgctatgtagaaggctactttctgcaccccactgggctggagctcctcgtggatcatgggagcacagatgctgggcactgggccgtggagcaggtgtggtacaacgggaagttctatgggagcccagaggaactggctcggaagtatgcagatggagaggtggacgtggtggtcctggaggacccgctgcctgggggcaaggggcatgacagcacagaggagccgcccctcttctcctcccacaagccccgcggggacttccccagccccatccatgtgagcggcccccgcttggtccagccccacggccctcgcttcaggctggagggcaacgctgtgctctacggcggctggagctttgccttccggctgcgctcctcctccgggctgcaggtcctgaacgtgcacttcggcggagagcgcattgcctatgaggtcagcgtgcaagaggcagtggcgctgtatggaggacacacacctgcaggcatgcagaccaagtacctcgatgtcggctggggcctgggcagcgtcactcatgagttagcccccggcatcgactgcccggagaccgccaccttcctggacactttccactactatgatgccgatgacccggtccattatccccgagccctctgcctctttgaaatgcccacaggggtgccccttcggcggcactttaattccaactttaaaggtggcttcaacttctatgcggggctgaagggccaggtgctggtgctgcggacaacttcaactgtctacaattatgattacatttgggactttatcttctaccccaacggggtgatggaggccaagatgcatgccactggctacgtccacgccaccttctacacccccgaggggctgcgccacggcactcgcctgcacacccacctgattggcaacatacacactcacttggtgcactaccgcgtagacctggatgtggcaggcaccaagaacagcttccagacactgcagatgaagctagaaaacatcaccaacccctggagcccaagacaccgcgtggtccagccaactctggagcagacgcagtactcctgggagcgccaggcggccttccgcttcaaaaggaagctgcccaagtacctgctctttaccagcccccaggagaacccctggggccacaagcgcagctaccgcctgcagatccactccatggccgaccaggtgctgcccccaggctggcaggaggagcaggccatcacctgggcaaggtaccccctggcagtgaccaagtaccgggagtcggagctgtgcagcagcagcatctaccaccagaacgacccctggcacccgcccgtggtctttgagcagtttcttcacaacaacgagaacattgaaaatgaggacctggtggcctgggtgacggtgggcttcctgcacatcccccactcagaggacattcccaacacagccacacctgggaactccgtgggcttcctgctccggccattcaacttcttcccagaggacccctccctggcatccagagacactgtgatcgtgtggcctcgggacaacggccccaactacgtccagcgctggatccctgaggacagggactgctcgatgcctcccccttttagctacaatgggacctatagacctgtggagcccaagtccgccgacaagacccacacctgccccccctgccccgccccccccgtggccggcccctccgtgttcctgttcccccccaagcccaaggacaccctgatgatctccaggacccccgaggtgacctgcgtggtggtggacgtgtcccacgaggaccccgaggtgaagttcaactggtacgtggacggcgtggaggtgcacaacgccaagaccaagcccagggaggagcagtacaactccacctacagggtggtgtccgtgctgaccgtgctgcaccaggactggctgaacggcaaggagtacaagtgcaaggtgtccaacaagggcctgccctcctccatcgagaagaccatctccaaggccaagggccagcccagggagccccaggtgtacaccctgcccccctccagggaggagatgaccaagaaccaggtgtccctgacctgcctggtgaagggcttctacccctccgacatcgccgtggagtgggagtccaacggccagcccgagaacaactacaagaccaccccccccgtgctggactccgacggctccttcttcctgtactccaagctgaccgtggacaagtccaggtggcagcagggcaacgtgttctcctgctccgtgatgcacgaggccctgcacaaccactacacccagaagtccctgtccctgtcccccggcaagtga

SEQ ID NO: 96 - DNA, 2949 bp, Artificial Sequence
  hDAO-Fc-Hepmut1-Cysmut
atgccggccctgggctgggccgtggctgccatcctgatgctgcagacggccatggcggagccctccccggggactctgcccaggaaggcaggggtgttttcagacctaagcaaccaagagctgaaggcagtgcacagcttcctctggtccaagaaggagctgaggctgcagccctccagtaccaccaccatggccaagaacaccgtgtttctcatcgagatgctgctgcccaagaagtaccatgtgctgaggtttctggataaaggtgaaaggcatcctgtgcgggaagcccgtgccgtcatcttctttggtgaccaggagcatcccaatgtcaccgagtttgctgtggggcccctgccagggcccgcctacatgcgagcactgtcccccaggcctgggtaccagtcctcctgggcatcgaggcccatctccacagcagagtatgccctcctctaccacaccctgcaggaagccaccaagcccctgcatcagttcttcctcaataccacaggcttctcattccaagactgccatgacagatgcctggccttcaccgatgtggccccccggggtgtggcttctggccagcgccgcagttggcttatcatacagcgctatgtagaaggctactttctgcaccccactgggctggagctcctcgtggatcatgggagcacagatgctgggcactgggccgtggagcaggtgtggtacaacgggaagttctatgggagcccagaggaactggctcggaagtatgcagatggagaggtggacgtggtggtcctggaggacccgctgcctgggggcaaggggcatgacagcacagaggagccgcccctcttctcctcccacaagccccgcggggacttccccagccccatccatgtgagcggcccccgcttggtccagccccacggccctcgcttcaggctggagggcaacgctgtgctctacggcggctggagctttgccttccggctgcgctcctcctccgggctgcaggtcctgaacgtgcacttcggcggagagcgcattgcctatgaggtcagcgtgcaagaggcagtggcgctgtatggaggacacacacctgcaggcatgcagaccaagtacctcgatgtcggctggggcctgggcagcgtcactcatgagttagcccccggcatcgactgcccggagaccgccaccttcctggacactttccactactatgatgccgatgacccggtccattatccccgagccctctgcctctttgaaatgcccacaggggtgccccttcggcggcactttaattccaactttaaaggtggcttcaacttctatgcggggctgaagggccaggtgctggtgctgcggacaacttcaactgtctacaattatgattacatttgggactttatcttctaccccaacggggtgatggaggccaagatgcatgccactggctacgtccacgccaccttctacacccccgaggggctgcgccacggcactcgcctgcacacccacctgattggcaacatacacactcacttggtgcactaccgcgtagacctggatgtggcaggcaccaagaacagcttccagacactgcagatgaagctagaaaacatcaccaacccctggagcccaagacaccgcgtggtccagccaactctggagcagacgcagtactcctgggagcgccaggcggccttcagcttcaaaaggaagctgcccaagtacctgctctttaccagcccccaggagaacccctggggccacaagcgcagctaccgcctgcagatccactccatggccgaccaggtgctgcccccaggctggcaggaggagcaggccatcacctgggcaaggtaccccctggcagtgaccaagtaccgggagtcggagctgtgcagcagcagcatctaccaccagaacgacccctggcacccgcccgtggtctttgagcagtttcttcacaacaacgagaacattgaaaatgaggacctggtggcctgggtgacggtgggcttcctgcacatcccccactcagaggacattcccaacacagccacacctgggaactccgtgggcttcctgctccggccattcaacttcttcccagaggacccctccctggcatccagagacactgtgatcgtgtggcctcgggacaacggccccaactacgtccagcgctggatccctgaggacagggactgctcgatgcctcccccttttagctacaatgggacctatagacctgtggagcccaagtccgccgacaagacccacacctgccccccctgccccgccccccccgtggccggcccctccgtgttcctgttcccccccaagcccaaggacaccctgatgatctccaggacccccgaggtgacctgcgtggtggtggacgtgtcccacgaggaccccgaggtgaagttcaactggtacgtggacggcgtggaggtgcacaacgccaagaccaagcccagggaggagcagtacaactccacctacagggtggtgtccgtgctgaccgtgctgcaccaggactggctgaacggcaaggagtacaagtgcaaggtgtccaacaagggcctgccctcctccatcgagaagaccatctccaaggccaagggccagcccagggagccccaggtgtacaccctgcccccctccagggaggagatgaccaagaaccaggtgtccctgacctgcctggtgaagggcttctacccctccgacatcgccgtggagtgggagtccaacggccagcccgagaacaactacaagaccaccccccccgtgctggactccgacggctccttcttcctgtactccaagctgaccgtggacaagtccaggtggcagcagggcaacgtgttctcctgctccgtgatgcacgaggccctgcacaaccactacacccagaagtccctgtccctgtcccccggcaagtga

SEQ ID NO: 97 - DNA, 2949 bp, Artificial Sequence
  hDAO-Fc-Hepmut2-Cysmut
atgccggccctgggctgggccgtggctgccatcctgatgctgcagacggccatggcggagccctccccggggactctgcccaggaaggcaggggtgttttcagacctaagcaaccaagagctgaaggcagtgcacagcttcctctggtccaagaaggagctgaggctgcagccctccagtaccaccaccatggccaagaacaccgtgtttctcatcgagatgctgctgcccaagaagtaccatgtgctgaggtttctggataaaggtgaaaggcatcctgtgcgggaagcccgtgccgtcatcttctttggtgaccaggagcatcccaatgtcaccgagtttgctgtggggcccctgccagggcccgcctacatgcgagcactgtcccccaggcctgggtaccagtcctcctgggcatcgaggcccatctccacagcagagtatgccctcctctaccacaccctgcaggaagccaccaagcccctgcatcagttcttcctcaataccacaggcttctcattccaagactgccatgacagatgcctggccttcaccgatgtggccccccggggtgtggcttctggccagcgccgcagttggcttatcatacagcgctatgtagaaggctactttctgcaccccactgggctggagctcctcgtggatcatgggagcacagatgctgggcactgggccgtggagcaggtgtggtacaacgggaagttctatgggagcccagaggaactggctcggaagtatgcagatggagaggtggacgtggtggtcctggaggacccgctgcctgggggcaaggggcatgacagcacagaggagccgcccctcttctcctcccacaagccccgcggggacttccccagccccatccatgtgagcggcccccgcttggtccagccccacggccctcgcttcaggctggagggcaacgctgtgctctacggcggctggagctttgccttccggctgcgctcctcctccgggctgcaggtcctgaacgtgcacttcggcggagagcgcattgcctatgaggtcagcgtgcaagaggcagtggcgctgtatggaggacacacacctgcaggcatgcagaccaagtacctcgatgtcggctggggcctgggcagcgtcactcatgagttagcccccggcatcgactgcccggagaccgccaccttcctggacactttccactactatgatgccgatgacccggtccattatccccgagccctctgcctctttgaaatgcccacaggggtgccccttcggcggcactttaattccaactttaaaggtggcttcaacttctatgcggggctgaagggccaggtgctggtgctgcggacaacttcaactgtctacaattatgattacatttgggactttatcttctaccccaacggggtgatggaggccaagatgcatgccactggctacgtccacgccaccttctacacccccgaggggctgcgccacggcactcgcctgcacacccacctgattggcaacatacacactcacttggtgcactaccgcgtagacctggatgtggcaggcaccaagaacagcttccagacactgcagatgaagctagaaaacatcaccaacccctggagcccaagacaccgcgtggtccagccaactctggagcagacgcagtactcctgggagcgccaggcggccttccgcttcaaaaggaagctgcccacgtacctgctctttaccagcccccaggagaacccctggggccacaagcgcagctaccgcctgcagatccactccatggccgaccaggtgctgcccccaggctggcaggaggagcaggccatcacctgggcaaggtaccccctggcagtgaccaagtaccgggagtcggagctgtgcagcagcagcatctaccaccagaacgacccctggcacccgcccgtggtctttgagcagtttcttcacaacaacgagaacattgaaaatgaggacctggtggcctgggtgacggtgggcttcctgcacatcccccactcagaggacattcccaacacagccacacctgggaactccgtgggcttcctgctccggccattcaacttcttcccagaggacccctccctggcatccagagacactgtgatcgtgtggcctcgggacaacggccccaactacgtccagcgctggatccctgaggacagggactgctcgatgcctcccccttttagctacaatgggacctatagacctgtggagcccaagtccgccgacaagacccacacctgccccccctgccccgccccccccgtggccggcccctccgtgttcctgttcccccccaagcccaaggacaccctgatgatctccaggacccccgaggtgacctgcgtggtggtggacgtgtcccacgaggaccccgaggtgaagttcaactggtacgtggacggcgtggaggtgcacaacgccaagaccaagcccagggaggagcagtacaactccacctacagggtggtgtccgtgctgaccgtgctgcaccaggactggctgaacggcaaggagtacaagtgcaaggtgtccaacaagggcctgccctcctccatcgagaagaccatctccaaggccaagggccagcccagggagccccaggtgtacaccctgcccccctccagggaggagatgaccaagaaccaggtgtccctgacctgcctggtgaagggcttctacccctccgacatcgccgtggagtgggagtccaacggccagcccgagaacaactacaagaccaccccccccgtgctggactccgacggctccttcttcctgtactccaagctgaccgtggacaagtccaggtggcagcagggcaacgtgttctcctgctccgtgatgcacgaggccctgcacaaccactacacccagaagtccctgtccctgtcccccggcaagtga

SEQ ID NO: 98 - DNA, 2949 bp, Artificial Sequence
  hDAO-Fc-Hepmut3-Cysmut
atgccggccctgggctgggccgtggctgccatcctgatgctgcagacggccatggcggagccctccccggggactctgcccaggaaggcaggggtgttttcagacctaagcaaccaagagctgaaggcagtgcacagcttcctctggtccaagaaggagctgaggctgcagccctccagtaccaccaccatggccaagaacaccgtgtttctcatcgagatgctgctgcccaagaagtaccatgtgctgaggtttctggataaaggtgaaaggcatcctgtgcgggaagcccgtgccgtcatcttctttggtgaccaggagcatcccaatgtcaccgagtttgctgtggggcccctgccagggcccgcctacatgcgagcactgtcccccaggcctgggtaccagtcctcctgggcatcgaggcccatctccacagcagagtatgccctcctctaccacaccctgcaggaagccaccaagcccctgcatcagttcttcctcaataccacaggcttctcattccaagactgccatgacagatgcctggccttcaccgatgtggccccccggggtgtggcttctggccagcgccgcagttggcttatcatacagcgctatgtagaaggctactttctgcaccccactgggctggagctcctcgtggatcatgggagcacagatgctgggcactgggccgtggagcaggtgtggtacaacgggaagttctatgggagcccagaggaactggctcggaagtatgcagatggagaggtggacgtggtggtcctggaggacccgctgcctgggggcaaggggcatgacagcacagaggagccgcccctcttctcctcccacaagccccgcggggacttccccagccccatccatgtgagcggcccccgcttggtccagccccacggccctcgcttcaggctggagggcaacgctgtgctctacggcggctggagctttgccttccggctgcgctcctcctccgggctgcaggtcctgaacgtgcacttcggcggagagcgcattgcctatgaggtcagcgtgcaagaggcagtggcgctgtatggaggacacacacctgcaggcatgcagaccaagtacctcgatgtcggctggggcctgggcagcgtcactcatgagttagcccccggcatcgactgcccggagaccgccaccttcctggacactttccactactatgatgccgatgacccggtccattatccccgagccctctgcctctttgaaatgcccacaggggtgccccttcggcggcactttaattccaactttaaaggtggcttcaacttctatgcggggctgaagggccaggtgctggtgctgcggacaacttcaactgtctacaattatgattacatttgggactttatcttctaccccaacggggtgatggaggccaagatgcatgccactggctacgtccacgccaccttctacacccccgaggggctgcgccacggcactcgcctgcacacccacctgattggcaacatacacactcacttggtgcactaccgcgtagacctggatgtggcaggcaccaagaacagcttccagacactgcagatgaagctagaaaacatcaccaacccctggagcccaagacaccgcgtggtccagccaactctggagcagacgcagtactcctgggagcgccaggcggccttccgcttcaaaacgaagctgcccaagtacctgctctttaccagcccccaggagaacccctggggccacaagcgcagctaccgcctgcagatccactccatggccgaccaggtgctgcccccaggctggcaggaggagcaggccatcacctgggcaaggtaccccctggcagtgaccaagtaccgggagtcggagctgtgcagcagcagcatctaccaccagaacgacccctggcacccgcccgtggtctttgagcagtttcttcacaacaacgagaacattgaaaatgaggacctggtggcctgggtgacggtgggcttcctgcacatcccccactcagaggacattcccaacacagccacacctgggaactccgtgggcttcctgctccggccattcaacttcttcccagaggacccctccctggcatccagagacactgtgatcgtgtggcctcgggacaacggccccaactacgtccagcgctggatccctgaggacagggactgctcgatgcctcccccttttagctacaatgggacctatagacctgtggagcccaagtccgccgacaagacccacacctgccccccctgccccgccccccccgtggccggcccctccgtgttcctgttcccccccaagcccaaggacaccctgatgatctccaggacccccgaggtgacctgcgtggtggtggacgtgtcccacgaggaccccgaggtgaagttcaactggtacgtggacggcgtggaggtgcacaacgccaagaccaagcccagggaggagcagtacaactccacctacagggtggtgtccgtgctgaccgtgctgcaccaggactggctgaacggcaaggagtacaagtgcaaggtgtccaacaagggcctgccctcctccatcgagaagaccatctccaaggccaagggccagcccagggagccccaggtgtacaccctgcccccctccagggaggagatgaccaagaaccaggtgtccctgacctgcctggtgaagggcttctacccctccgacatcgccgtggagtgggagtccaacggccagcccgagaacaactacaagaccaccccccccgtgctggactccgacggctccttcttcctgtactccaagctgaccgtggacaagtccaggtggcagcagggcaacgtgttctcctgctccgtgatgcacgaggccctgcacaaccactacacccagaagtccctgtccctgtcccccggcaagtga

SEQ ID NO: 99 - DNA, 2949 bp, Artificial Sequence
  hDAO-Fc-Hepmut4-Cysmut
atgccggccctgggctgggccgtggctgccatcctgatgctgcagacggccatggcggagccctccccggggactctgcccaggaaggcaggggtgttttcagacctaagcaaccaagagctgaaggcagtgcacagcttcctctggtccaagaaggagctgaggctgcagccctccagtaccaccaccatggccaagaacaccgtgtttctcatcgagatgctgctgcccaagaagtaccatgtgctgaggtttctggataaaggtgaaaggcatcctgtgcgggaagcccgtgccgtcatcttctttggtgaccaggagcatcccaatgtcaccgagtttgctgtggggcccctgccagggcccgcctacatgcgagcactgtcccccaggcctgggtaccagtcctcctgggcatcgaggcccatctccacagcagagtatgccctcctctaccacaccctgcaggaagccaccaagcccctgcatcagttcttcctcaataccacaggcttctcattccaagactgccatgacagatgcctggccttcaccgatgtggccccccggggtgtggcttctggccagcgccgcagttggcttatcatacagcgctatgtagaaggctactttctgcaccccactgggctggagctcctcgtggatcatgggagcacagatgctgggcactgggccgtggagcaggtgtggtacaacgggaagttctatgggagcccagaggaactggctcggaagtatgcagatggagaggtggacgtggtggtcctggaggacccgctgcctgggggcaaggggcatgacagcacagaggagccgcccctcttctcctcccacaagccccgcggggacttccccagccccatccatgtgagcggcccccgcttggtccagccccacggccctcgcttcaggctggagggcaacgctgtgctctacggcggctggagctttgccttccggctgcgctcctcctccgggctgcaggtcctgaacgtgcacttcggcggagagcgcattgcctatgaggtcagcgtgcaagaggcagtggcgctgtatggaggacacacacctgcaggcatgcagaccaagtacctcgatgtcggctggggcctgggcagcgtcactcatgagttagcccccggcatcgactgcccggagaccgccaccttcctggacactttccactactatgatgccgatgacccggtccattatccccgagccctctgcctctttgaaatgcccacaggggtgccccttcggcggcactttaattccaactttaaaggtggcttcaacttctatgcggggctgaagggccaggtgctggtgctgcggacaacttcaactgtctacaattatgattacatttgggactttatcttctaccccaacggggtgatggaggccaagatgcatgccactggctacgtccacgccaccttctacacccccgaggggctgcgccacggcactcgcctgcacacccacctgattggcaacatacacactcacttggtgcactaccgcgtagacctggatgtggcaggcaccaagaacagcttccagacactgcagatgaagctagaaaacatcaccaacccctggagcccaagacaccgcgtggtccagccaactctggagcagacgcagtactcctgggagcgccaggcggccttcagcttcaaaacgaagctgcccaagtacctgctctttaccagcccccaggagaacccctggggccacaagcgcagctaccgcctgcagatccactccatggccgaccaggtgctgcccccaggctggcaggaggagcaggccatcacctgggcaaggtaccccctggcagtgaccaagtaccgggagtcggagctgtgcagcagcagcatctaccaccagaacgacccctggcacccgcccgtggtctttgagcagtttcttcacaacaacgagaacattgaaaatgaggacctggtggcctgggtgacggtgggcttcctgcacatcccccactcagaggacattcccaacacagccacacctgggaactccgtgggcttcctgctccggccattcaacttcttcccagaggacccctccctggcatccagagacactgtgatcgtgtggcctcgggacaacggccccaactacgtccagcgctggatccctgaggacagggactgctcgatgcctcccccttttagctacaatgggacctatagacctgtggagcccaagtccgccgacaagacccacacctgccccccctgccccgccccccccgtggccggcccctccgtgttcctgttcccccccaagcccaaggacaccctgatgatctccaggacccccgaggtgacctgcgtggtggtggacgtgtcccacgaggaccccgaggtgaagttcaactggtacgtggacggcgtggaggtgcacaacgccaagaccaagcccagggaggagcagtacaactccacctacagggtggtgtccgtgctgaccgtgctgcaccaggactggctgaacggcaaggagtacaagtgcaaggtgtccaacaagggcctgccctcctccatcgagaagaccatctccaaggccaagggccagcccagggagccccaggtgtacaccctgcccccctccagggaggagatgaccaagaaccaggtgtccctgacctgcctggtgaagggcttctacccctccgacatcgccgtggagtgggagtccaacggccagcccgagaacaactacaagaccaccccccccgtgctggactccgacggctccttcttcctgtactccaagctgaccgtggacaagtccaggtggcagcagggcaacgtgttctcctgctccgtgatgcacgaggccctgcacaaccactacacccagaagtccctgtccctgtcccccggcaagtga

SEQ ID NO: 100 - DNA, 2949 bp, Artificial Sequence
  hDAO-Fc-Hepmut5-Cysmut
atgccggccctgggctgggccgtggctgccatcctgatgctgcagacggccatggcggagccctccccggggactctgcccaggaaggcaggggtgttttcagacctaagcaaccaagagctgaaggcagtgcacagcttcctctggtccaagaaggagctgaggctgcagccctccagtaccaccaccatggccaagaacaccgtgtttctcatcgagatgctgctgcccaagaagtaccatgtgctgaggtttctggataaaggtgaaaggcatcctgtgcgggaagcccgtgccgtcatcttctttggtgaccaggagcatcccaatgtcaccgagtttgctgtggggcccctgccagggcccgcctacatgcgagcactgtcccccaggcctgggtaccagtcctcctgggcatcgaggcccatctccacagcagagtatgccctcctctaccacaccctgcaggaagccaccaagcccctgcatcagttcttcctcaataccacaggcttctcattccaagactgccatgacagatgcctggccttcaccgatgtggccccccggggtgtggcttctggccagcgccgcagttggcttatcatacagcgctatgtagaaggctactttctgcaccccactgggctggagctcctcgtggatcatgggagcacagatgctgggcactgggccgtggagcaggtgtggtacaacgggaagttctatgggagcccagaggaactggctcggaagtatgcagatggagaggtggacgtggtggtcctggaggacccgctgcctgggggcaaggggcatgacagcacagaggagccgcccctcttctcctcccacaagccccgcggggacttccccagccccatccatgtgagcggcccccgcttggtccagccccacggccctcgcttcaggctggagggcaacgctgtgctctacggcggctggagctttgccttccggctgcgctcctcctccgggctgcaggtcctgaacgtgcacttcggcggagagcgcattgcctatgaggtcagcgtgcaagaggcagtggcgctgtatggaggacacacacctgcaggcatgcagaccaagtacctcgatgtcggctggggcctgggcagcgtcactcatgagttagcccccggcatcgactgcccggagaccgccaccttcctggacactttccactactatgatgccgatgacccggtccattatccccgagccctctgcctctttgaaatgcccacaggggtgccccttcggcggcactttaattccaactttaaaggtggcttcaacttctatgcggggctgaagggccaggtgctggtgctgcggacaacttcaactgtctacaattatgattacatttgggactttatcttctaccccaacggggtgatggaggccaagatgcatgccactggctacgtccacgccaccttctacacccccgaggggctgcgccacggcactcgcctgcacacccacctgattggcaacatacacactcacttggtgcactaccgcgtagacctggatgtggcaggcaccaagaacagcttccagacactgcagatgaagctagaaaacatcaccaacccctggagcccaagacaccgcgtggtccagccaactctggagcagacgcagtactcctgggagcgccaggcggccttccgcttcaaaacgaagctgcccacgtacctgctctttaccagcccccaggagaacccctggggccacaagcgcagctaccgcctgcagatccactccatggccgaccaggtgctgcccccaggctggcaggaggagcaggccatcacctgggcaaggtaccccctggcagtgaccaagtaccgggagtcggagctgtgcagcagcagcatctaccaccagaacgacccctggcacccgcccgtggtctttgagcagtttcttcacaacaacgagaacattgaaaatgaggacctggtggcctgggtgacggtgggcttcctgcacatcccccactcagaggacattcccaacacagccacacctgggaactccgtgggcttcctgctccggccattcaacttcttcccagaggacccctccctggcatccagagacactgtgatcgtgtggcctcgggacaacggccccaactacgtccagcgctggatccctgaggacagggactgctcgatgcctcccccttttagctacaatgggacctatagacctgtggagcccaagtccgccgacaagacccacacctgccccccctgccccgccccccccgtggccggcccctccgtgttcctgttcccccccaagcccaaggacaccctgatgatctccaggacccccgaggtgacctgcgtggtggtggacgtgtcccacgaggaccccgaggtgaagttcaactggtacgtggacggcgtggaggtgcacaacgccaagaccaagcccagggaggagcagtacaactccacctacagggtggtgtccgtgctgaccgtgctgcaccaggactggctgaacggcaaggagtacaagtgcaaggtgtccaacaagggcctgccctcctccatcgagaagaccatctccaaggccaagggccagcccagggagccccaggtgtacaccctgcccccctccagggaggagatgaccaagaaccaggtgtccctgacctgcctggtgaagggcttctacccctccgacatcgccgtggagtgggagtccaacggccagcccgagaacaactacaagaccaccccccccgtgctggactccgacggctccttcttcctgtactccaagctgaccgtggacaagtccaggtggcagcagggcaacgtgttctcctgctccgtgatgcacgaggccctgcacaaccactacacccagaagtccctgtccctgtcccccggcaagtga

SEQ ID NO: 101 - DNA, 2949 bp, Artificial Sequence
  hDAO-Fc-Hepmut6-Cysmut
atgccggccctgggctgggccgtggctgccatcctgatgctgcagacggccatggcggagccctccccggggactctgcccaggaaggcaggggtgttttcagacctaagcaaccaagagctgaaggcagtgcacagcttcctctggtccaagaaggagctgaggctgcagccctccagtaccaccaccatggccaagaacaccgtgtttctcatcgagatgctgctgcccaagaagtaccatgtgctgaggtttctggataaaggtgaaaggcatcctgtgcgggaagcccgtgccgtcatcttctttggtgaccaggagcatcccaatgtcaccgagtttgctgtggggcccctgccagggcccgcctacatgcgagcactgtcccccaggcctgggtaccagtcctcctgggcatcgaggcccatctccacagcagagtatgccctcctctaccacaccctgcaggaagccaccaagcccctgcatcagttcttcctcaataccacaggcttctcattccaagactgccatgacagatgcctggccttcaccgatgtggccccccggggtgtggcttctggccagcgccgcagttggcttatcatacagcgctatgtagaaggctactttctgcaccccactgggctggagctcctcgtggatcatgggagcacagatgctgggcactgggccgtggagcaggtgtggtacaacgggaagttctatgggagcccagaggaactggctcggaagtatgcagatggagaggtggacgtggtggtcctggaggacccgctgcctgggggcaaggggcatgacagcacagaggagccgcccctcttctcctcccacaagccccgcggggacttccccagccccatccatgtgagcggcccccgcttggtccagccccacggccctcgcttcaggctggagggcaacgctgtgctctacggcggctggagctttgccttccggctgcgctcctcctccgggctgcaggtcctgaacgtgcacttcggcggagagcgcattgcctatgaggtcagcgtgcaagaggcagtggcgctgtatggaggacacacacctgcaggcatgcagaccaagtacctcgatgtcggctggggcctgggcagcgtcactcatgagttagcccccggcatcgactgcccggagaccgccaccttcctggacactttccactactatgatgccgatgacccggtccattatccccgagccctctgcctctttgaaatgcccacaggggtgccccttcggcggcactttaattccaactttaaaggtggcttcaacttctatgcggggctgaagggccaggtgctggtgctgcggacaacttcaactgtctacaattatgattacatttgggactttatcttctaccccaacggggtgatggaggccaagatgcatgccactggctacgtccacgccaccttctacacccccgaggggctgcgccacggcactcgcctgcacacccacctgattggcaacatacacactcacttggtgcactaccgcgtagacctggatgtggcaggcaccaagaacagcttccagacactgcagatgaagctagaaaacatcaccaacccctggagcccaagacaccgcgtggtccagccaactctggagcagacgcagtactcctgggagcgccaggcggccttccgcttcggacagacgctgcccaagtacctgctctttaccagcccccaggagaacccctggggccacaagcgcagctaccgcctgcagatccactccatggccgaccaggtgctgcccccaggctggcaggaggagcaggccatcacctgggcaaggtaccccctggcagtgaccaagtaccgggagtcggagctgtgcagcagcagcatctaccaccagaacgacccctggcacccgcccgtggtctttgagcagtttcttcacaacaacgagaacattgaaaatgaggacctggtggcctgggtgacggtgggcttcctgcacatcccccactcagaggacattcccaacacagccacacctgggaactccgtgggcttcctgctccggccattcaacttcttcccagaggacccctccctggcatccagagacactgtgatcgtgtggcctcgggacaacggccccaactacgtccagcgctggatccctgaggacagggactgctcgatgcctcccccttttagctacaatgggacctatagacctgtggagcccaagtccgccgacaagacccacacctgccccccctgccccgccccccccgtggccggcccctccgtgttcctgttcccccccaagcccaaggacaccctgatgatctccaggacccccgaggtgacctgcgtggtggtggacgtgtcccacgaggaccccgaggtgaagttcaactggtacgtggacggcgtggaggtgcacaacgccaagaccaagcccagggaggagcagtacaactccacctacagggtggtgtccgtgctgaccgtgctgcaccaggactggctgaacggcaaggagtacaagtgcaaggtgtccaacaagggcctgccctcctccatcgagaagaccatctccaaggccaagggccagcccagggagccccaggtgtacaccctgcccccctccagggaggagatgaccaagaaccaggtgtccctgacctgcctggtgaagggcttctacccctccgacatcgccgtggagtgggagtccaacggccagcccgagaacaactacaagaccaccccccccgtgctggactccgacggctccttcttcctgtactccaagctgaccgtggacaagtccaggtggcagcagggcaacgtgttctcctgctccgtgatgcacgaggccctgcacaaccactacacccagaagtccctgtccctgtcccccggcaagtga

SEQ ID NO: 102 - DNA, 2949 bp, Artificial Sequence
  hDAO-Fc-Hepmut7-Cysmut
atgccggccctgggctgggccgtggctgccatcctgatgctgcagacggccatggcggagccctccccggggactctgcccaggaaggcaggggtgttttcagacctaagcaaccaagagctgaaggcagtgcacagcttcctctggtccaagaaggagctgaggctgcagccctccagtaccaccaccatggccaagaacaccgtgtttctcatcgagatgctgctgcccaagaagtaccatgtgctgaggtttctggataaaggtgaaaggcatcctgtgcgggaagcccgtgccgtcatcttctttggtgaccaggagcatcccaatgtcaccgagtttgctgtggggcccctgccagggcccgcctacatgcgagcactgtcccccaggcctgggtaccagtcctcctgggcatcgaggcccatctccacagcagagtatgccctcctctaccacaccctgcaggaagccaccaagcccctgcatcagttcttcctcaataccacaggcttctcattccaagactgccatgacagatgcctggccttcaccgatgtggccccccggggtgtggcttctggccagcgccgcagttggcttatcatacagcgctatgtagaaggctactttctgcaccccactgggctggagctcctcgtggatcatgggagcacagatgctgggcactgggccgtggagcaggtgtggtacaacgggaagttctatgggagcccagaggaactggctcggaagtatgcagatggagaggtggacgtggtggtcctggaggacccgctgcctgggggcaaggggcatgacagcacagaggagccgcccctcttctcctcccacaagccccgcggggacttccccagccccatccatgtgagcggcccccgcttggtccagccccacggccctcgcttcaggctggagggcaacgctgtgctctacggcggctggagctttgccttccggctgcgctcctcctccgggctgcaggtcctgaacgtgcacttcggcggagagcgcattgcctatgaggtcagcgtgcaagaggcagtggcgctgtatggaggacacacacctgcaggcatgcagaccaagtacctcgatgtcggctggggcctgggcagcgtcactcatgagttagcccccggcatcgactgcccggagaccgccaccttcctggacactttccactactatgatgccgatgacccggtccattatccccgagccctctgcctctttgaaatgcccacaggggtgccccttcggcggcactttaattccaactttaaaggtggcttcaacttctatgcggggctgaagggccaggtgctggtgctgcggacaacttcaactgtctacaattatgattacatttgggactttatcttctaccccaacggggtgatggaggccaagatgcatgccactggctacgtccacgccaccttctacacccccgaggggctgcgccacggcactcgcctgcacacccacctgattggcaacatacacactcacttggtgcactaccgcgtagacctggatgtggcaggcaccaagaacagcttccagacactgcagatgaagctagaaaacatcaccaacccctggagcccaagacaccgcgtggtccagccaactctggagcagacgcagtactcctgggagcgccaggcggccttcagcttcaaaaggaagctgcccacgtacctgctctttaccagcccccaggagaacccctggggccacaagcgcagctaccgcctgcagatccactccatggccgaccaggtgctgcccccaggctggcaggaggagcaggccatcacctgggcaaggtaccccctggcagtgaccaagtaccgggagtcggagctgtgcagcagcagcatctaccaccagaacgacccctggcacccgcccgtggtctttgagcagtttcttcacaacaacgagaacattgaaaatgaggacctggtggcctgggtgacggtgggcttcctgcacatcccccactcagaggacattcccaacacagccacacctgggaactccgtgggcttcctgctccggccattcaacttcttcccagaggacccctccctggcatccagagacactgtgatcgtgtggcctcgggacaacggccccaactacgtccagcgctggatccctgaggacagggactgctcgatgcctcccccttttagctacaatgggacctatagacctgtggagcccaagtccgccgacaagacccacacctgccccccctgccccgccccccccgtggccggcccctccgtgttcctgttcccccccaagcccaaggacaccctgatgatctccaggacccccgaggtgacctgcgtggtggtggacgtgtcccacgaggaccccgaggtgaagttcaactggtacgtggacggcgtggaggtgcacaacgccaagaccaagcccagggaggagcagtacaactccacctacagggtggtgtccgtgctgaccgtgctgcaccaggactggctgaacggcaaggagtacaagtgcaaggtgtccaacaagggcctgccctcctccatcgagaagaccatctccaaggccaagggccagcccagggagccccaggtgtacaccctgcccccctccagggaggagatgaccaagaaccaggtgtccctgacctgcctggtgaagggcttctacccctccgacatcgccgtggagtgggagtccaacggccagcccgagaacaactacaagaccaccccccccgtgctggactccgacggctccttcttcctgtactccaagctgaccgtggacaagtccaggtggcagcagggcaacgtgttctcctgctccgtgatgcacgaggccctgcacaaccactacacccagaagtccctgtccctgtcccccggcaagtga

SEQ ID NO: 103 - protein, 585 aa, Homo sapiens [sequence omitted]

SEQ ID NO: 104 - DNA, 21 bp, Artificial Sequence
  forward primer
cagaccacaggcttctcattc

SEQ ID NO: 105 - DNA, 18 bp, Artificial Sequence
  reverse primer
gaggaagaactgatgcag

SEQ ID NO: 106 - protein, 751 aa, Artificial Sequence
  hDAO-Hepmut4 Asn168Gln
MPALGWAVAAILMLQTAMAEPSPGTLPRKAGVFSDLSNQELKAVHSFLWSKKELRLQPSSTTTMAKNTVFLIEMLLPKKYHVLRFLDKGERHPVREARAVIFFGDQEHPNVTEFAVGPLPGPCYMRALSPRPGYQSSWASRPISTAEYALLYHTLQEATKPLHQFFLQTTGFSFQDCHDRCLAFTDVAPRGVASGQRRSWLIIQRYVEGYFLHPTGLELLVDHGSTDAGHWAVEQVWYNGKFYGSPEELARKYADGEVDVVVLEDPLPGGKGHDSTEEPPLFSSHKPRGDFPSPIHVSGPRLVQPHGPRFRLEGNAVLYGGWSFAFRLRSSSGLQVLNVHFGGERIAYEVSVQEAVALYGGHTPAGMQTKYLDVGWGLGSVTHELAPGIDCPETATFLDTFHYYDADDPVHYPRALCLFEMPTGVPLRRHFNSNFKGGFNFYAGLKGQVLVLRTTSTVYNYDYIWDFIFYPNGVMEAKMHATGYVHATFYTPEGLRHGTRLHTHLIGNIHTHLVHYRVDLDVAGTKNSFQTLQMKLENITNPWSPRHRVVQPTLEQTQYSWERQAAFSFKTKLPKYLLFTSPQENPWGHKRSYRLQIHSMADQVLPPGWQEEQAITWARYPLAVTKYRESELCSSSIYHQNDPWHPPVVFEQFLHNNENIENEDLVAWVTVGFLHIPHSEDIPNTATPGNSVGFLLRPFNFFPEDPSLASRDTVIVWPRDNGPNYVQRWIPEDRDCSMPPPFSYNGTYRPV